European Patent Specification EP 4 463 553 B1, published October 1, 2025. Title: Please add. Applicant: Arnatar. The sequence listing filed with the application follows.

SEQUENCE LISTING (234 sequences)

SEQ ID NO: 1 - DNA, 19 bp, synthetic construct
  source 1..19: mol_type = other DNA
gcgtcaccaaaaagcgcaa

SEQ ID NO: 2 - RNA, 19 nt, synthetic construct
  source 1..19: mol_type = other RNA
gcgtcaccaaaaagcgcaa

SEQ ID NO: 3 - DNA, 18 bp, synthetic construct
  source 1..18: mol_type = other DNA
cgggtggatgctgagaac

SEQ ID NO: 4 - DNA, 21 bp, synthetic construct
  source 1..21: mol_type = other DNA
tgcttcccattgtcaatctcc

SEQ ID NO: 5 - DNA, 23 bp, synthetic construct
  source 1..23: mol_type = other DNA
agtgaggagctgcgtgagaccaa

SEQ ID NO: 6 - DNA, 22 bp, synthetic construct
  source 1..22: mol_type = other DNA
ggaccaggtggaacagtataag

SEQ ID NO: 7 - DNA, 20 bp, synthetic construct
  source 1..20: mol_type = other DNA
tcaatgcggattcgagactg

SEQ ID NO: 8 - DNA, 28 bp, synthetic construct
  source 1..28: mol_type = other DNA
cagcttggcggagtatgtcttttctagc

SEQ ID NO: 9 - DNA, 19 bp, synthetic construct
  source 1..19: mol_type = other DNA
agggttacatgaagcacgc

SEQ ID NO: 10 - DNA, 22 bp, synthetic construct
  source 1..22: mol_type = other DNA
agagaacttgtccttaacggtg

SEQ ID NO: 11 - DNA, 23 bp, synthetic construct
  source 1..23: mol_type = other DNA
agggaactgaagccatcggtcac

SEQ ID NO: 12 - DNA, 21 bp, synthetic construct
  source 1..21: mol_type = other DNA
gcttggcttcttctggactca

SEQ ID NO: 13 - DNA, 18 bp, synthetic construct
  source 1..18: mol_type = other DNA
tcgcgagcttcaccatga

SEQ ID NO: 14 - DNA, 24 bp, synthetic construct
  source 1..24: mol_type = other DNA
cgccacttgtccgcttcacactcc

SEQ ID NO: 15 - RNA, 21 nt, synthetic construct
  source 1..21: mol_type = other RNA
  modified_base 20: mod_base = OTHER; note = 2'-deoxy thymidine
  modified_base 21: mod_base = OTHER; note = 2'-deoxy thymidine
gcgtcaccaaaaagcgcaatt

SEQ ID NO: 16 - RNA, 21 nt, synthetic construct
  source 1..21: mol_type = other RNA
  modified_base 1: mod_base = OTHER; note = 2'-O-methyl guanosine
  modified_base 2: mod_base = OTHER; note = 2'-O-methyl cytidine 5'-thiophosphate
  modified_base 3: mod_base = OTHER; note = 2'-O-methyl guanosine 5'-thiophosphate
  modified_base 4: mod_base = OTHER; note = 2'-O-methyl uridine
  modified_base 5: mod_base = OTHER; note = 2'-O-methyl cytidine
  modified_base 6: mod_base = OTHER; note = 2'-O-methyl adenosine
  modified_base 7: mod_base = OTHER; note = 2'-fluoro cytidine
  modified_base 8: mod_base = OTHER; note = 2'-O-methyl cytidine
  modified_base 9: mod_base = OTHER; note = 2'-fluoro adenosine
  modified_base 10: mod_base = OTHER; note = 2'-fluoro adenosine
  modified_base 11: mod_base = OTHER; note = 2'-fluoro adenosine
  modified_base 12: mod_base = OTHER; note = 2'-O-methyl adenosine
  modified_base 13: mod_base = OTHER; note = 2'-O-methyl adenosine
  modified_base 14: mod_base = OTHER; note = 2'-O-methyl guanosine
  modified_base 15: mod_base = OTHER; note = 2'-O-methyl cytidine
  modified_base 16: mod_base = OTHER; note = 2'-O-methyl guanosine
  modified_base 17: mod_base = OTHER; note = 2'-O-methyl cytidine
  modified_base 18: mod_base = OTHER; note = 2'-O-methyl adenosine
  modified_base 19: mod_base = OTHER; note = 2'-O-methyl adenosine
  modified_base 20: mod_base = OTHER; note = 2'-deoxy thymidine 5'-thiophosphate
  modified_base 21: mod_base = OTHER; note = 2'-deoxy thymidine 5'-thiophosphate
gcgtcaccaaaaagcgcaatt

SEQ ID NO: 17 - RNA, 21 nt, synthetic construct
  source 1..21: mol_type = other RNA
  modified_base 1: mod_base = OTHER; note = 2'-O-methyl guanosine
  modified_base 2: mod_base = OTHER; note = 2'-O-methyl cytidine 5'-thiophosphate
  modified_base 3: mod_base = OTHER; note = 2'-O-methyl guanosine 5'-thiophosphate
  modified_base 4: mod_base = OTHER; note = 2'-O-methyl uridine
  modified_base 5: mod_base = OTHER; note = 2'-O-methyl cytidine
  modified_base 6: mod_base = OTHER; note = 2'-O-methyl adenosine
  modified_base 7: mod_base = OTHER; note = 2'-fluoro cytidine
  modified_base 8: mod_base = OTHER; note = 2'-O-methyl cytidine
  modified_base 9: mod_base = OTHER; note = 2'-fluoro adenosine
  modified_base 10: mod_base = OTHER; note = 2'-fluoro adenosine
  modified_base 11: mod_base = OTHER; note = 2'-fluoro adenosine
  modified_base 12: mod_base = OTHER; note = 2'-O-methyl adenosine
  modified_base 13: mod_base = OTHER; note = 2'-O-methyl adenosine
  modified_base 14: mod_base = OTHER; note = 2'-O-methyl guanosine
  modified_base 15: mod_base = OTHER; note = 2'-O-methyl cytidine
  modified_base 16: mod_base = OTHER; note = 2'-O-methyl guanosine
  modified_base 17: mod_base = OTHER; note = 2'-O-methyl cytidine
  modified_base 18: mod_base = OTHER; note = 2'-O-methyl adenosine
  modified_base 19: mod_base = OTHER; note = 2'-O-methyl adenosine
  modified_base 20: mod_base = OTHER; note = 2'-deoxy thymidine 5'-thiophosphate
  modified_base 21: mod_base = OTHER; note = 2'-deoxy thymidine 5'-thiophosphate
  misc_feature 21: note = 3'-O attached to a GalNAc-comprising compound via a linker
gcgtcaccaaaaagcgcaatt

SEQ ID NO: 18 - RNA, 21 nt, synthetic construct
  source 1..21: mol_type = other RNA
  modified_base 1: mod_base = OTHER; note = 2'-O-methyl guanosine
  modified_base 2: mod_base = OTHER; note = 2'-O-methyl cytidine
  modified_base 3: mod_base = OTHER; note = 2'-O-methyl guanosine
  modified_base 20: mod_base = OTHER; note = 2'-deoxy thymidine
  modified_base 21: mod_base = OTHER; note = 2'-deoxy thymidine
gcgtcaccaaaaagcgcaatt

SEQ ID NO: 19 - RNA, 21 nt, synthetic construct
  source 1..21: mol_type = other RNA
  modified_base 1: mod_base = OTHER; note = 2'-O-methyl guanosine
  modified_base 2: mod_base = OTHER; note = 2'-O-methyl cytidine
  modified_base 20: mod_base = OTHER; note = 2'-deoxy thymidine
  modified_base 21: mod_base = OTHER; note = 2'-deoxy thymidine
gcgtcaccaaaaagcgcaatt

SEQ ID NO: 20 - RNA, 21 nt, synthetic construct
  source 1..21: mol_type = other RNA
  modified_base 1: mod_base = OTHER; note = 2'-O-methyl guanosine
  modified_base 2: mod_base = OTHER; note = 2'-O-methyl cytidine 5'-thiophosphate
  modified_base 3: mod_base = OTHER; note = guanosine 5'-thiophosphate
  modified_base 20: mod_base = OTHER; note = 2'-deoxy thymidine 5'-thiophosphate
  modified_base 21: mod_base = OTHER; note = 2'-deoxy thymidine 5'-thiophosphate
gcgtcaccaaaaagcgcaatt

SEQ ID NO: 21 - RNA, 21 nt, synthetic construct
  source 1..21: mol_type = other RNA
  modified_base 1: mod_base = OTHER; note = 2'-O-methyl guanosine
  modified_base 2: mod_base = OTHER; note = 2'-O-methyl cytidine 5'-thiophosphate
  modified_base 3: mod_base = OTHER; note = 2'-O-methyl guanosine 5'-thiophosphate
  modified_base 4: mod_base = OTHER; note = uridine 5'-thiophosphate
  modified_base 19: mod_base = OTHER; note = 2'-O-methyl adenosine 5'-thiophosphate
  modified_base 20: mod_base = OTHER; note = 2'-deoxy thymidine 5'-thiophosphate
  modified_base 21: mod_base = OTHER; note = 2'-deoxy thymidine 5'-thiophosphate
gcgtcaccaaaaagcgcaatt

SEQ ID NO: 22 - RNA, 21 nt, synthetic construct
  source 1..21: mol_type = other RNA
  modified_base 1: mod_base = OTHER; note = 2'-O-methyl guanosine
  modified_base 2: mod_base = OTHER; note = 2'-fluoro cytidine 5'-thiophosphate
  modified_base 3: mod_base = OTHER; note = 2'-O-methyl guanosine 5'-thiophosphate
  modified_base 4: mod_base = OTHER; note = 2'-O-methyl uridine
  modified_base 6: mod_base = OTHER; note = 2'-O-methyl adenosine 5'-thiophosphate
  modified_base 8: mod_base = OTHER; note = 2'-O-methyl cytidine 5'-thiophosphate
  modified_base 9: mod_base = OTHER; note = 2'-fluoro adenosine
  modified_base 10: mod_base = OTHER; note = 2'-fluoro adenosine
  modified_base 11: mod_base = OTHER; note = 2'-O-methyl adenosine
  modified_base 12: mod_base = OTHER; note = 2'-O-methyl adenosine
  modified_base 14: mod_base = OTHER; note = 2'-O-methyl guanosine 5'-thiophosphate
  modified_base 16: mod_base = OTHER; note = 2'-O-methyl guanosine 5'-thiophosphate
  modified_base 17: mod_base = OTHER; note = 2'-O-methyl cytidine
  modified_base 18: mod_base = OTHER; note = 2'-fluoro adenosine
  modified_base 19: mod_base = OTHER; note = 2'-O-methyl adenosine
  modified_base 20: mod_base = OTHER; note = 2'-deoxy thymidine 5'-thiophosphate
  modified_base 21: mod_base = OTHER; note = 2'-deoxy thymidine 5'-thiophosphate
gcgtcaccaaaaagcgcaatt

SEQ ID NO: 23 - RNA, 21 nt, synthetic construct
  source 1..21: mol_type = other RNA
  modified_base 1: mod_base = OTHER; note = 2'-O-methyl guanosine
  modified_base 2: mod_base = OTHER; note = 2'-fluoro cytidine 5'-thiophosphate
  modified_base 3: mod_base = OTHER; note = 2'-O-methyl guanosine 5'-thiophosphate
  modified_base 4: mod_base = OTHER; note = 2'-O-methyl uridine
  modified_base 6: mod_base = OTHER; note = 2'-O-methyl adenosine 5'-thiophosphate
  modified_base 8: mod_base = OTHER; note = 2'-O-methyl cytidine 5'-thiophosphate
  modified_base 9: mod_base = OTHER; note = 2'-fluoro adenosine
  modified_base 10: mod_base = OTHER; note = 2'-fluoro adenosine
  modified_base 11: mod_base = OTHER; note = 2'-O-methyl adenosine
  modified_base 12: mod_base = OTHER; note = 2'-O-methyl adenosine
  modified_base 14: mod_base = OTHER; note = 2'-O-methyl guanosine 5'-thiophosphate
  modified_base 16: mod_base = OTHER; note = 2'-O-methyl guanosine 5'-thiophosphate
  modified_base 17: mod_base = OTHER; note = 2'-O-methyl cytidine
  modified_base 18: mod_base = OTHER; note = 2'-fluoro adenosine
  modified_base 19: mod_base = OTHER; note = 2'-O-methyl adenosine
  modified_base 20: mod_base = OTHER; note = 2'-deoxy thymidine 5'-thiophosphate
  modified_base 21: mod_base = OTHER; note = 2'-deoxy thymidine 5'-thiophosphate
  misc_feature 21: note = 3'-O attached to a GalNAc-comprising compound via a linker
gcgtcaccaaaaagcgcaatt

SEQ ID NO: 24 - RNA, 21 nt, synthetic construct
  source 1..21: mol_type = other RNA
  modified_base 1: mod_base = OTHER; note = 2'-O-methyl guanosine
  modified_base 2: mod_base = OTHER; note = 2'-fluoro cytidine 5'-thiophosphate
  modified_base 3: mod_base = OTHER; note = 2'-O-methyl guanosine 5'-thiophosphate
  modified_base 4: mod_base = OTHER; note = 2'-O-methyl uridine
  modified_base 6: mod_base = OTHER; note = 2'-O-methyl adenosine 5'-thiophosphate
  modified_base 8: mod_base = OTHER; note = 2'-O-methyl cytidine 5'-thiophosphate
  modified_base 9: mod_base = OTHER; note = 2'-fluoro adenosine
  modified_base 10: mod_base = OTHER; note = 2'-fluoro adenosine
  modified_base 11: mod_base = OTHER; note = 2'-O-methyl adenosine
  modified_base 12: mod_base = OTHER; note = 2'-O-methyl adenosine
  modified_base 14: mod_base = OTHER; note = 2'-O-methyl guanosine 5'-thiophosphate
  modified_base 16: mod_base = OTHER; note = 2'-O-methyl guanosine 5'-thiophosphate
  modified_base 17: mod_base = OTHER; note = 2'-O-methyl cytidine
  modified_base 19: mod_base = OTHER; note = 2'-O-methyl adenosine 5'-thiophosphate
  modified_base 20: mod_base = OTHER; note = 2'-deoxy thymidine 5'-thiophosphate
  modified_base 21: mod_base = OTHER; note = 2'-deoxy thymidine 5'-thiophosphate
gcgtcaccaaaaagcgcaatt

SEQ ID NO: 25 - RNA, 21 nt, synthetic construct
  source 1..21: mol_type = other RNA
  modified_base 1: mod_base = OTHER; note = 2'-O-methyl guanosine
  modified_base 2: mod_base = OTHER; note = 2'-fluoro cytidine 5'-thiophosphate
  modified_base 3: mod_base = OTHER; note = 2'-O-methyl guanosine 5'-thiophosphate
  modified_base 4: mod_base = OTHER; note = 2'-O-methyl uridine
  modified_base 6: mod_base = OTHER; note = 2'-O-methyl adenosine 5'-thiophosphate
  modified_base 8: mod_base = OTHER; note = 2'-O-methyl cytidine 5'-thiophosphate
  modified_base 9: mod_base = OTHER; note = 2'-fluoro adenosine
  modified_base 10: mod_base = OTHER; note = 2'-fluoro adenosine
  modified_base 12: mod_base = OTHER; note = 2'-O-methyl adenosine 5'-thiophosphate
  modified_base 14: mod_base = OTHER; note = 2'-O-methyl guanosine 5'-thiophosphate
  modified_base 16: mod_base = OTHER; note = 2'-O-methyl guanosine 5'-thiophosphate
  modified_base 17: mod_base = OTHER; note = 2'-O-methyl cytidine
  modified_base 19: mod_base = OTHER; note = 2'-O-methyl adenosine 5'-thiophosphate
  modified_base 20: mod_base = OTHER; note = 2'-deoxy thymidine 5'-thiophosphate
  modified_base 21: mod_base = OTHER; note = 2'-deoxy thymidine 5'-thiophosphate
gcgtcaccaaaaagcgcaatt

SEQ ID NO: 26 - RNA, 21 nt, synthetic construct
  source 1..21: mol_type = other RNA
  modified_base 1: mod_base = OTHER; note = 2'-O-methyl guanosine
  modified_base 2: mod_base = OTHER; note = 2'-fluoro cytidine 5'-thiophosphate
  modified_base 3: mod_base = OTHER; note = 2'-O-methyl guanosine 5'-thiophosphate
  modified_base 4: mod_base = OTHER; note = 2'-O-methyl uridine
  modified_base 5: mod_base = OTHER; note = 2'-deoxy cytidine
  modified_base 6: mod_base = OTHER; note = 2'-O-methyl adenosine 5'-thiophosphate
  modified_base 7: mod_base = OTHER; note = 2'-deoxy cytidine
  modified_base 8: mod_base = OTHER; note = 2'-O-methyl cytidine 5'-thiophosphate
  modified_base 9: mod_base = OTHER; note = 2'-fluoro adenosine
  modified_base 10: mod_base = OTHER; note = 2'-fluoro adenosine
  modified_base 11: mod_base = OTHER; note = 2'-O-methyl adenosine
  modified_base 12: mod_base = OTHER; note = 2'-O-methyl adenosine
  modified_base 13: mod_base = OTHER; note = 2'-deoxy adenosine
  modified_base 14: mod_base = OTHER; note = 2'-O-methyl guanosine 5'-thiophosphate
  modified_base 15: mod_base = OTHER; note = 2'-deoxy cytidine
  modified_base 16: mod_base = OTHER; note = 2'-O-methyl guanosine 5'-thiophosphate
  modified_base 17: mod_base = OTHER; note = 2'-O-methyl cytidine
  modified_base 18: mod_base = OTHER; note = 2'-fluoro adenosine
  modified_base 19: mod_base = OTHER; note = 2'-O-methyl adenosine
  modified_base 20: mod_base = OTHER; note = 2'-deoxy thymidine 5'-thiophosphate
  modified_base 21: mod_base = OTHER; note = 2'-deoxy thymidine 5'-thiophosphate
gcgtcaccaaaaagcgcaatt

SEQ ID NO: 27 - RNA, 21 nt, synthetic construct
  source 1..21: mol_type = other RNA
  modified_base 1: mod_base = OTHER; note = 2'-O-methyl guanosine
  modified_base 2: mod_base = OTHER; note = 2'-fluoro cytidine 5'-thiophosphate
  modified_base 3: mod_base = OTHER; note = 2'-O-methyl guanosine 5'-thiophosphate
  modified_base 4: mod_base = OTHER; note = 2'-O-methyl uridine
  modified_base 5: mod_base = OTHER; note = 2'-deoxy cytidine
  modified_base 6: mod_base = OTHER; note = 2'-O-methyl adenosine 5'-thiophosphate
  modified_base 7: mod_base = OTHER; note = 2'-deoxy cytidine
  modified_base 8: mod_base = OTHER; note = 2'-O-methyl cytidine 5'-thiophosphate
  modified_base 9: mod_base = OTHER; note = 2'-fluoro adenosine
  modified_base 10: mod_base = OTHER; note = 2'-fluoro adenosine
  modified_base 11: mod_base = OTHER; note = 2'-O-methyl adenosine
  modified_base 12: mod_base = OTHER; note = 2'-O-methyl adenosine
  modified_base 13: mod_base = OTHER; note = 2'-deoxy adenosine
  modified_base 14: mod_base = OTHER; note = 2'-O-methyl guanosine 5'-thiophosphate
  modified_base 15: mod_base = OTHER; note = 2'-deoxy cytidine
  modified_base 16: mod_base = OTHER; note = 2'-O-methyl guanosine 5'-thiophosphate
  modified_base 17: mod_base = OTHER; note = 2'-O-methyl cytidine
  modified_base 18: mod_base = OTHER; note = 2'-fluoro adenosine
  modified_base 19: mod_base = OTHER; note = 2'-O-methyl adenosine
  modified_base 20: mod_base = OTHER; note = 2'-deoxy thymidine 5'-thiophosphate
  modified_base 21: mod_base = OTHER; note = 2'-deoxy thymidine 5'-thiophosphate
  misc_feature 21: note = 3'-O attached to a GalNAc-comprising compound via a linker
gcgtcaccaaaaagcgcaatt

SEQ ID NO: 28 - RNA, 21 nt, synthetic construct
  source 1..21: mol_type = other RNA
  modified_base 1: mod_base = OTHER; note = 2'-O-methyl guanosine
  modified_base 2: mod_base = OTHER; note = 2'-fluoro cytidine 5'-thiophosphate
  modified_base 3: mod_base = OTHER; note = 2'-O-methyl guanosine 5'-thiophosphate
  modified_base 4: mod_base = OTHER; note = 2'-O-methyl uridine
  modified_base 5: mod_base = OTHER; note = cytidine 5'-thiophosphate
  modified_base 6: mod_base = OTHER; note = 2'-O-methyl adenosine 5'-thiophosphate
  modified_base 7: mod_base = OTHER; note = cytidine 5'-thiophosphate
  modified_base 8: mod_base = OTHER; note = 2'-O-methyl cytidine 5'-thiophosphate
  modified_base 9: mod_base = OTHER; note = 2'-fluoro adenosine
  modified_base 10: mod_base = OTHER; note = 2'-fluoro adenosine
  modified_base 11: mod_base = OTHER; note = 2'-O-methyl adenosine
  modified_base 12: mod_base = OTHER; note = 2'-O-methyl adenosine
  modified_base 13: mod_base = OTHER; note = adenosine 5'-thiophosphate
  modified_base 14: mod_base = OTHER; note = 2'-O-methyl guanosine 5'-thiophosphate
  modified_base 15: mod_base = OTHER; note = cytidine 5'-thiophosphate
  modified_base 16: mod_base = OTHER; note = 2'-O-methyl guanosine 5'-thiophosphate
  modified_base 17: mod_base = OTHER; note = 2'-O-methyl cytidine
  modified_base 18: mod_base = OTHER; note = 2'-fluoro adenosine
  modified_base 19: mod_base = OTHER; note = 2'-O-methyl adenosine
  modified_base 20: mod_base = OTHER; note = 2'-deoxy thymidine 5'-thiophosphate
  modified_base 21: mod_base = OTHER; note = 2'-deoxy thymidine 5'-thiophosphate
  misc_feature 21: note = 3'-O attached to a GalNAc-comprising compound via a linker
gcgtcaccaaaaagcgcaatt

SEQ ID NO: 29 - RNA, 21 nt, synthetic construct
  source 1..21: mol_type = other RNA
  modified_base 1: mod_base = OTHER; note = 2'-O-methyl guanosine
  modified_base 2: mod_base = OTHER; note = 2'-fluoro cytidine 5'-thiophosphate
  modified_base 3: mod_base = OTHER; note = 2'-O-methyl guanosine 5'-thiophosphate
  modified_base 4: mod_base = OTHER; note = 2'-O-methyl uridine
  modified_base 5: mod_base = OTHER; note = 2'-fluoro cytidine
  modified_base 6: mod_base = OTHER; note = 2'-O-methyl adenosine
  modified_base 7: mod_base = OTHER; note = 2'-fluoro cytidine
  modified_base 8: mod_base = OTHER; note = 2'-O-methyl cytidine
  modified_base 9: mod_base = OTHER; note = 2'-fluoro adenosine
  modified_base 10: mod_base = OTHER; note = 2'-fluoro adenosine
  modified_base 11: mod_base = OTHER; note = 2'-O-methyl adenosine
  modified_base 12: mod_base = OTHER; note = 2'-O-methyl adenosine
  modified_base 13: mod_base = OTHER; note = 2'-fluoro adenosine
  modified_base 14: mod_base = OTHER; note = 2'-O-methyl guanosine
  modified_base 15: mod_base = OTHER; note = 2'-fluoro cytidine
  modified_base 16: mod_base = OTHER; note = 2'-O-methyl guanosine
  modified_base 17: mod_base = OTHER; note = 2'-O-methyl cytidine
  modified_base 18: mod_base = OTHER; note = 2'-fluoro adenosine
  modified_base 19: mod_base = OTHER; note = 2'-O-methyl adenosine
  modified_base 20: mod_base = OTHER; note = 2'-deoxy thymidine 5'-thiophosphate
  modified_base 21: mod_base = OTHER; note = 2'-deoxy thymidine 5'-thiophosphate
  misc_feature 21: note = 3'-O attached to a GalNAc-comprising compound via a linker
gcgtcaccaaaaagcgcaatt

SEQ ID NO: 30 - RNA, 21 nt, synthetic construct
  source 1..21: mol_type = other RNA
  modified_base 1: mod_base = OTHER; note = 2'-O-methyl guanosine
  modified_base 2: mod_base = OTHER; note = 2'-fluoro cytidine 5'-thiophosphate
  modified_base 3: mod_base = OTHER; note = 2'-O-methyl guanosine 5'-thiophosphate
  modified_base 4: mod_base = OTHER; note = 2'-O-methyl uridine
  modified_base 5: mod_base = OTHER; note = 2'-fluoro cytidine
  modified_base 6: mod_base = OTHER; note = 2'-O-methyl adenosine
  modified_base 7: mod_base = OTHER; note = 2'-fluoro cytidine
  modified_base 8: mod_base = OTHER; note = 2'-O-methyl cytidine
  modified_base 9: mod_base = OTHER; note = 2'-fluoro adenosine
  modified_base 10: mod_base = OTHER; note = 2'-fluoro adenosine
  modified_base 11: mod_base = OTHER; note = 2'-O-methyl adenosine
  modified_base 12: mod_base = OTHER; note = 2'-O-methyl adenosine
  modified_base 13: mod_base = OTHER; note = 2'-fluoro adenosine
  modified_base 14: mod_base = OTHER; note = 2'-O-methyl guanosine
  modified_base 15: mod_base = OTHER; note = 2'-fluoro cytidine
  modified_base 16: mod_base = OTHER; note = 2'-O-methyl guanosine
  modified_base 17: mod_base = OTHER; note = 2'-O-methyl cytidine
  modified_base 18: mod_base = OTHER; note = 2'-fluoro adenosine
  modified_base 19: mod_base = OTHER; note = 2'-O-methyl adenosine
  modified_base 20: mod_base = OTHER; note = 2'-deoxy thymidine 5'-thiophosphate
  modified_base 21: mod_base = OTHER; note = 2'-deoxy thymidine 5'-thiophosphate
gcgtcaccaaaaagcgcaatt

SEQ ID NO: 31 - RNA, 21 nt, synthetic construct
  source 1..21: mol_type = other RNA
  modified_base 1: mod_base = OTHER; note = 2'-O-methyl guanosine
  modified_base 2: mod_base = OTHER; note = 2'-fluoro cytidine 5'-thiophosphate
  modified_base 3: mod_base = OTHER; note = 2'-O-methyl guanosine 5'-thiophosphate
  modified_base 4: mod_base = OTHER; note = 2'-O-methyl uridine
  modified_base 5: mod_base = OTHER; note = 2'-deoxy cytidine 5'-thiophosphate
  modified_base 6: mod_base = OTHER; note = 2'-O-methyl adenosine 5'-thiophosphate
  modified_base 7: mod_base = OTHER; note = 2'-deoxy cytidine 5'-thiophosphate
  modified_base 8: mod_base = OTHER; note = 2'-O-methyl cytidine 5'-thiophosphate
  modified_base 9: mod_base = OTHER; note = 2'-fluoro adenosine
  modified_base 10: mod_base = OTHER; note = 2'-fluoro adenosine
  modified_base 11: mod_base = OTHER; note = 2'-O-methyl adenosine
  modified_base 12: mod_base = OTHER; note = 2'-O-methyl adenosine
  modified_base 13: mod_base = OTHER; note = 2'-deoxy adenosine 5'-thiophosphate
  modified_base 14: mod_base = OTHER; note = 2'-O-methyl guanosine 5'-thiophosphate
  modified_base 15: mod_base = OTHER; note = 2'-deoxy cytidine 5'-thiophosphate
  modified_base 16: mod_base = OTHER; note = 2'-O-methyl guanosine 5'-thiophosphate
  modified_base 17: mod_base = OTHER; note = 2'-O-methyl cytidine
  modified_base 18: mod_base = OTHER; note = 2'-fluoro adenosine
  modified_base 19: mod_base = OTHER; note = 2'-O-methyl adenosine
  modified_base 20: mod_base = OTHER; note = 2'-deoxy thymidine 5'-thiophosphate
  modified_base 21: mod_base = OTHER; note = 2'-deoxy thymidine 5'-thiophosphate
  misc_feature 21: note = 3'-O attached to a GalNAc-comprising compound via a linker
gcgtcaccaaaaagcgcaatt

SEQ ID NO: 32 - RNA, 21 nt, synthetic construct
  source 1..21: mol_type = other RNA
  modified_base 1: mod_base = OTHER; note = 2'-O-methyl guanosine
  modified_base 2: mod_base = OTHER; note = 2'-fluoro cytidine 5'-thiophosphate
  modified_base 3: mod_base = OTHER; note = 2'-O-methyl guanosine 5'-thiophosphate
  modified_base 4: mod_base = OTHER; note = 2'-O-methyl uridine
  modified_base 5: mod_base = OTHER; note = 2'-deoxy cytidine 5'-thiophosphate
  modified_base 6: mod_base = OTHER; note = 2'-O-methyl adenosine
  modified_base 7: mod_base = OTHER; note = 2'-deoxy cytidine 5'-thiophosphate
  modified_base 8: mod_base = OTHER; note = 2'-O-methyl cytidine
  modified_base 9: mod_base = OTHER; note = 2'-fluoro adenosine
  modified_base 10: mod_base = OTHER; note = 2'-fluoro adenosine
  modified_base 11: mod_base = OTHER; note = 2'-O-methyl adenosine
  modified_base 12: mod_base = OTHER; note = 2'-O-methyl adenosine
  modified_base 13: mod_base = OTHER; note = 2'-deoxy adenosine 5'-thiophosphate
  modified_base 14: mod_base = OTHER; note = 2'-O-methyl guanosine
  modified_base 15: mod_base = OTHER; note = 2'-deoxy cytidine 5'-thiophosphate
  modified_base 16: mod_base = OTHER; note = 2'-O-methyl guanosine
  modified_base 17: mod_base = OTHER; note = 2'-O-methyl cytidine
  modified_base 18: mod_base = OTHER; note = 2'-fluoro adenosine
  modified_base 19: mod_base = OTHER; note = 2'-O-methyl adenosine
  modified_base 20: mod_base = OTHER; note = 2'-deoxy thymidine 5'-thiophosphate
  modified_base 21: mod_base = OTHER; note = 2'-deoxy thymidine 5'-thiophosphate
  misc_feature 21: note = 3'-O attached to a GalNAc-comprising compound via a linker
gcgtcaccaaaaagcgcaatt

SEQ ID NO: 33 - RNA, 21 nt, synthetic construct
  source 1..21: mol_type = other RNA
  modified_base 20: mod_base = OTHER; note = 2'-deoxy thymidine
  modified_base 21: mod_base = OTHER; note = 2'-deoxy thymidine
ttgcgctttttggtgacgctt

SEQ ID NO: 34 - RNA, 21 nt, synthetic construct
  source 1..21: mol_type = other RNA
  modified_base 1: mod_base = OTHER; note = 2'-O-methyl uridine
  modified_base 2: mod_base = OTHER; note = 2'-fluoro uridine 5'-thiophosphate
  modified_base 3: mod_base = OTHER; note = 2'-O-methyl guanosine 5'-thiophosphate
  modified_base 4: mod_base = OTHER; note = 2'-O-methyl cytidine
  modified_base 5: mod_base = OTHER; note = 2'-O-methyl guanosine
  modified_base 6: mod_base = OTHER; note = 2'-fluoro cytidine
  modified_base 7: mod_base = OTHER; note = 2'-O-methyl uridine
  modified_base 8: mod_base = OTHER; note = 2'-fluoro uridine
  modified_base 9: mod_base = OTHER; note = 2'-fluoro uridine
  modified_base 10: mod_base = OTHER; note = 2'-O-methyl uridine
  modified_base 11: mod_base = OTHER; note = 2'-O-methyl uridine
  modified_base 12: mod_base = OTHER; note = 2'-O-methyl guanosine
  modified_base 13: mod_base = OTHER; note = 2'-O-methyl guanosine
  modified_base 14: mod_base = OTHER; note = 2'-fluoro uridine
  modified_base 15: mod_base = OTHER; note = 2'-O-methyl guanosine
  modified_base 16: mod_base = OTHER; note = 2'-fluoro adenosine
  modified_base 17: mod_base = OTHER; note = 2'-O-methyl cytidine
  modified_base 18: mod_base = OTHER; note = 2'-O-methyl guanosine
  modified_base 19: mod_base = OTHER; note = 2'-O-methyl cytidine
  modified_base 20: mod_base = OTHER; note = 2'-deoxy thymidine 5'-thiophosphate
  modified_base 21: mod_base = OTHER; note = 2'-deoxy thymidine 5'-thiophosphate
ttgcgctttttggtgacgctt

SEQ ID NO: 35 - RNA, 21 nt, synthetic construct
  source 1..21: mol_type = other RNA
  modified_base 1: mod_base = OTHER; note = 2'-O-methyl guanosine
  modified_base 2: mod_base = OTHER; note = 2'-O-methyl cytidine
  modified_base 20: mod_base = OTHER; note = 2'-O-methyl uridine
  modified_base 21: mod_base = OTHER; note = 2'-O-methyl uridine
gcgtcaccaaaaagcgcaatt

SEQ ID NO: 36 - RNA, 21 nt, synthetic construct
  source 1..21: mol_type = other RNA
  modified_base 20: mod_base = OTHER; note = 2'-O-methyl uridine
  modified_base 21: mod_base = OTHER; note = 2'-O-methyl uridine
gcgtcaccaaaaagcgcaatt

SEQ ID NO: 37 - RNA, 21 nt, synthetic construct
  source 1..21: mol_type = other RNA
  modified_base 1: mod_base = OTHER; note = 2'-O-methyl guanosine
  modified_base 2: mod_base = OTHER; note = 2'-O-methyl cytidine
  modified_base 3: mod_base = OTHER; note = 2'-O-methyl guanosine
  modified_base 19: mod_base = OTHER; note = 2'-O-methyl adenosine
  modified_base 20: mod_base = OTHER; note = 2'-O-methyl uridine
  modified_base 21: mod_base = OTHER; note = 2'-O-methyl uridine
gcgtcaccaaaaagcgcaatt

SEQ ID NO: 38 - RNA, 21 nt, synthetic construct
  source 1..21: mol_type = other RNA
  modified_base 19: mod_base = OTHER; note = 2'-O-methyl adenosine
  modified_base 20: mod_base = OTHER; note = 2'-O-methyl uridine
  modified_base 21: mod_base = OTHER; note = 2'-O-methyl uridine
gcgtcaccaaaaagcgcaatt

SEQ ID NO: 39 - RNA, 21 nt, synthetic construct
  source 1..21: mol_type = other RNA
  modified_base 1: mod_base = OTHER; note = 2'-O-methyl guanosine
  modified_base 2: mod_base = OTHER; note = 2'-O-methyl cytidine 5'-thiophosphate
  modified_base 3: mod_base = OTHER; note = guanosine 5'-thiophosphate
  modified_base 20: mod_base = OTHER; note = 2'-O-methyl uridine
  modified_base 21: mod_base = OTHER; note = 2'-O-methyl uridine
gcgtcaccaaaaagcgcaatt

SEQ ID NO: 40 - RNA, 21 nt, synthetic construct
  source 1..21: mol_type = other RNA
  modified_base 1: mod_base = OTHER; note = 2'-O-methyl guanosine
  modified_base 2: mod_base = OTHER; note = 2'-O-methyl cytidine 5'-thiophosphate
  modified_base 3: mod_base = OTHER; note = 2'-O-methyl guanosine 5'-thiophosphate
  modified_base 4: mod_base = OTHER; note = uridine 5'-thiophosphate
  modified_base 19: mod_base = OTHER; note = 2'-O-methyl adenosine
  modified_base 20: mod_base = OTHER; note = 2'-O-methyl uridine
  modified_base 21: mod_base = OTHER; note = 2'-O-methyl uridine
gcgtcaccaaaaagcgcaatt

SEQ ID NO: 41 - RNA, 21 nt, synthetic construct
  source 1..21: mol_type = other RNA
  modified_base 1: mod_base = OTHER; note = 2'-O-methyl guanosine
  modified_base 2: mod_base = OTHER; note = 2'-O-methyl cytidine
  modified_base 3: mod_base = OTHER; note = 2'-O-methyl guanosine
  modified_base 4: mod_base = OTHER; note = 2'-O-methyl uridine
  modified_base 5: mod_base = OTHER; note = 2'-O-methyl cytidine
  modified_base 6: mod_base = OTHER; note = 2'-O-methyl adenosine
  modified_base 8: mod_base = OTHER; note = 2'-O-methyl cytidine
  modified_base 13: mod_base = OTHER; note = 2'-O-methyl adenosine
  modified_base 14: mod_base = OTHER; note = 2'-O-methyl guanosine
  modified_base 15: mod_base = OTHER; note = 2'-O-methyl cytidine
  modified_base 16: mod_base = OTHER; note = 2'-O-methyl guanosine
  modified_base 17: mod_base = OTHER; note = 2'-O-methyl cytidine
  modified_base 18: mod_base = OTHER; note = 2'-O-methyl adenosine
  modified_base 19: mod_base = OTHER; note = 2'-O-methyl adenosine
  modified_base 20: mod_base = OTHER; note = 2'-O-methyl uridine
  modified_base 21: mod_base = OTHER; note = 2'-O-methyl uridine
gcgtcaccaaaaagcgcaatt

SEQ ID NO: 42 - RNA, 21 nt, synthetic construct
  source 1..21: mol_type = other RNA
  modified_base 1: mod_base = OTHER; note = 2'-O-methyl guanosine
  modified_base 2: mod_base = OTHER; note = 2'-O-methyl cytidine 5'-thiophosphate
  modified_base 3: mod_base = OTHER; note = 2'-O-methyl guanosine 5'-thiophosphate
  modified_base 4: mod_base = OTHER; note = 2'-O-methyl uridine 5'-thiophosphate
  modified_base 18: mod_base = OTHER; note = 2'-O-methyl adenosine
  modified_base 19: mod_base = OTHER; note = 2'-O-methyl adenosine
  modified_base 20: mod_base = OTHER; note = 2'-O-methyl uridine
  modified_base 21: mod_base = OTHER; note = 2'-O-methyl uridine
gcgtcaccaaaaagcgcaatt

SEQ ID NO: 43 - RNA, 21 nt, synthetic construct
  source 1..21: mol_type = other RNA
  modified_base 1: mod_base = OTHER; note = 2'-O-methyl guanosine
  modified_base 2: mod_base = OTHER; note = 2'-O-methyl cytidine 5'-thiophosphate
  modified_base 3: mod_base = OTHER; note = 2'-O-methyl guanosine 5'-thiophosphate
  modified_base 4: mod_base = OTHER; note = 2'-O-methyl uridine 5'-thiophosphate
  modified_base 5: mod_base = OTHER; note = 2'-O-methyl cytidine
  modified_base 17: mod_base = OTHER; note = 2'-O-methyl cytidine
  modified_base 18: mod_base = OTHER; note = 2'-O-methyl adenosine
  modified_base 19: mod_base = OTHER; note = 2'-O-methyl adenosine
  modified_base 20: mod_base = OTHER; note = 2'-O-methyl uridine
  modified_base 21: mod_base = OTHER; note = 2'-O-methyl uridine
gcgtcaccaaaaagcgcaatt

SEQ ID NO: 44 - RNA, 21 nt, synthetic construct
  source 1..21: mol_type = other RNA
  modified_base 1: mod_base = OTHER; note = 2'-O-methyl guanosine
  modified_base 2: mod_base = OTHER; note = 2'-O-methyl cytidine 5'-thiophosphate
  modified_base 3: mod_base = OTHER; note = 2'-O-methyl guanosine 5'-thiophosphate
  modified_base 4: mod_base = OTHER; note = uridine 5'-thiophosphate
  modified_base 19: mod_base = OTHER; note = 2'-O-methyl adenosine
  modified_base 20: mod_base = OTHER; note = 2'-O-methyl uridine 5'-thiophosphate
  modified_base 21: mod_base = OTHER; note = 2'-O-methyl uridine 5'-thiophosphate
gcgtcaccaaaaagcgcaatt

SEQ ID NO: 45 - RNA, 21 nt, synthetic construct
  source 1..21: mol_type = other RNA
  modified_base 1: mod_base = OTHER; note = 2'-O-methyl guanosine
  modified_base 2: mod_base = OTHER; note = 2'-O-methyl cytidine 5'-thiophosphate
  modified_base 3: mod_base = OTHER; note = 2'-O-methyl guanosine 5'-thiophosphate
  modified_base 4: mod_base = OTHER; note = 2'-O-methyl uridine 5'-thiophosphate
  modified_base 5: mod_base = OTHER; note = 2'-O-methyl cytidine
  modified_base 6: mod_base = OTHER; note = 2'-O-methyl adenosine
  modified_base 8: mod_base = OTHER; note = 2'-O-methyl cytidine
  modified_base 12: mod_base = OTHER; note = 2'-O-methyl adenosine
  modified_base 14: mod_base = OTHER; note = 2'-O-methyl guanosine
  modified_base 16: mod_base = OTHER; note = 2'-O-methyl guanosine
  modified_base 17: mod_base = OTHER; note = 2'-O-methyl cytidine
  modified_base 18: mod_base = OTHER; note = 2'-O-methyl adenosine
  modified_base 19: mod_base = OTHER; note = 2'-O-methyl adenosine
  modified_base 20: mod_base = OTHER; note = 2'-O-methyl uridine 5'-thiophosphate
  modified_base 21: mod_base = OTHER; note = 2'-O-methyl uridine 5'-thiophosphate
gcgtcaccaaaaagcgcaatt

SEQ ID NO: 46 - RNA, 21 nt, synthetic construct
  source 1..21: mol_type = other RNA
  modified_base 1: mod_base = OTHER; note = 2'-O-methyl guanosine
  modified_base 2: mod_base = OTHER; note = 2'-O-methyl cytidine 5'-thiophosphate
  modified_base 3: mod_base = OTHER; note = 2'-O-methyl guanosine 5'-thiophosphate
  modified_base 4: mod_base = OTHER; note = 2'-O-methyl uridine 5'-thiophosphate
  modified_base 6: mod_base = OTHER; note = 2'-O-methyl adenosine
  modified_base 8: mod_base = OTHER; note = 2'-O-methyl cytidine
  modified_base 12: mod_base = OTHER; note = 2'-O-methyl adenosine
  modified_base 14: mod_base = OTHER; note = 2'-O-methyl guanosine
  modified_base 16: mod_base = OTHER; note = 2'-O-methyl guanosine
  modified_base 17: mod_base = OTHER; note = 2'-O-methyl cytidine
  modified_base 18: mod_base = OTHER; note = 2'-O-methyl adenosine
  modified_base 19: mod_base = OTHER; note = 2'-O-methyl adenosine
  modified_base 20: mod_base = OTHER; note = 2'-O-methyl uridine 5'-thiophosphate
  modified_base 21: mod_base = OTHER; note = 2'-O-methyl uridine 5'-thiophosphate
gcgtcaccaaaaagcgcaatt

SEQ ID NO: 47 - RNA, 21 nt, synthetic construct
  source 1..21: mol_type = other RNA
  modified_base 1: mod_base = OTHER; note = 2'-O-methyl guanosine
  modified_base 2: mod_base = OTHER; note = 2'-O-methyl cytidine 5'-thiophosphate
  modified_base 3: mod_base = OTHER; note = 2'-O-methyl guanosine 5'-thiophosphate
  modified_base 4: mod_base = OTHER; note = 2'-O-methyl uridine 5'-thiophosphate
  modified_base 6: mod_base = OTHER; note = 2'-O-methyl adenosine
  modified_base 8: mod_base = OTHER; note = 2'-O-methyl cytidine
  modified_base 12: mod_base = OTHER; note = 2'-O-methyl adenosine
  modified_base 14: mod_base = OTHER; note = 2'-O-methyl guanosine
  modified_base 16: mod_base = OTHER; note = 2'-O-methyl guanosine
  modified_base 17: mod_base = OTHER; note = 2'-O-methyl cytidine
  modified_base 18: mod_base = OTHER; note = 2'-O-methyl adenosine
  modified_base 19: mod_base = OTHER; note = 2'-O-methyl adenosine
  modified_base 20: mod_base = OTHER; note = 2'-O-methyl uridine 5'-thiophosphate
  modified_base 21: mod_base = OTHER; note = 2'-O-methyl uridine 5'-thiophosphate
  misc_feature 21: note = 3'-O attached to a GalNAc-comprising compound via a linker
gcgtcaccaaaaagcgcaatt

SEQ ID NO: 48 - RNA, 21 nt, synthetic construct
  source 1..21: mol_type = other RNA
  modified_base 1: mod_base = OTHER; note = 2'-O-methyl guanosine
  modified_base 2: mod_base = OTHER; note = 2'-O-methyl cytidine 5'-thiophosphate
  modified_base 3: mod_base = OTHER; note = 2'-O-methyl guanosine 5'-thiophosphate
  modified_base 4: mod_base = OTHER; note = 2'-O-methyl uridine 5'-thiophosphate
  modified_base 6: mod_base = OTHER; note = 2'-O-methyl adenosine
  modified_base 8: mod_base = OTHER; note = 2'-O-methyl cytidine
  modified_base 12: mod_base = OTHER; note = 2'-O-methyl adenosine
  modified_base 14: mod_base = OTHER; note = 2'-O-methyl guanosine
  modified_base 16: mod_base = OTHER; note = 2'-O-methyl guanosine
  modified_base 18: mod_base = OTHER; note = 2'-O-methyl adenosine
  modified_base 19: mod_base = OTHER; note = 2'-O-methyl adenosine
  modified_base 20: mod_base = OTHER; note = 2'-O-methyl uridine 5'-thiophosphate
  modified_base 21: mod_base = OTHER; note = 2'-O-methyl uridine 5'-thiophosphate
gcgtcaccaaaaagcgcaatt

SEQ ID NO: 49 - RNA, 21 nt, synthetic construct
  source 1..21: mol_type = other RNA
  modified_base 1: mod_base = OTHER; note = 2'-O-methyl guanosine
  modified_base 2: mod_base = OTHER; note = 2'-O-methyl cytidine 5'-thiophosphate
  modified_base 3: mod_base = OTHER; note = 2'-O-methyl guanosine 5'-thiophosphate
  modified_base 4: mod_base = OTHER; note = 2'-O-methyl uridine
  modified_base 6: mod_base = OTHER; note = 2'-O-methyl adenosine 5'-thiophosphate
  modified_base 8: mod_base = OTHER; note = 2'-O-methyl cytidine 5'-thiophosphate
  modified_base 12: mod_base = OTHER; note = 2'-O-methyl adenosine
  modified_base 14: mod_base = OTHER; note = 2'-O-methyl guanosine 5'-thiophosphate
  modified_base 16: mod_base = OTHER; note = 2'-O-methyl guanosine 5'-thiophosphate
  modified_base 17: mod_base = OTHER; note = 2'-O-methyl cytidine
  modified_base 18: mod_base = OTHER; note = 2'-O-methyl adenosine
  modified_base 19: mod_base = OTHER; note = 2'-O-methyl adenosine
  modified_base 20: mod_base = OTHER; note = 2'-O-methyl uridine 5'-thiophosphate
  modified_base 21: mod_base = OTHER; note = 2'-O-methyl uridine 5'-thiophosphate
gcgtcaccaaaaagcgcaatt

SEQ ID NO: 50 - RNA, 21 nt, synthetic construct
  source 1..21: mol_type = other RNA
  modified_base 1: mod_base = OTHER; note = 2'-O-methyl guanosine
  modified_base 2: mod_base = OTHER; note = 2'-O-methyl cytidine 5'-thiophosphate
  modified_base 3: mod_base = OTHER; note = 2'-O-methyl guanosine 5'-thiophosphate
  modified_base 4: mod_base = OTHER; note = 2'-O-methyl uridine
  modified_base 6: mod_base = OTHER; note = 2'-O-methyl adenosine 5'-thiophosphate
  modified_base 8: mod_base = OTHER; note = 2'-O-methyl cytidine 5'-thiophosphate
  modified_base 10: mod_base = OTHER; note = adenosine 5'-thiophosphate
  modified_base 11: mod_base = OTHER; note = adenosine 5'-thiophosphate
  modified_base 12: mod_base = OTHER; note = 2'-O-methyl adenosine 5'-thiophosphate
  modified_base 14: mod_base = OTHER; note = 2'-O-methyl guanosine 5'-thiophosphate
  modified_base 16: mod_base = OTHER; note = 2'-O-methyl guanosine 5'-thiophosphate
  modified_base 17: mod_base = OTHER; note = 2'-O-methyl cytidine
  modified_base 18: mod_base = OTHER; note = 2'-O-methyl adenosine
  modified_base 19: mod_base = OTHER; note = 2'-O-methyl adenosine
  modified_base 20: mod_base = OTHER; note = 2'-O-methyl uridine 5'-thiophosphate
  modified_base 21: mod_base = OTHER; note = 2'-O-methyl uridine 5'-thiophosphate
gcgtcaccaaaaagcgcaatt

SEQ ID NO: 51 - RNA, 21 nt, synthetic construct
  source 1..21: mol_type = other RNA
  modified_base 1: mod_base = OTHER; note = 2'-O-methyl guanosine
  modified_base 2: mod_base = OTHER; note = 2'-O-methyl cytidine 5'-thiophosphate
  modified_base 3: mod_base = OTHER; note = 2'-O-methyl guanosine 5'-thiophosphate
  modified_base 4: mod_base = OTHER; note = 2'-O-methyl uridine
  modified_base 6: mod_base = OTHER; note = 2'-O-methyl adenosine 5'-thiophosphate
  modified_base 8: mod_base = OTHER; note = 2'-O-methyl cytidine 5'-thiophosphate
  modified_base 9: mod_base = OTHER; note = 2'-fluoro adenosine
  modified_base 10: mod_base = OTHER; note = 2'-fluoro adenosine
  modified_base 11: mod_base = OTHER; note = 2'-O-methyl adenosine
  modified_base 12: mod_base = OTHER; note = 2'-O-methyl adenosine
  modified_base 14: mod_base = OTHER; note = 2'-O-methyl guanosine 5'-thiophosphate
  modified_base 16: mod_base = OTHER; note = 2'-O-methyl guanosine 5'-thiophosphate
  modified_base 17: mod_base = OTHER; note = 2'-O-methyl cytidine
  modified_base 18: mod_base = OTHER; note = 2'-O-methyl adenosine
  modified_base 19: mod_base = OTHER; note = 2'-O-methyl adenosine
  modified_base 20: mod_base = OTHER; note = 2'-O-methyl uridine 5'-thiophosphate
  modified_base 21: mod_base = OTHER; note = 2'-O-methyl uridine 5'-thiophosphate
gcgtcaccaaaaagcgcaatt

SEQ ID NO: 52 - RNA, 21 nt, synthetic construct
  source 1..21: mol_type = other RNA
  modified_base 1: mod_base = OTHER; note = 2'-O-methyl guanosine
  modified_base 2: mod_base = OTHER; note = 2'-O-methyl cytidine 5'-thiophosphate
  modified_base 3: mod_base = OTHER; note = 2'-O-methyl guanosine 5'-thiophosphate
  modified_base 4: mod_base = OTHER; note = 2'-O-methyl uridine
  modified_base 6: mod_base = OTHER; note = 2'-O-methyl adenosine 5'-thiophosphate
  modified_base 8: mod_base = OTHER; note = 2'-O-methyl cytidine 5'-thiophosphate
  modified_base 9: mod_base = OTHER; note = 2'-fluoro adenosine
  modified_base 10: mod_base = OTHER; note = 2'-fluoro adenosine
  modified_base 11: mod_base = OTHER; note = 2'-O-methyl adenosine
  modified_base 12: mod_base = OTHER; note = 2'-O-methyl adenosine
  modified_base 14: mod_base = OTHER; note = 2'-O-methyl guanosine 5'-thiophosphate
  modified_base 16: mod_base = OTHER; note = 2'-O-methyl guanosine 5'-thiophosphate
  modified_base 17: mod_base = OTHER; note = 2'-O-methyl cytidine
  modified_base 18: mod_base = OTHER; note = 2'-O-methyl adenosine
  modified_base 19: mod_base = OTHER; note = 2'-O-methyl adenosine
  modified_base 20: mod_base = OTHER; note = 2'-O-methyl uridine 5'-thiophosphate
  modified_base 21: mod_base = OTHER; note = 2'-O-methyl uridine 5'-thiophosphate
  misc_feature 21: note = 3'-O attached to a GalNAc-comprising compound via a linker
gcgtcaccaaaaagcgcaatt

SEQ ID NO: 53 - RNA, 21 nt, synthetic construct
  source 1..21: mol_type = other RNA
  modified_base 1: mod_base = OTHER; note = 2'-O-methyl guanosine
  modified_base 2: mod_base = OTHER; note = 2'-O-methyl cytidine 5'-thiophosphate
  modified_base 3: mod_base = OTHER; note = 2'-O-methyl guanosine 5'-thiophosphate
  modified_base 4: mod_base = OTHER; note = 2'-O-methyl uridine
  modified_base 6: mod_base = OTHER; note = 2'-O-methyl adenosine 5'-thiophosphate
  modified_base 8: mod_base = OTHER; note = 2'-O-methyl cytidine 5'-thiophosphate
  modified_base 9: mod_base = OTHER; note = 2'-fluoro adenosine
  modified_base 10: mod_base = OTHER; note = 2'-O-methyl adenosine
  modified_base 11: mod_base = OTHER; note = 2'-fluoro adenosine
  modified_base 12: mod_base = OTHER; note = 2'-O-methyl adenosine
  modified_base 14: mod_base = OTHER; note = 2'-O-methyl guanosine 5'-thiophosphate
  modified_base 16: mod_base = OTHER; note = 2'-O-methyl guanosine 5'-thiophosphate
  modified_base 17: mod_base = OTHER; note = 2'-O-methyl cytidine
  modified_base 18: mod_base = OTHER; note = 2'-O-methyl adenosine
  modified_base 19: mod_base = OTHER; note = 2'-O-methyl adenosine
  modified_base 20: mod_base = OTHER; note = 2'-O-methyl uridine 5'-thiophosphate
  modified_base 21: mod_base = OTHER; note = 2'-O-methyl uridine 5'-thiophosphate
gcgtcaccaaaaagcgcaatt

SEQ ID NO: 54 - RNA, 21 nt, synthetic construct
  source 1..21: mol_type = other RNA
  modified_base 1: mod_base = OTHER; note = 2'-O-methyl guanosine
  modified_base 2: mod_base = OTHER; note = 2'-O-methyl cytidine 5'-thiophosphate
  modified_base 3: mod_base = OTHER; note = 2'-O-methyl guanosine 5'-thiophosphate
  modified_base 4: mod_base = OTHER; note = 2'-O-methyl uridine
  modified_base 6: mod_base = OTHER; note = 2'-O-methyl adenosine 5'-thiophosphate
  modified_base 8: mod_base = OTHER; note = 2'-O-methyl cytidine 5'-thiophosphate
  modified_base 9: mod_base = OTHER; note = 2'-fluoro adenosine
  modified_base 11: mod_base = OTHER; note = adenosine 5'-thiophosphate
  modified_base 12: mod_base = OTHER; note = 2'-O-methyl adenosine 5'-thiophosphate
  modified_base 14: mod_base = OTHER; note = 2'-O-methyl guanosine 5'-thiophosphate
  modified_base 16: mod_base = OTHER; note = 2'-O-methyl guanosine 5'-thiophosphate
  modified_base 17: mod_base = OTHER; note = 2'-O-methyl cytidine
  modified_base 18: mod_base = OTHER; note = 2'-O-methyl adenosine
  modified_base 19: mod_base = OTHER; note = 2'-O-methyl adenosine
  modified_base 20: mod_base = OTHER; note = 2'-O-methyl uridine 5'-thiophosphate
  modified_base 21: mod_base = OTHER; note = 2'-O-methyl uridine 5'-thiophosphate
gcgtcaccaaaaagcgcaatt

SEQ ID NO: 55 - RNA, 21 nt, synthetic construct
  source 1..21: mol_type = other RNA
  modified_base 1: mod_base = OTHER; note = 2'-O-methyl guanosine
  modified_base 2: mod_base = OTHER; note = 2'-O-methyl cytidine 5'-thiophosphate
  modified_base 3: mod_base = OTHER; note = 2'-O-methyl guanosine 5'-thiophosphate
  modified_base 4: mod_base = OTHER; note = 2'-O-methyl uridine
  modified_base 6: mod_base = OTHER; note = 2'-O-methyl adenosine 5'-thiophosphate
  modified_base 8: mod_base = OTHER; note = 2'-O-methyl cytidine 5'-thiophosphate
  modified_base 9: mod_base = OTHER; note = 2'-fluoro adenosine
  modified_base 11: mod_base = OTHER; note = 2'-O-methyl adenosine 5'-thiophosphate
  modified_base 12: mod_base = OTHER; note = 2'-O-methyl adenosine
  modified_base 14: mod_base = OTHER; note = 2'-O-methyl guanosine 5'-thiophosphate
  modified_base 16: mod_base = OTHER; note = 2'-O-methyl guanosine 5'-thiophosphate
  modified_base 17: mod_base = OTHER; note = 2'-O-methyl cytidine
  modified_base 18: mod_base = OTHER; note = 2'-O-methyl adenosine
  modified_base 19: mod_base = OTHER; note = 2'-O-methyl adenosine
  modified_base 20: mod_base = OTHER; note = 2'-O-methyl uridine 5'-thiophosphate
  modified_base 21: mod_base = OTHER; note = 2'-O-methyl uridine 5'-thiophosphate
gcgtcaccaaaaagcgcaatt

SEQ ID NO: 56 - RNA, 21 nt, synthetic construct
  source 1..21: mol_type = other RNA
  modified_base 1: mod_base = OTHER; note = 2'-O-methyl guanosine
  modified_base 2: mod_base = OTHER; note = 2'-O-methyl cytidine 5'-thiophosphate
  modified_base 3: mod_base = OTHER; note = 2'-O-methyl guanosine 5'-thiophosphate
  modified_base 4: mod_base = OTHER; note = 2'-O-methyl uridine
  modified_base 6: mod_base = OTHER; note = 2'-O-methyl adenosine 5'-thiophosphate
  modified_base 8: mod_base = OTHER; note = 2'-O-methyl cytidine 5'-thiophosphate
  modified_base 9: mod_base = OTHER; note = 2'-fluoro adenosine
  modified_base 10: mod_base = OTHER; note = 2'-fluoro adenosine
  modified_base 12: mod_base = OTHER; note = 2'-O-methyl adenosine 5'-thiophosphate
  modified_base 14: mod_base = OTHER; note = 2'-O-methyl guanosine 5'-thiophosphate
  modified_base 16: mod_base = OTHER; note = 2'-O-methyl guanosine 5'-thiophosphate
  modified_base 17: mod_base = OTHER; note = 2'-O-methyl cytidine
  modified_base 18: mod_base = OTHER; note = 2'-O-methyl adenosine
  modified_base 19: mod_base = OTHER; note = 2'-O-methyl adenosine
  modified_base 20: mod_base = OTHER; note = 2'-O-methyl uridine 5'-thiophosphate
  modified_base 21: mod_base = OTHER; note = 2'-O-methyl uridine 5'-thiophosphate
gcgtcaccaaaaagcgcaatt

SEQ ID NO: 57 - RNA, 21 nt, synthetic construct
  source 1..21: mol_type = other RNA
  modified_base 1: mod_base = OTHER; note = 2'-O-methyl uridine
  modified_base 2: mod_base = OTHER; note = 2'-fluoro uridine 5'-thiophosphate
  modified_base 3: mod_base = OTHER; note = 2'-O-methyl guanosine 5'-thiophosphate
  modified_base 4: mod_base = OTHER; note = 2'-O-methyl cytidine
  modified_base 5: mod_base = OTHER; note = 2'-O-methyl guanosine
  modified_base 6: mod_base = OTHER; note = 2'-fluoro cytidine
  modified_base 7: mod_base = OTHER; note = 2'-O-methyl uridine
  modified_base 8: mod_base = OTHER; note = 2'-fluoro uridine
  modified_base 9: mod_base = OTHER; note = 2'-fluoro uridine
  modified_base 10: mod_base = OTHER; note = 2'-O-methyl uridine
  modified_base 11: mod_base = OTHER; note = 2'-O-methyl uridine
  modified_base 12: mod_base = OTHER; note = 2'-O-methyl guanosine
  modified_base 13: mod_base = OTHER; note = 2'-O-methyl guanosine
  modified_base 14: mod_base = OTHER; note = 2'-fluoro uridine
  modified_base 15: mod_base = OTHER; note = 2'-O-methyl guanosine
  modified_base 16: mod_base = OTHER; note = 2'-deoxy adenosine 5'-thiophosphate
  modified_base 17: mod_base = OTHER; note = 2'-O-methyl cytidine
  modified_base 18: mod_base = OTHER; note = 2'-O-methyl guanosine
  modified_base 19: mod_base = OTHER; note = 2'-O-methyl cytidine
  modified_base 20: mod_base = OTHER; note = 2'-O-methyl uridine 5'-thiophosphate
  modified_base 21: mod_base = OTHER; note = 2'-O-methyl uridine 5'-thiophosphate
ttgcgctttttggtgacgctt

SEQ ID NO: 58 - RNA, 21 nt, synthetic construct
  source 1..21: mol_type = other RNA
  modified_base 1: mod_base = OTHER; note = 2'-O-methyl uridine
  modified_base 2: mod_base = OTHER; note = 2'-fluoro uridine 5'-thiophosphate
  modified_base 3: mod_base = OTHER; note = 2'-O-methyl guanosine 5'-thiophosphate
  modified_base 4: mod_base = OTHER; note = 2'-fluoro cytidine
  modified_base 5: mod_base = OTHER; note = 2'-O-methyl guanosine
  modified_base 6: mod_base = OTHER; note = 2'-fluoro cytidine
  modified_base 7: mod_base = OTHER; note = 2'-O-methyl uridine
  modified_base 8: mod_base = OTHER; note = 2'-O-methyl uridine
  modified_base 9: mod_base = OTHER; note = 2'-fluoro uridine
  modified_base 10: mod_base = OTHER; note = 2'-O-methyl uridine
  modified_base 11: mod_base = OTHER; note = 2'-O-methyl uridine
  modified_base 12: mod_base = OTHER; note = 2'-fluoro guanosine
  modified_base 13: mod_base = OTHER; note = 2'-O-methyl guanosine
  modified_base 14: mod_base = OTHER; note = 2'-fluoro uridine
  modified_base 15: mod_base = OTHER; note = 2'-O-methyl guanosine
  modified_base 16: mod_base = OTHER; note = 2'-fluoro adenosine
  modified_base 17: mod_base = OTHER; note = 2'-O-methyl cytidine
  modified_base 18: mod_base = OTHER; note = 2'-O-methyl guanosine
  modified_base 19: mod_base = OTHER; note = 2'-fluoro cytidine
  modified_base 20: mod_base = OTHER; note = 2'-O-methyl uridine
  modified_base 21: mod_base = OTHER; note = 2'-O-methyl uridine 5'-thiophosphate
ttgcgctttttggtgacgctt

SEQ ID NO: 59 - RNA, 21 nt, synthetic construct
  source 1..21: mol_type = other RNA
  modified_base 1: mod_base = OTHER; note = 2'-O-methyl uridine
  modified_base 2: mod_base = OTHER; note = 2'-deoxy thymidine 5'-thiophosphate
  modified_base 3: mod_base = OTHER; note = 2'-O-methyl guanosine 5'-thiophosphate
  modified_base 4: mod_base = OTHER; note = 2'-O-methyl cytidine
  modified_base 5: mod_base = OTHER; note = 2'-O-methyl guanosine
  modified_base 6: mod_base = OTHER; note = 2'-fluoro cytidine
  modified_base 7: mod_base = OTHER; note = 2'-O-methyl uridine
  modified_base 8: mod_base = OTHER; note = 2'-fluoro uridine
  modified_base 9: mod_base = OTHER; note = 2'-fluoro uridine
  modified_base 10: mod_base = OTHER; note = 2'-O-methyl uridine
  modified_base 11: mod_base = OTHER; note = 2'-O-methyl uridine
  modified_base 12: mod_base = OTHER; note = 2'-O-methyl guanosine
  modified_base 13: mod_base = OTHER; note = 2'-O-methyl guanosine
  modified_base 14: mod_base = OTHER; note = 2'-fluoro uridine
  modified_base 15: mod_base = OTHER; note = 2'-O-methyl guanosine
  modified_base 16: mod_base = OTHER; note = 2'-fluoro adenosine
  modified_base 17: mod_base = OTHER; note = 2'-O-methyl cytidine
  modified_base 18: mod_base = OTHER; note = 2'-O-methyl guanosine
  modified_base 19: mod_base = OTHER; note = 2'-O-methyl cytidine
  modified_base 20: mod_base = OTHER; note = 2'-O-methyl uridine 5'-thiophosphate
  modified_base 21: mod_base = OTHER; note = 2'-O-methyl uridine 5'-thiophosphate
ttgcgctttttggtgacgctt

SEQ ID NO: 60 - RNA, 21 nt, synthetic construct
  source 1..21: mol_type = other RNA
  modified_base 1: mod_base = OTHER; note = 2'-O-methyl uridine
  modified_base 2: mod_base = OTHER; note = 2'-deoxy thymidine 5'-thiophosphate
  modified_base 3: mod_base = OTHER; note = 2'-O-methyl guanosine 5'-thiophosphate
  modified_base 4: mod_base = OTHER; note = 2'-fluoro cytidine
  modified_base 5: mod_base = OTHER; note = 2'-O-methyl guanosine
  modified_base 6: mod_base = OTHER; note = 2'-fluoro cytidine
  modified_base 7: mod_base = OTHER; note = 2'-O-methyl uridine
  modified_base 8: mod_base = OTHER; note = 2'-O-methyl uridine
  modified_base 9: mod_base = OTHER; note = 2'-fluoro uridine
  modified_base 10: mod_base = OTHER; note = 2'-O-methyl uridine
  modified_base 11: mod_base = OTHER; note = 2'-O-methyl uridine
  modified_base 12: mod_base = OTHER; note = 2'-fluoro guanosine
  modified_base 13: mod_base = OTHER; note = 2'-O-methyl guanosine
  modified_base 14: mod_base = OTHER; note = 2'-fluoro uridine
  modified_base 15: mod_base = OTHER; note = 2'-O-methyl guanosine
  modified_base 16: mod_base = OTHER; note = 2'-fluoro adenosine
  modified_base 17: mod_base = OTHER; note = 2'-O-methyl cytidine
  modified_base 18: mod_base = OTHER; note = 2'-O-methyl guanosine
  modified_base 19: mod_base = OTHER; note = 2'-fluoro cytidine
  modified_base 20: mod_base = OTHER; note = 2'-O-methyl uridine 5'-thiophosphate
  modified_base 21: mod_base = OTHER; note = 2'-O-methyl uridine 5'-thiophosphate
ttgcgctttttggtgacgctt

SEQ ID NO: 61 - RNA, 21 nt, synthetic construct
  source 1..21: mol_type = other RNA
  modified_base 1: mod_base = OTHER; note = 2'-O-methyl uridine
  modified_base 2: mod_base = OTHER; note = 2'-deoxy thymidine 5'-thiophosphate
  modified_base 3: mod_base = OTHER; note = 2'-O-methyl guanosine 5'-thiophosphate
  modified_base 4: mod_base = OTHER; note = 2'-O-methyl cytidine
  modified_base 5: mod_base = OTHER; note = 2'-O-methyl guanosine
  modified_base 6: mod_base = OTHER; note = 2'-fluoro cytidine
  modified_base 7: mod_base = OTHER; note = 2'-deoxy thymidine 5'-thiophosphate
  modified_base 8: mod_base = OTHER; note = 2'-fluoro uridine
  modified_base 9: mod_base = OTHER; note = 2'-fluoro uridine
  modified_base 10: mod_base = OTHER; note = 2'-O-methyl uridine
  modified_base 11: mod_base = OTHER; note = 2'-O-methyl uridine
  modified_base 12: mod_base = OTHER; note = 2'-O-methyl guanosine
  modified_base 13: mod_base = OTHER; note = 2'-O-methyl guanosine
  modified_base 14: mod_base = OTHER; note = 2'-fluoro uridine
  modified_base 15: mod_base = OTHER; note = 2'-O-methyl guanosine
  modified_base 16: mod_base = OTHER; note = 2'-fluoro adenosine
  modified_base 17: mod_base = OTHER; note = 2'-O-methyl cytidine
  modified_base 18: mod_base = OTHER; note = 2'-O-methyl guanosine
  modified_base 19: mod_base = OTHER; note = 2'-O-methyl cytidine
  modified_base 20: mod_base = OTHER; note = 2'-O-methyl uridine 5'-thiophosphate
  modified_base 21: mod_base = OTHER; note = 2'-O-methyl uridine 5'-thiophosphate
ttgcgctttttggtgacgctt

SEQ ID NO: 62 - RNA, 21 nt, synthetic construct
  source 1..21: mol_type = other RNA
  modified_base 1: mod_base = OTHER; note = 2'-O-methyl uridine
  modified_base 2: mod_base = OTHER; note = 2'-deoxy thymidine 5'-thiophosphate
  modified_base 3: mod_base = OTHER; note = 2'-O-methyl guanosine 5'-thiophosphate
  modified_base 4: mod_base = OTHER; note = 2'-O-methyl cytidine
  modified_base 5: mod_base = OTHER; note = 2'-O-methyl guanosine
  modified_base 6: mod_base = OTHER; note = 2'-fluoro cytidine
  modified_base 7: mod_base = OTHER; note = 2'-deoxy thymidine 5'-thiophosphate
  modified_base 8: mod_base = OTHER; note = 2'-O-methyl uridine
  modified_base 9: mod_base = OTHER; note = 2'-fluoro uridine
  modified_base 10: mod_base = OTHER; note = 2'-O-methyl uridine
  modified_base 11: mod_base = OTHER; note = 2'-O-methyl uridine
  modified_base 12: mod_base = OTHER; note = 2'-O-methyl guanosine
  modified_base 13: mod_base = OTHER; note = 2'-O-methyl guanosine
  modified_base 14: mod_base = OTHER; note = 2'-fluoro uridine
  modified_base 15: mod_base = OTHER; note = 2'-O-methyl guanosine
  modified_base 16: mod_base = OTHER; note = 2'-fluoro adenosine
  modified_base 17: mod_base = OTHER; note = 2'-O-methyl cytidine
  modified_base 18: mod_base = OTHER; note = 2'-O-methyl guanosine
  modified_base 19: mod_base = OTHER; note = 2'-O-methyl cytidine
  modified_base 20: mod_base = OTHER; note = 2'-O-methyl uridine 5'-thiophosphate
  modified_base 21: mod_base = OTHER; note = 2'-O-methyl uridine 5'-thiophosphate
ttgcgctttttggtgacgctt

SEQ ID NO: 63 - RNA, 21 nt, synthetic construct
  source 1..21: mol_type = other RNA
  modified_base 1: mod_base = OTHER; note = 2'-O-methyl uridine
  modified_base 2: mod_base = OTHER; note = 2'-deoxy thymidine 5'-thiophosphate
  modified_base 3: mod_base = OTHER; note = 2'-O-methyl guanosine 5'-thiophosphate
  modified_base 4: mod_base = OTHER; note = 2'-O-methyl cytidine
  modified_base 5: mod_base = OTHER; note = 2'-O-methyl guanosine
  modified_base 6: mod_base = OTHER; note = 2'-fluoro cytidine
  modified_base 7: mod_base = OTHER; note = 2'-deoxy thymidine 5'-thiophosphate
  modified_base 8: mod_base = OTHER; note = 2'-O-methyl uridine
  modified_base 9: mod_base = OTHER; note = 2'-fluoro uridine
  modified_base 10: mod_base = OTHER; note = 2'-O-methyl uridine
  modified_base 11: mod_base = OTHER; note = 2'-O-methyl uridine
  modified_base 12: mod_base = OTHER; note = 2'-O-methyl guanosine
  modified_base 13: mod_base = OTHER; note = 2'-O-methyl guanosine
  modified_base 14: mod_base = OTHER; note = 2'-fluoro uridine
  modified_base 15: mod_base = OTHER; note = 2'-O-methyl guanosine
  modified_base 16: mod_base = OTHER; note = 2'-deoxy adenosine 5'-thiophosphate
  modified_base 17: mod_base = OTHER; note = 2'-O-methyl cytidine
  modified_base 18: mod_base = OTHER; note = 2'-O-methyl guanosine
  modified_base 19: mod_base = OTHER; note = 2'-O-methyl cytidine
  modified_base 20: mod_base = OTHER; note = 2'-O-methyl uridine 5'-thiophosphate
  modified_base 21: mod_base = OTHER; note = 2'-O-methyl uridine 5'-thiophosphate
ttgcgctttttggtgacgctt

SEQ ID NO: 64 - RNA, 21 nt, synthetic construct
  source 1..21: mol_type = other RNA
  modified_base 1: mod_base = OTHER; note = 2'-O-methyl uridine
  modified_base 2: mod_base = OTHER; note = 2'-deoxy thymidine 5'-thiophosphate
  modified_base 3: mod_base = OTHER; note = 2'-O-methyl guanosine 5'-thiophosphate
  modified_base 4: mod_base = OTHER; note = 2'-O-methyl cytidine
  modified_base 5: mod_base = OTHER; note = 2'-O-methyl guanosine
  modified_base 6: mod_base = OTHER; note = 2'-fluoro cytidine
  modified_base 7: mod_base = OTHER; note = 2'-deoxy thymidine
  modified_base 8: mod_base = OTHER; note = 2'-O-methyl uridine 5'-thiophosphate
  modified_base 9: mod_base = OTHER; note = 2'-fluoro uridine
  modified_base 10: mod_base = OTHER; note = 2'-O-methyl uridine
  modified_base 11: mod_base = OTHER; note = 2'-O-methyl uridine
  modified_base 12: mod_base = OTHER; note = 2'-O-methyl guanosine
  modified_base 13: mod_base = OTHER; note = 2'-O-methyl guanosine
  modified_base 14: mod_base = OTHER; note = 2'-fluoro uridine
  modified_base 15: mod_base = OTHER; note = 2'-O-methyl guanosine
  modified_base 16: mod_base = OTHER; note = 2'-fluoro adenosine
  modified_base 17: mod_base = OTHER; note = 2'-O-methyl cytidine
  modified_base 18: mod_base = OTHER; note = 2'-O-methyl guanosine
  modified_base 19: mod_base = OTHER; note = 2'-O-methyl cytidine
  modified_base 20: mod_base = OTHER; note = 2'-O-methyl uridine 5'-thiophosphate
  modified_base 21: mod_base = OTHER; note = 2'-O-methyl uridine 5'-thiophosphate
ttgcgctttttggtgacgctt

SEQ ID NO: 65 - RNA, 21 nt, synthetic construct
  source 1..21: mol_type = other RNA
  modified_base 1: mod_base = OTHER; note = 2'-O-methyl uridine
  modified_base 2: mod_base = OTHER; note = 2'-deoxy thymidine 5'-thiophosphate
  modified_base 3: mod_base = OTHER; note = 2'-O-methyl guanosine 5'-thiophosphate
  modified_base 4: mod_base = OTHER; note = 2'-O-methyl cytidine
  modified_base 5: mod_base = OTHER; note = 2'-O-methyl guanosine
  modified_base 6: mod_base = OTHER; note = 2'-fluoro cytidine
  modified_base 7: mod_base = OTHER; note = 2'-deoxy thymidine
  modified_base 8: mod_base = OTHER; note = 2'-O-methyl uridine 5'-thiophosphate
  modified_base 9: mod_base = OTHER; note = 2'-fluoro uridine
  modified_base 10: mod_base = OTHER; note = 2'-O-methyl uridine
  modified_base 11: mod_base = OTHER; note = 2'-O-methyl uridine
  modified_base 12: mod_base = OTHER; note = 2'-fluoro guanosine
  modified_base 13: mod_base = OTHER; note = 2'-O-methyl guanosine
  modified_base 14: mod_base = OTHER; note = 2'-fluoro uridine
  modified_base 15: mod_base = OTHER; note = 2'-O-methyl guanosine
  modified_base 16: mod_base = OTHER; note = 2'-fluoro adenosine
  modified_base 17: mod_base = OTHER; note = 2'-O-methyl cytidine
  modified_base 18: mod_base = OTHER; note = 2'-O-methyl guanosine
  modified_base 19: mod_base = OTHER; note = 2'-deoxy cytidine
  modified_base 20: mod_base = OTHER; note = 2'-O-methyl uridine 5'-thiophosphate
  modified_base 21: mod_base = OTHER; note = 2'-O-methyl uridine 5'-thiophosphate
ttgcgctttttggtgacgctt

SEQ ID NO: 66 - RNA, 21 nt, synthetic construct
  source 1..21: mol_type = other RNA
  modified_base 1: mod_base = OTHER; note = 2'-O-methyl uridine
  modified_base 2: mod_base = OTHER; note = 2'-deoxy thymidine 5'-thiophosphate
  modified_base 3: mod_base = OTHER; note = 2'-O-methyl guanosine 5'-thiophosphate
  modified_base 4: mod_base = OTHER; note = 2'-O-methyl cytidine
  modified_base 5: mod_base = OTHER; note = 2'-O-methyl guanosine
  modified_base 6: mod_base = OTHER; note = 2'-fluoro cytidine
  modified_base 7: mod_base = OTHER; note = 2'-deoxy thymidine
  modified_base 8: mod_base = OTHER; note = 2'-O-methyl uridine 5'-thiophosphate
  modified_base 9: mod_base = OTHER; note = 2'-fluoro uridine
  modified_base 10: mod_base = OTHER; note = 2'-O-methyl uridine
  modified_base 11: mod_base = OTHER; note = 2'-O-methyl uridine
  modified_base 12: mod_base = OTHER; note = 2'-deoxy guanosine
  modified_base 13: mod_base = OTHER; note = 2'-O-methyl guanosine 5'-thiophosphate
  modified_base 14: mod_base = OTHER; note = 2'-fluoro uridine
  modified_base 15: mod_base = OTHER; note = 2'-O-methyl guanosine
  modified_base 16: mod_base = OTHER; note = 2'-fluoro adenosine
  modified_base 17: mod_base = OTHER; note = 2'-O-methyl cytidine
  modified_base 18: mod_base = OTHER; note = 2'-O-methyl guanosine
  modified_base 19: mod_base = OTHER; note = 2'-deoxy cytidine
  modified_base 20: mod_base = OTHER; note = 2'-O-methyl uridine 5'-thiophosphate
  modified_base 21: mod_base = OTHER; note = 2'-O-methyl uridine 5'-thiophosphate
ttgcgctttttggtgacgctt

SEQ ID NO: 67 - RNA, 21 nt, synthetic construct
  source 1..21: mol_type = other RNA
  modified_base 1: mod_base = OTHER; note = 2'-O-methyl uridine
  modified_base 2: mod_base = OTHER; note = 2'-deoxy thymidine 5'-thiophosphate
  modified_base 3: mod_base = OTHER; note = 2'-O-methyl guanosine 5'-thiophosphate
  modified_base 4: mod_base = OTHER; note = 2'-fluoro cytidine
  modified_base 5: mod_base = OTHER; note = 2'-O-methyl guanosine
  modified_base 6: mod_base = OTHER; note = 2'-fluoro cytidine
  modified_base 7: mod_base = OTHER; note = 2'-deoxy thymidine
  modified_base 8: mod_base = OTHER; note = 2'-O-methyl uridine 5'-thiophosphate
  modified_base 9: mod_base = OTHER; note = 2'-fluoro uridine
  modified_base 10: mod_base = OTHER; note = 2'-O-methyl uridine
  modified_base 11: mod_base = OTHER; note = 2'-O-methyl uridine
  modified_base 12: mod_base = OTHER; note = 2'-fluoro guanosine
  modified_base 13: mod_base = OTHER; note = 2'-O-methyl guanosine
  modified_base 14: mod_base = OTHER; note = 2'-fluoro uridine
  modified_base 15: mod_base = OTHER; note = 2'-O-methyl guanosine
  modified_base 16: mod_base = OTHER; note = 2'-fluoro adenosine
  modified_base 17: mod_base = OTHER; note = 2'-O-methyl cytidine
  modified_base 18: mod_base = OTHER; note = 2'-O-methyl guanosine
  modified_base 19: mod_base = OTHER; note = 2'-deoxy cytidine
  modified_base 20: mod_base = OTHER; note = 2'-O-methyl uridine 5'-thiophosphate
  modified_base 21: mod_base = OTHER; note = 2'-O-methyl uridine 5'-thiophosphate
ttgcgctttttggtgacgctt

SEQ ID NO: 68 - RNA, 21 nt, synthetic construct
  source 1..21: mol_type = other RNA
  modified_base 1: mod_base = OTHER; note = 2'-O-methyl uridine
  modified_base 2: mod_base = OTHER; note = 2'-deoxy thymidine 5'-thiophosphate
  modified_base 3: mod_base = OTHER; note = 2'-O-methyl guanosine 5'-thiophosphate
  modified_base 4: mod_base = OTHER; note = 2'-deoxy cytidine
  modified_base 5: mod_base = OTHER; note = 2'-O-methyl guanosine 5'-thiophosphate
  modified_base 6: mod_base = OTHER; note = 2'-fluoro cytidine
  modified_base 7: mod_base = OTHER; note = 2'-deoxy thymidine
  modified_base 8: mod_base = OTHER; note = 2'-O-methyl uridine 5'-thiophosphate
  modified_base 9: mod_base = OTHER; note = 2'-fluoro uridine
  modified_base 10: mod_base = OTHER; note = 2'-O-methyl uridine
  modified_base 11: mod_base = OTHER; note = 2'-O-methyl uridine
  modified_base 12: mod_base = OTHER; note = 2'-deoxy guanosine
  modified_base 13: mod_base = OTHER; note = 2'-O-methyl guanosine 5'-thiophosphate
  modified_base 14: mod_base = OTHER; note = 2'-fluoro uridine
  modified_base 15: mod_base = OTHER; note = 2'-O-methyl guanosine
  modified_base 16: mod_base = OTHER; note = 2'-fluoro adenosine
  modified_base 17: mod_base = OTHER; note = 2'-O-methyl cytidine
  modified_base 18: mod_base = OTHER; note = 2'-O-methyl guanosine
  modified_base 19: mod_base = OTHER; note = 2'-deoxy cytidine
  modified_base 20: mod_base = OTHER; note = 2'-O-methyl uridine 5'-thiophosphate
  modified_base 21: mod_base = OTHER; note = 2'-O-methyl uridine 5'-thiophosphate
ttgcgctttttggtgacgctt

SEQ ID NO: 69 - RNA, 21 nt, synthetic construct
  source 1..21: mol_type = other RNA
  modified_base 1: mod_base = OTHER; note = 2'-O-methyl uridine
  modified_base 2: mod_base = OTHER; note = 2'-deoxy thymidine 5'-thiophosphate
  modified_base 3: mod_base = OTHER; note = 2'-O-methyl guanosine 5'-thiophosphate
  modified_base 4: mod_base = OTHER; note = 2'-deoxy cytidine
  modified_base 5: mod_base = OTHER; note = 2'-O-methyl guanosine 5'-thiophosphate
  modified_base 6: mod_base = OTHER; note = 2'-fluoro cytidine
  modified_base 7: mod_base = OTHER; note = 2'-deoxy thymidine
  modified_base 8: mod_base = OTHER; note = 2'-O-methyl uridine 5'-thiophosphate
  modified_base 9: mod_base = OTHER; note = 2'-fluoro uridine
  modified_base 10: mod_base = OTHER; note = 2'-O-methyl uridine
  modified_base 11: mod_base = OTHER; note = 2'-O-methyl uridine
  modified_base 12: mod_base = OTHER; note = 2'-fluoro guanosine
  modified_base 13: mod_base = OTHER; note = 2'-O-methyl guanosine
  modified_base 14: mod_base = OTHER; note = 2'-fluoro uridine
  modified_base 15: mod_base = OTHER; note = 2'-O-methyl guanosine
  modified_base 16: mod_base = OTHER; note = 2'-fluoro adenosine
  modified_base 17: mod_base = OTHER; note = 2'-O-methyl cytidine
  modified_base 18: mod_base = OTHER; note = 2'-O-methyl guanosine
  modified_base 19: mod_base = OTHER; note = 2'-deoxy cytidine
  modified_base 20: mod_base = OTHER; note = 2'-O-methyl uridine 5'-thiophosphate
  modified_base 21: mod_base = OTHER; note = 2'-O-methyl uridine 5'-thiophosphate
ttgcgctttttggtgacgctt

SEQ ID NO: 70 - RNA, 21 nt, synthetic construct
  source 1..21: mol_type = other RNA
  modified_base 1: mod_base = OTHER; note = 2'-O-methyl uridine
  modified_base 2: mod_base = OTHER; note = 2'-deoxy thymidine 5'-thiophosphate
  modified_base 3: mod_base = OTHER; note = 2'-O-methyl guanosine 5'-thiophosphate
  modified_base 4: mod_base = OTHER; note = 2'-fluoro cytidine
  modified_base 5: mod_base = OTHER; note = 2'-O-methyl guanosine
  modified_base 6: mod_base = OTHER; note = 2'-fluoro cytidine
  modified_base 7: mod_base = OTHER; note = 2'-deoxy thymidine
  modified_base 8: mod_base = OTHER; note = 2'-O-methyl uridine 5'-thiophosphate
  modified_base 9: mod_base = OTHER; note = 2'-fluoro uridine
  modified_base 10: mod_base = OTHER; note = 2'-O-methyl uridine
  modified_base 11: mod_base = OTHER; note = 2'-O-methyl uridine
  modified_base 12: mod_base = OTHER; note = 2'-fluoro guanosine
  modified_base 13: mod_base = OTHER; note = 2'-O-methyl guanosine
  modified_base 14: mod_base = OTHER; note = 2'-fluoro uridine
  modified_base 15: mod_base = OTHER; note = 2'-O-methyl guanosine
  modified_base 16: mod_base = OTHER; note = 2'-fluoro adenosine
  modified_base 17: mod_base = OTHER; note = 2'-O-methyl cytidine
  modified_base 18: mod_base = OTHER; note = 2'-O-methyl guanosine
  modified_base 19: mod_base = OTHER; note = 2'-fluoro cytidine
  modified_base 20: mod_base = OTHER; note = 2'-O-methyl uridine
  modified_base 21: mod_base = OTHER; note = 2'-O-methyl uridine 5'-thiophosphate
ttgcgctttttggtgacgctt

SEQ ID NO: 71 - RNA, 21 nt, synthetic construct
  source 1..21: mol_type = other RNA
  modified_base 1: mod_base = OTHER; note = 2'-O-methyl uridine
  modified_base 2: mod_base = OTHER; note = 2'-fluoro uridine 5'-thiophosphate
  modified_base 3: mod_base = OTHER; note = 2'-O-methyl guanosine 5'-thiophosphate
  modified_base 4: mod_base = OTHER; note = 2'-O-methyl cytidine
  modified_base 5: mod_base = OTHER; note = 2'-O-methyl guanosine
  modified_base 6: mod_base = OTHER; note = 2'-fluoro cytidine
  modified_base 7: mod_base = OTHER; note = 2'-deoxy thymidine 5'-thiophosphate
  modified_base 8: mod_base = OTHER; note = 2'-fluoro uridine
  modified_base 9: mod_base = OTHER; note = 2'-fluoro uridine
  modified_base 10: mod_base = OTHER; note = 2'-O-methyl uridine
  modified_base 11: mod_base = OTHER; note = 2'-O-methyl uridine
  modified_base 12: mod_base = OTHER; note = 2'-O-methyl guanosine
  modified_base 13: mod_base = OTHER; note = 2'-O-methyl guanosine
  modified_base 14: mod_base = OTHER; note = 2'-fluoro uridine
  modified_base 15: mod_base = OTHER; note = 2'-O-methyl guanosine
  modified_base 16: mod_base = OTHER; note = 2'-fluoro adenosine
  modified_base 17: mod_base = OTHER; note = 2'-O-methyl cytidine
  modified_base 18: mod_base = OTHER; note = 2'-O-methyl guanosine
  modified_base 19: mod_base = OTHER; note = 2'-O-methyl cytidine
  modified_base 20: mod_base = OTHER; note = 2'-O-methyl uridine 5'-thiophosphate
  modified_base 21: mod_base = OTHER; note = 2'-O-methyl uridine 5'-thiophosphate
ttgcgctttttggtgacgctt

SEQ ID NO: 72 - RNA, 21 nt, synthetic construct
  source 1..21: mol_type = other RNA
  modified_base 1: mod_base = OTHER; note = 2'-O-methyl uridine
  modified_base 2: mod_base = OTHER; note = 2'-fluoro uridine 5'-thiophosphate
  modified_base 3: mod_base = OTHER; note = 2'-O-methyl guanosine 5'-thiophosphate
  modified_base 4: mod_base = OTHER; note = 2'-O-methyl cytidine
  modified_base 5: mod_base = OTHER; note = 2'-O-methyl guanosine
  modified_base 6: mod_base = OTHER; note = 2'-fluoro cytidine
  modified_base 7: mod_base = OTHER; note = 2'-deoxy thymidine 5'-thiophosphate
  modified_base 8: mod_base = OTHER; note = 2'-O-methyl uridine
  modified_base 9: mod_base = OTHER; note = 2'-fluoro uridine
  modified_base 10: mod_base = OTHER; note = 2'-O-methyl uridine
  modified_base 11: mod_base = OTHER; note = 2'-O-methyl uridine
  modified_base 12: mod_base = OTHER; note = 2'-O-methyl guanosine
  modified_base 13: mod_base = OTHER; note = 2'-O-methyl guanosine
  modified_base 14: mod_base = OTHER; note = 2'-fluoro uridine
  modified_base 15: mod_base = OTHER; note = 2'-O-methyl guanosine
  modified_base 16: mod_base = OTHER; note = 2'-fluoro adenosine
  modified_base 17: mod_base = OTHER; note = 2'-O-methyl cytidine
  modified_base 18: mod_base = OTHER; note = 2'-O-methyl guanosine
  modified_base 19: mod_base = OTHER; note = 2'-O-methyl cytidine
  modified_base 20: mod_base = OTHER; note = 2'-O-methyl uridine 5'-thiophosphate
  modified_base 21: mod_base = OTHER; note = 2'-O-methyl uridine 5'-thiophosphate
ttgcgctttttggtgacgctt

SEQ ID NO: 73 - RNA, 21 nt, synthetic construct
  source 1..21: mol_type = other RNA
  modified_base 1: mod_base = OTHER; note = 2'-O-methyl uridine
  modified_base 2: mod_base = OTHER; note = 2'-O-methyl uridine 5'-thiophosphate
  modified_base 3: mod_base = OTHER; note = 2'-O-methyl guanosine 5'-thiophosphate
  modified_base 4: mod_base = OTHER; note = 2'-O-methyl cytidine
  modified_base 5: mod_base = OTHER; note = 2'-O-methyl guanosine
  modified_base 6: mod_base = OTHER; note = 2'-fluoro cytidine
  modified_base 7: mod_base = OTHER; note = 2'-deoxy thymidine 5'-thiophosphate
  modified_base 8: mod_base = OTHER; note = 2'-O-methyl uridine
  modified_base 9: mod_base = OTHER; note = 2'-fluoro uridine
  modified_base 10: mod_base = OTHER; note = 2'-O-methyl uridine
  modified_base 11: mod_base = OTHER; note = 2'-O-methyl uridine
  modified_base 12: mod_base = OTHER; note = 2'-O-methyl guanosine
  modified_base 13: mod_base = OTHER; note = 2'-O-methyl guanosine
  modified_base 14: mod_base = OTHER; note = 2'-fluoro uridine
  modified_base 15: mod_base = OTHER; note = 2'-O-methyl guanosine
  modified_base 16: mod_base = OTHER; note = 2'-fluoro adenosine
  modified_base 17: mod_base = OTHER; note = 2'-O-methyl cytidine
  modified_base 18: mod_base = OTHER; note = 2'-O-methyl guanosine
  modified_base 19: mod_base = OTHER; note = 2'-O-methyl cytidine
  modified_base 20: mod_base = OTHER; note = 2'-O-methyl uridine 5'-thiophosphate
  modified_base 21: mod_base = OTHER; note = 2'-O-methyl uridine 5'-thiophosphate
ttgcgctttttggtgacgctt

SEQ ID NO: 74 - RNA, 21 nt, synthetic construct
  source 1..21: mol_type = other RNA
  modified_base 1: mod_base = OTHER; note = 2'-O-methyl cytidine
  modified_base 2: mod_base = OTHER; note = 2'-O-methyl uridine 5'-thiophosphate
  modified_base 3: mod_base = OTHER; note = 2'-O-methyl cytidine 5'-thiophosphate
  modified_base 4: mod_base = OTHER; note = 2'-O-methyl uridine
  modified_base 5: mod_base = OTHER; note = 2'-O-methyl guanosine
  modified_base 6: mod_base = OTHER; note = 2'-O-methyl adenosine
  modified_base 7: mod_base = OTHER; note = 2'-fluoro guanosine
  modified_base 8: mod_base = OTHER; note = 2'-O-methyl uridine
  modified_base 9: mod_base = OTHER; note = 2'-fluoro uridine
  modified_base 10: mod_base = OTHER; note = 2'-fluoro cytidine
  modified_base 11: mod_base = OTHER; note = 2'-fluoro uridine
  modified_base 12: mod_base = OTHER; note = 2'-O-methyl guanosine
  modified_base 13: mod_base = OTHER; note = 2'-O-methyl guanosine
  modified_base 14: mod_base = OTHER; note = 2'-O-methyl guanosine
  modified_base 15: mod_base = OTHER; note = 2'-O-methyl adenosine
  modified_base 16: mod_base = OTHER; note = 2'-O-methyl uridine
  modified_base 17: mod_base = OTHER; note = 2'-O-methyl uridine
  modified_base 18: mod_base = OTHER; note = 2'-O-methyl uridine
  modified_base 19: mod_base = OTHER; note = 2'-O-methyl guanosine
  modified_base 20: mod_base = OTHER; note = 2'-deoxy thymidine 5'-thiophosphate
  modified_base 21: mod_base = OTHER; note = 2'-deoxy thymidine 5'-thiophosphate
ctctgagttctgggatttgtt

SEQ ID NO: 75 - RNA, 21 nt, synthetic construct
  source 1..21: mol_type = other RNA
  modified_base 1: mod_base = OTHER; note = 2'-O-methyl cytidine
  modified_base 2: mod_base = OTHER; note = 2'-O-methyl uridine 5'-thiophosphate
  modified_base 3: mod_base = OTHER; note = 2'-O-methyl cytidine 5'-thiophosphate
  modified_base 4: mod_base = OTHER; note = 2'-O-methyl uridine
  modified_base 5: mod_base = OTHER; note = 2'-O-methyl guanosine
  modified_base 6: mod_base = OTHER; note = 2'-O-methyl adenosine
  modified_base 7: mod_base = OTHER; note = 2'-fluoro guanosine
  modified_base 8: mod_base = OTHER; note = 2'-O-methyl uridine
  modified_base 9: mod_base = OTHER; note = 2'-fluoro uridine
  modified_base 10: mod_base = OTHER; note = 2'-fluoro cytidine
  modified_base 11: mod_base = OTHER; note = 2'-fluoro uridine
  modified_base 12: mod_base = OTHER; note = 2'-O-methyl guanosine
  modified_base 13: mod_base = OTHER; note = 2'-O-methyl guanosine
  modified_base 14: mod_base = OTHER; note = 2'-O-methyl guanosine
  modified_base 15: mod_base = OTHER; note = 2'-O-methyl adenosine
  modified_base 16: mod_base = OTHER; note = 2'-O-methyl uridine
  modified_base 17: mod_base = OTHER; note = 2'-O-methyl uridine
  modified_base 18: mod_base = OTHER; note = 2'-O-methyl uridine
  modified_base 19: mod_base = OTHER; note = 2'-O-methyl guanosine
  modified_base 20: mod_base = OTHER; note = 2'-deoxy thymidine 5'-thiophosphate
  modified_base 21: mod_base = OTHER; note = 2'-deoxy thymidine 5'-thiophosphate
  misc_feature 21: note = 3'-O attached to a GalNAc-comprising compound via a linker
ctctgagttctgggatttgtt

SEQ ID NO: 76 - RNA, 21 nt, synthetic construct
  source 1..21: mol_type = other RNA
  modified_base 1: mod_base = OTHER; note = 2'-O-methyl cytidine
  modified_base 2: mod_base = OTHER; note = 2'-fluoro uridine 5'-thiophosphate
  modified_base 3: mod_base = OTHER; note = 2'-O-methyl cytidine 5'-thiophosphate
  modified_base 4: mod_base = OTHER; note = 2'-O-methyl uridine
  modified_base 6: mod_base = OTHER; note = 2'-O-methyl adenosine 5'-thiophosphate
  modified_base 8: mod_base = OTHER; note = 2'-O-methyl uridine 5'-thiophosphate
  modified_base 9: mod_base = OTHER; note = 2'-fluoro uridine
  modified_base 10: mod_base = OTHER; note = 2'-fluoro cytidine
  modified_base 11: mod_base = OTHER; note = 2'-O-methyl uridine
  modified_base 12: mod_base = OTHER; note = 2'-O-methyl guanosine
  modified_base 14: mod_base = OTHER; note = 2'-O-methyl guanosine 5'-thiophosphate
  modified_base 16: mod_base = OTHER; note = 2'-O-methyl uridine 5'-thiophosphate
  modified_base 17: mod_base = OTHER; note = 2'-O-methyl uridine
  modified_base 18: mod_base = OTHER; note = 2'-fluoro uridine
  modified_base 19: mod_base = OTHER; note = 2'-O-methyl guanosine
  modified_base 20: mod_base = OTHER; note = 2'-deoxy thymidine 5'-thiophosphate
  modified_base 21: mod_base = OTHER; note = 2'-deoxy thymidine 5'-thiophosphate
ctctgagttctgggatttgtt

SEQ ID NO: 77 - RNA, 21 nt, synthetic construct
  source 1..21: mol_type = other RNA
  modified_base 1: mod_base = OTHER; note = 2'-O-methyl cytidine
  modified_base 2: mod_base = OTHER; note = 2'-fluoro adenosine 5'-thiophosphate
  modified_base 3: mod_base = OTHER; note = 2'-O-methyl adenosine 5'-thiophosphate
  modified_base 4: mod_base = OTHER; note = 2'-O-methyl adenosine
  modified_base 5: mod_base = OTHER; note = 2'-O-methyl uridine
  modified_base 6: mod_base = OTHER; note = 2'-fluoro cytidine
  modified_base 7: mod_base = OTHER; note = 2'-O-methyl cytidine
  modified_base 8: mod_base = OTHER; note = 2'-fluoro cytidine
  modified_base 9: mod_base = OTHER; note = 2'-fluoro adenosine
  modified_base 10: mod_base = OTHER; note = 2'-O-methyl guanosine
  modified_base 11: mod_base = OTHER; note = 2'-O-methyl adenosine
  modified_base 12: mod_base = OTHER; note = 2'-O-methyl adenosine
  modified_base 13: mod_base = OTHER; note = 2'-O-methyl cytidine
  modified_base 14: mod_base = OTHER; note = 2'-fluoro uridine
  modified_base 15: mod_base = OTHER; note = 2'-O-methyl cytidine
  modified_base 16: mod_base = OTHER; note = 2'-fluoro adenosine
  modified_base 17: mod_base = OTHER; note = 2'-O-methyl guanosine
  modified_base 18: mod_base = OTHER; note = 2'-O-methyl adenosine
  modified_base 19: mod_base = OTHER; note = 2'-O-methyl guanosine
  modified_base 20: mod_base = OTHER; note = 2'-deoxy thymidine 5'-thiophosphate
  modified_base 21: mod_base = OTHER; note = 2'-deoxy thymidine 5'-thiophosphate
caaatcccagaactcagagtt

SEQ ID NO: 78 - RNA, 19 nt, synthetic construct
  source 1..19: mol_type = other RNA
  modified_base 1: mod_base = OTHER; note = 2'-O-methyl cytidine
  modified_base 2: mod_base = OTHER; note = 2'-O-methyl uridine 5'-thiophosphate
  modified_base 3: mod_base = OTHER; note = 2'-O-methyl cytidine 5'-thiophosphate
  modified_base 4: mod_base = OTHER; note = uridine 5'-thiophosphate
  modified_base 17: mod_base = OTHER; note = 2'-O-methyl uridine
  modified_base 18: mod_base = OTHER; note = 2'-O-methyl uridine
  modified_base 19: mod_base = OTHER; note = 2'-O-methyl guanosine
ctctgagttctgggatttg

SEQ ID NO: 79 - RNA, 19 nt, synthetic construct
  source 1..19: mol_type = other RNA
  modified_base 1: mod_base = OTHER; note = 2'-O-methyl cytidine
  modified_base 2: mod_base = OTHER; note = 2'-O-methyl uridine 5'-thiophosphate
  modified_base 3: mod_base = OTHER; note = 2'-O-methyl cytidine 5'-thiophosphate
  modified_base 4: mod_base = OTHER; note = uridine 5'-thiophosphate
  modified_base 17: mod_base = OTHER; note = 2'-O-methyl uridine
  modified_base 18: mod_base = OTHER; note = 2'-O-methyl uridine 5'-thiophosphate
  modified_base 19: mod_base = OTHER; note = 2'-O-methyl guanosine 5'-thiophosphate
ctctgagttctgggatttg

SEQ ID NO: 80 - RNA, 21 nt, synthetic construct
  source 1..21: mol_type = other RNA
  modified_base 1: mod_base = OTHER; note = 2'-O-methyl cytidine
  modified_base 2: mod_base = OTHER; note = 2'-O-methyl uridine 5'-thiophosphate
  modified_base 3: mod_base = OTHER; note = 2'-O-methyl cytidine 5'-thiophosphate
  modified_base 4: mod_base = OTHER; note = 2'-O-methyl uridine 5'-thiophosphate
  modified_base 6: mod_base = OTHER; note = 2'-O-methyl adenosine
  modified_base 8: mod_base = OTHER; note = 2'-O-methyl uridine
  modified_base 12: mod_base = OTHER; note = 2'-O-methyl guanosine
  modified_base 14: mod_base = OTHER; note = 2'-O-methyl guanosine
  modified_base 16: mod_base = OTHER; note = 2'-O-methyl uridine
  modified_base 17: mod_base = OTHER; note = 2'-O-methyl uridine
  modified_base 18: mod_base = OTHER; note = 2'-O-methyl uridine
  modified_base 19: mod_base = OTHER; note = 2'-O-methyl guanosine
  modified_base 20: mod_base = OTHER; note = 2'-O-methyl uridine 5'-thiophosphate
  modified_base 21: mod_base = OTHER; note = 2'-O-methyl uridine 5'-thiophosphate
ctctgagttctgggatttgtt

SEQ ID NO: 81 - RNA, 21 nt, synthetic construct
  source 1..21: mol_type = other RNA
  modified_base 1: mod_base = OTHER; note = 2'-O-methyl cytidine
  modified_base 2: mod_base = OTHER; note = 2'-O-methyl uridine 5'-thiophosphate
  modified_base 3: mod_base = OTHER; note = 2'-O-methyl cytidine 5'-thiophosphate
  modified_base 4: mod_base = OTHER; note = 2'-O-methyl uridine 5'-thiophosphate
  modified_base 6: mod_base = OTHER; note = 2'-O-methyl adenosine
  modified_base 8: mod_base = OTHER; note = 2'-O-methyl uridine
  modified_base 12: mod_base = OTHER; note = 2'-O-methyl guanosine
  modified_base 14: mod_base = OTHER; note = 2'-O-methyl guanosine
  modified_base 16: mod_base = OTHER; note = 2'-O-methyl uridine
  modified_base 18: mod_base = OTHER; note = 2'-O-methyl uridine
  modified_base 19: mod_base = OTHER; note = 2'-O-methyl guanosine
  modified_base 20: mod_base = OTHER; note = 2'-O-methyl uridine 5'-thiophosphate
  modified_base 21: mod_base = OTHER; note = 2'-O-methyl uridine 5'-thiophosphate
ctctgagttctgggatttgtt

SEQ ID NO: 82 - RNA, 21 nt, synthetic construct
  source 1..21: mol_type = other RNA
  modified_base 1: mod_base = OTHER; note = 2'-O-methyl cytidine
  modified_base 2: mod_base = OTHER; note = 2'-O-methyl uridine 5'-thiophosphate
  modified_base 3: mod_base = OTHER; note = 2'-O-methyl cytidine 5'-thiophosphate
  modified_base 4: mod_base = OTHER; note = 2'-O-methyl uridine
  modified_base 6: mod_base = OTHER; note = 2'-O-methyl adenosine 5'-thiophosphate
  modified_base 8: mod_base = OTHER; note = 2'-O-methyl uridine 5'-thiophosphate
  modified_base 9: mod_base = OTHER; note = 2'-fluoro uridine
  modified_base 10: mod_base = OTHER; note = 2'-fluoro cytidine
  modified_base 11: mod_base = OTHER; note = 2'-O-methyl uridine
  modified_base 12: mod_base = OTHER; note = 2'-O-methyl guanosine
  modified_base 14: mod_base = OTHER; note = 2'-O-methyl guanosine 5'-thiophosphate
  modified_base 16: mod_base = OTHER; note = 2'-O-methyl uridine 5'-thiophosphate
  modified_base 17: mod_base = OTHER; note = 2'-O-methyl uridine
  modified_base 18: mod_base = OTHER; note = 2'-O-methyl uridine
  modified_base 19: mod_base = OTHER; note = 2'-O-methyl guanosine
  modified_base 20: mod_base = OTHER; note = 2'-O-methyl uridine 5'-thiophosphate
  modified_base 21: mod_base = OTHER; note = 2'-O-methyl uridine 5'-thiophosphate
  misc_feature 21: note = 3'-O attached to a GalNAc-comprising compound via a linker
ctctgagttctgggatttgtt

SEQ ID NO: 83 - RNA, 21 nt, synthetic construct
  source 1..21: mol_type = other RNA
  modified_base 1: mod_base = OTHER; note = 2'-O-methyl cytidine
  modified_base 2: mod_base = OTHER; note = 2'-O-methyl uridine 5'-thiophosphate
  modified_base 3: mod_base = OTHER; note = 2'-O-methyl cytidine 5'-thiophosphate
  modified_base 4: mod_base = OTHER; note = 2'-O-methyl uridine
  modified_base 6: mod_base = OTHER; note = 2'-O-methyl adenosine 5'-thiophosphate
  modified_base 8: mod_base = OTHER; note = 2'-O-methyl uridine 5'-thiophosphate
  modified_base 9: mod_base = OTHER; note = 2'-fluoro uridine
  modified_base 10: mod_base = OTHER; note = 2'-fluoro cytidine
  modified_base 12: mod_base = OTHER; note = 2'-O-methyl guanosine 5'-thiophosphate
  modified_base 14: mod_base = OTHER; note = 2'-O-methyl guanosine 5'-thiophosphate
  modified_base 16: mod_base = OTHER; note = 2'-O-methyl uridine 5'-thiophosphate
  modified_base 17: mod_base = OTHER; note = 2'-O-methyl uridine
  modified_base 18: mod_base = OTHER; note = 2'-O-methyl uridine
  modified_base 19: mod_base = OTHER; note = 2'-O-methyl guanosine
  modified_base 20: mod_base = OTHER; note = 2'-O-methyl uridine
  modified_base 21: mod_base = OTHER; note = 2'-O-methyl uridine
  misc_feature 21: note = 3'-O attached to a GalNAc-comprising compound via a linker
ctctgagttctgggatttgtt

SEQ ID NO: 84 - RNA, 21 nt, synthetic construct
  source 1..21: mol_type = other RNA
  modified_base 1: mod_base = OTHER; note = 2'-O-methyl cytidine
  modified_base 2: mod_base = OTHER; note = 2'-deoxy adenosine 5'-thiophosphate
  modified_base 3: mod_base = OTHER; note = 2'-O-methyl adenosine 5'-thiophosphate
  modified_base 4: mod_base = OTHER; note = 2'-O-methyl adenosine
  modified_base 5: mod_base = OTHER; note = 2'-O-methyl uridine
  modified_base 6: mod_base = OTHER; note = 2'-fluoro cytidine
  modified_base 7: mod_base = OTHER; note = 2'-deoxy cytidine 5'-thiophosphate
  modified_base 8: mod_base = OTHER; note = 2'-O-methyl cytidine
  modified_base 9: mod_base = OTHER; note = 2'-fluoro adenosine
  modified_base 10: mod_base = OTHER; note = 2'-O-methyl guanosine
  modified_base 11: mod_base = OTHER; note = 2'-O-methyl adenosine
  modified_base 12: mod_base = OTHER; note = 2'-O-methyl adenosine
  modified_base 13: mod_base = OTHER; note = 2'-O-methyl cytidine
  modified_base 14: mod_base = OTHER; note = 2'-fluoro uridine
  modified_base 15: mod_base = OTHER; note = 2'-O-methyl cytidine
  modified_base 16: mod_base = OTHER; note = 2'-fluoro adenosine
  modified_base 17: mod_base = OTHER; note = 2'-O-methyl guanosine
  modified_base 18: mod_base = OTHER; note = 2'-O-methyl adenosine
  modified_base 19: mod_base = OTHER; note = 2'-O-methyl guanosine
  modified_base 20: mod_base = OTHER; note = 2'-O-methyl uridine 5'-thiophosphate
  modified_base 21: mod_base = OTHER; note = 2'-O-methyl uridine 5'-thiophosphate
caaatcccagaactcagagtt

SEQ ID NO: 85 - RNA, 21 nt, synthetic construct
  source 1..21: mol_type = other RNA
  modified_base 1: mod_base = OTHER; note = 2'-O-methyl cytidine
  modified_base 2: mod_base = OTHER; note = 2'-deoxy adenosine 5'-thiophosphate
  modified_base 3: mod_base = OTHER; note = 2'-O-methyl adenosine 5'-thiophosphate
  modified_base 4: mod_base = OTHER; note = 2'-O-methyl adenosine
  modified_base 5: mod_base = OTHER; note = 2'-O-methyl uridine
  modified_base 6: mod_base = OTHER; note = 2'-fluoro cytidine
  modified_base 7: mod_base = OTHER; note = 2'-deoxy cytidine 5'-thiophosphate
  modified_base 8: mod_base = OTHER; note = 2'-fluoro cytidine
  modified_base 9: mod_base = OTHER; note = 2'-fluoro adenosine
  modified_base 10: mod_base = OTHER; note = 2'-O-methyl guanosine
  modified_base 11: mod_base = OTHER; note = 2'-O-methyl adenosine
  modified_base 12: mod_base = OTHER; note = 2'-O-methyl adenosine
  modified_base 13: mod_base = OTHER; note = 2'-O-methyl cytidine
  modified_base 14: mod_base = OTHER; note = 2'-fluoro uridine
  modified_base 15: mod_base = OTHER; note = 2'-O-methyl cytidine
  modified_base 16: mod_base = OTHER; note = 2'-fluoro adenosine
  modified_base 17: mod_base = OTHER; note = 2'-O-methyl guanosine
  modified_base 18: mod_base = OTHER; note = 2'-O-methyl adenosine
  modified_base 19: mod_base = OTHER; note = 2'-O-methyl guanosine
  modified_base 20: mod_base = OTHER; note = 2'-O-methyl uridine 5'-thiophosphate
  modified_base 21: mod_base = OTHER; note = 2'-O-methyl uridine 5'-thiophosphate
caaatcccagaactcagagtt

SEQ ID NO: 86 - RNA, 21 nt, synthetic construct
  source 1..21: mol_type = other RNA
  modified_base 1: mod_base = OTHER; note = 2'-O-methyl cytidine
  modified_base 2: mod_base = OTHER; note = 2'-deoxy adenosine 5'-thiophosphate
  modified_base 3: mod_base = OTHER; note = 2'-O-methyl adenosine 5'-thiophosphate
  modified_base 4: mod_base = OTHER; note = 2'-fluoro adenosine
  modified_base 5: mod_base = OTHER; note = 2'-O-methyl uridine
  modified_base 6: mod_base = OTHER; note = 2'-fluoro cytidine
  modified_base 7: mod_base = OTHER; note = 2'-deoxy cytidine
  modified_base 8: mod_base = OTHER; note = 2'-O-methyl cytidine 5'-thiophosphate
  modified_base 9: mod_base = OTHER; note = 2'-fluoro adenosine
  modified_base 10: mod_base = OTHER; note = 2'-O-methyl guanosine
  modified_base 11: mod_base = OTHER; note = 2'-O-methyl adenosine
  modified_base 12: mod_base = OTHER; note = 2'-fluoro adenosine
  modified_base 13: mod_base = OTHER; note = 2'-O-methyl cytidine
  modified_base 14: mod_base = OTHER; note = 2'-fluoro uridine
  modified_base 15: mod_base = OTHER; note = 2'-O-methyl cytidine
  modified_base 16: mod_base = OTHER; note = 2'-fluoro adenosine
  modified_base 17: mod_base = OTHER; note = 2'-O-methyl guanosine
  modified_base 18: mod_base = OTHER; note = 2'-O-methyl adenosine
  modified_base 19: mod_base = OTHER; note = 2'-deoxy guanosine
  modified_base 20: mod_base = OTHER; note = 2'-O-methyl uridine 5'-thiophosphate
  modified_base 21: mod_base = OTHER; note = 2'-O-methyl uridine 5'-thiophosphate
caaatcccagaactcagagtt

SEQ ID NO: 87 - RNA, 21 nt, synthetic construct
  source 1..21: mol_type = other RNA
  modified_base 1: mod_base = OTHER; note = 2'-O-methyl cytidine
  modified_base 2: mod_base = OTHER; note = 2'-fluoro adenosine 5'-thiophosphate
  modified_base 3: mod_base = OTHER; note = 2'-O-methyl adenosine 5'-thiophosphate
  modified_base 4: mod_base = OTHER; note = 2'-O-methyl adenosine
  modified_base 5: mod_base = OTHER; note = 2'-O-methyl uridine
  modified_base 6: mod_base = OTHER; note = 2'-fluoro cytidine
  modified_base 7: mod_base = OTHER; note = 2'-deoxy cytidine
  modified_base 8: mod_base = OTHER; note = 2'-O-methyl cytidine 5'-thiophosphate
  modified_base 9: mod_base = OTHER; note = 2'-fluoro adenosine
  modified_base 10: mod_base = OTHER; note = 2'-O-methyl guanosine
  modified_base 11: mod_base = OTHER; note = 2'-O-methyl adenosine
  modified_base 12: mod_base = OTHER; note = 2'-O-methyl adenosine
  modified_base 13: mod_base = OTHER; note = 2'-O-methyl cytidine
  modified_base 14: mod_base = OTHER; note = 2'-fluoro uridine
  modified_base 15: mod_base = OTHER; note = 2'-O-methyl cytidine
  modified_base 16: mod_base = OTHER; note = 2'-fluoro adenosine
  modified_base 17: mod_base = OTHER; note = 2'-O-methyl guanosine
  modified_base 18: mod_base = OTHER; note = 2'-O-methyl adenosine
  modified_base 19: mod_base = OTHER; note = 2'-O-methyl guanosine
  modified_base 20: mod_base = OTHER; note = 2'-O-methyl uridine 5'-thiophosphate
  modified_base 21: mod_base = OTHER; note = 2'-O-methyl uridine 5'-thiophosphate
caaatcccagaactcagagtt

SEQ ID NO: 88 - RNA, 21 nt, synthetic construct
  source 1..21: mol_type = other RNA
  modified_base 1: mod_base = OTHER; note = 2'-O-methyl cytidine
  modified_base 2: mod_base = OTHER; note = 2'-deoxy adenosine 5'-thiophosphate
  modified_base 3: mod_base = OTHER; note = 2'-O-methyl adenosine 5'-thiophosphate
  modified_base 4: mod_base = OTHER; note = 2'-O-methyl adenosine
  modified_base 5: mod_base = OTHER; note = 2'-O-methyl uridine
  modified_base 6: mod_base = OTHER; note = 2'-fluoro cytidine
  modified_base 7: mod_base = OTHER; note = 2'-deoxy cytidine
  modified_base 8: mod_base = OTHER; note = 2'-O-methyl cytidine 5'-thiophosphate
  modified_base 9: mod_base = OTHER; note = 2'-fluoro adenosine
  modified_base 10: mod_base = OTHER; note = 2'-O-methyl guanosine
  modified_base 11: mod_base = OTHER; note = 2'-O-methyl adenosine
  modified_base 12: mod_base = OTHER; note = 2'-O-methyl adenosine
  modified_base 13: mod_base = OTHER; note = 2'-O-methyl cytidine
  modified_base 14: mod_base = OTHER; note = 2'-fluoro uridine
  modified_base 15: mod_base = OTHER; note = 2'-O-methyl cytidine
  modified_base 16: mod_base = OTHER; note = 2'-fluoro adenosine
  modified_base 17: mod_base = OTHER; note = 2'-O-methyl guanosine
  modified_base 18: mod_base = OTHER; note = 2'-O-methyl adenosine
  modified_base 19: mod_base = OTHER; note = 2'-O-methyl guanosine
  modified_base 20: mod_base = OTHER; note = 2'-O-methyl uridine 5'-thiophosphate
  modified_base 21: mod_base = OTHER; note = 2'-O-methyl uridine 5'-thiophosphate
caaatcccagaactcagagtt

SEQ ID NO: 89 - RNA, 21 nt, synthetic construct
  source 1..21: mol_type = other RNA
  modified_base 1: mod_base = OTHER; note = 2'-O-methyl guanosine
  modified_base 2: mod_base = OTHER; note = 2'-O-methyl guanosine 5'-thiophosphate
  modified_base 3: mod_base = OTHER; note = 2'-O-methyl adenosine 5'-thiophosphate
  modified_base 4: mod_base = OTHER; note = 2'-O-methyl uridine
  modified_base 5: mod_base = OTHER; note = 2'-O-methyl adenosine
  modified_base 6: mod_base = OTHER; note = 2'-O-methyl guanosine
  modified_base 7: mod_base = OTHER; note = 2'-fluoro uridine
  modified_base 8: mod_base = OTHER; note = 2'-O-methyl uridine
  modified_base 9: mod_base = OTHER; note = 2'-fluoro adenosine
  modified_base 10: mod_base = OTHER; note = 2'-fluoro cytidine
  modified_base 11: mod_base = OTHER; note = 2'-fluoro uridine
  modified_base 12: mod_base = OTHER; note = 2'-O-methyl guanosine
  modified_base 13: mod_base = OTHER; note = 2'-O-methyl adenosine
  modified_base 14: mod_base = OTHER; note = 2'-O-methyl cytidine
  modified_base 15: mod_base = OTHER; note = 2'-O-methyl cytidine
  modified_base 16: mod_base = OTHER; note = 2'-O-methyl guanosine
  modified_base 17: mod_base = OTHER; note = 2'-O-methyl guanosine
  modified_base 18: mod_base = OTHER; note = 2'-O-methyl guanosine
  modified_base 19: mod_base = OTHER; note = 2'-O-methyl adenosine
  modified_base 20: mod_base = OTHER; note = 2'-deoxy thymidine 5'-thiophosphate
  modified_base 21: mod_base = OTHER; note = 2'-deoxy thymidine 5'-thiophosphate
ggatagttactgaccgggatt

SEQ ID NO: 90 - RNA, 21 nt, synthetic construct
  source 1..21: mol_type = other RNA
  modified_base 1: mod_base = OTHER; note = 2'-O-methyl uridine
  modified_base 2: mod_base = OTHER; note = 2'-fluoro cytidine 5'-thiophosphate
  modified_base 3: mod_base = OTHER; note = 2'-O-methyl cytidine 5'-thiophosphate
  modified_base 4: mod_base = OTHER; note = 2'-O-methyl cytidine
  modified_base 5: mod_base = OTHER; note = 2'-O-methyl guanosine
  modified_base 6: mod_base = OTHER; note = 2'-fluoro guanosine
  modified_base 7: mod_base = OTHER; note = 2'-O-methyl uridine
  modified_base 8: mod_base = OTHER; note = 2'-fluoro cytidine
  modified_base 9: mod_base = OTHER; note = 2'-fluoro adenosine
  modified_base 10: mod_base = OTHER; note = 2'-O-methyl guanosine
  modified_base 11: mod_base = OTHER; note = 2'-O-methyl uridine
  modified_base 12: mod_base = OTHER; note = 2'-O-methyl adenosine
  modified_base 13: mod_base = OTHER; note = 2'-O-methyl adenosine
  modified_base 14: mod_base = OTHER; note = 2'-fluoro cytidine
  modified_base 15: mod_base = OTHER; note = 2'-O-methyl uridine
  modified_base 16: mod_base = OTHER; note = 2'-fluoro adenosine
  modified_base 17: mod_base = OTHER; note = 2'-O-methyl uridine
  modified_base 18: mod_base = OTHER; note = 2'-O-methyl cytidine
  modified_base 19: mod_base = OTHER; note = 2'-O-methyl cytidine
  modified_base 20: mod_base = OTHER; note = 2'-deoxy thymidine 5'-thiophosphate
  modified_base 21: mod_base = OTHER; note = 2'-deoxy thymidine 5'-thiophosphate
tcccggtcagtaactatcctt

SEQ ID NO: 91 - RNA, 21 nt, synthetic construct
  source 1..21: mol_type = other RNA
  modified_base 1: mod_base = OTHER; note = 2'-O-methyl guanosine
  modified_base 2: mod_base = OTHER; note = 2'-O-methyl guanosine 5'-thiophosphate
  modified_base 3: mod_base = OTHER; note = 2'-O-methyl adenosine 5'-thiophosphate
  modified_base 4: mod_base = OTHER; note = 2'-O-methyl uridine
  modified_base 6: mod_base = OTHER; note = 2'-O-methyl guanosine 5'-thiophosphate
  modified_base 8: mod_base = OTHER; note = 2'-O-methyl uridine 5'-thiophosphate
  modified_base 9: mod_base = OTHER; note = 2'-fluoro adenosine
  modified_base 10: mod_base = OTHER; note = 2'-fluoro cytidine
  modified_base 11: mod_base = OTHER; note = 2'-O-methyl uridine
  modified_base 12: mod_base = OTHER; note = 2'-O-methyl guanosine
  modified_base 14: mod_base = OTHER; note = 2'-O-methyl cytidine 5'-thiophosphate
  modified_base 16: mod_base = OTHER; note = 2'-O-methyl guanosine 5'-thiophosphate
  modified_base 17: mod_base = OTHER; note = 2'-O-methyl guanosine
  modified_base 18: mod_base = OTHER; note = 2'-O-methyl guanosine
  modified_base 19: mod_base = OTHER; note = 2'-O-methyl adenosine
  modified_base 20: mod_base = OTHER; note = 2'-O-methyl uridine 5'-thiophosphate
  modified_base 21: mod_base = OTHER; note = 2'-O-methyl uridine 5'-thiophosphate
ggatagttactgaccgggatt

SEQ ID NO: 92 - RNA, 21 nt, synthetic construct
  source 1..21: mol_type = other RNA
  modified_base 1: mod_base = OTHER; note = 2'-O-methyl guanosine
  modified_base 2: mod_base = OTHER; note = 2'-O-methyl guanosine 5'-thiophosphate
  modified_base 3: mod_base = OTHER; note = 2'-O-methyl adenosine 5'-thiophosphate
  modified_base 4: mod_base = OTHER; note = 2'-O-methyl uridine
  modified_base 6: mod_base = OTHER; note = 2'-O-methyl guanosine 5'-thiophosphate
  modified_base 8: mod_base = OTHER; note = 2'-O-methyl uridine 5'-thiophosphate
  modified_base 9: mod_base = OTHER; note = 2'-fluoro adenosine
  modified_base 10: mod_base = OTHER; note = 2'-fluoro cytidine
  modified_base 12: mod_base = OTHER; note = 2'-O-methyl guanosine 5'-thiophosphate
  modified_base 14: mod_base = OTHER; note = 2'-O-methyl cytidine 5'-thiophosphate
  modified_base 16: mod_base = OTHER; note = 2'-O-methyl guanosine 5'-thiophosphate
  modified_base 17: mod_base = OTHER; note = 2'-O-methyl guanosine
  modified_base 18: mod_base = OTHER; note = 2'-O-methyl guanosine
  modified_base 19: mod_base = OTHER; note = 2'-O-methyl adenosine
  modified_base 20: mod_base = OTHER; note = 2'-O-methyl uridine 5'-thiophosphate
  modified_base 21: mod_base = OTHER; note = 2'-O-methyl uridine 5'-thiophosphate
ggatagttactgaccgggatt

SEQ ID NO: 93 - RNA, 21 nt, synthetic construct
  source 1..21: mol_type = other RNA
  modified_base 1: mod_base = OTHER; note = 2'-O-methyl uridine
  modified_base 2: mod_base = OTHER; note = 2'-fluoro cytidine 5'-thiophosphate
  modified_base 3: mod_base = OTHER; note = 2'-O-methyl cytidine 5'-thiophosphate
  modified_base 4: mod_base = OTHER; note = 2'-O-methyl cytidine
  modified_base 5: mod_base = OTHER; note = 2'-O-methyl guanosine
  modified_base 6: mod_base = OTHER; note = 2'-fluoro guanosine
  modified_base 7: mod_base = OTHER; note = 2'-deoxy thymidine
  modified_base 8: mod_base = OTHER; note = 2'-O-methyl cytidine 5'-thiophosphate
  modified_base 9: mod_base = OTHER; note = 2'-fluoro adenosine
  modified_base 10: mod_base = OTHER; note = 2'-O-methyl guanosine
  modified_base 11: mod_base = OTHER; note = 2'-O-methyl uridine
  modified_base 12: mod_base = OTHER; note = 2'-O-methyl adenosine
  modified_base 13: mod_base = OTHER; note = 2'-O-methyl adenosine
  modified_base 14: mod_base = OTHER; note = 2'-fluoro cytidine
  modified_base 15: mod_base = OTHER; note = 2'-O-methyl uridine
  modified_base 16: mod_base = OTHER; note = 2'-fluoro adenosine
  modified_base 17: mod_base = OTHER; note = 2'-O-methyl uridine
  modified_base 18: mod_base = OTHER; note = 2'-O-methyl cytidine
  modified_base 19: mod_base = OTHER; note = 2'-O-methyl cytidine
  modified_base 20: mod_base = OTHER; note = 2'-O-methyl uridine 5'-thiophosphate
  modified_base 21: mod_base = OTHER; note = 2'-O-methyl uridine 5'-thiophosphate
tcccggtcagtaactatcctt

SEQ ID NO: 94 - RNA, 21 nt, synthetic construct
  source 1..21: mol_type = other RNA
  modified_base 1: mod_base = OTHER; note = 2'-O-methyl uridine
  modified_base 2: mod_base = OTHER; note = 2'-deoxy cytidine 5'-thiophosphate
  modified_base 3: mod_base = OTHER; note = 2'-O-methyl cytidine 5'-thiophosphate
  modified_base 4: mod_base = OTHER; note = 2'-O-methyl cytidine
  modified_base 5: mod_base = OTHER; note = 2'-O-methyl guanosine
  modified_base 6: mod_base = OTHER; note = 2'-fluoro guanosine
  modified_base 7: mod_base = OTHER; note = 2'-deoxy thymidine
  modified_base 8: mod_base = OTHER; note = 2'-O-methyl cytidine 5'-thiophosphate
  modified_base 9: mod_base = OTHER; note = 2'-fluoro adenosine
  modified_base 10: mod_base = OTHER; note = 2'-O-methyl guanosine
  modified_base 11: mod_base = OTHER; note = 2'-O-methyl uridine
  modified_base 12: mod_base = OTHER; note = 2'-O-methyl adenosine
  modified_base 13: mod_base = OTHER; note = 2'-O-methyl adenosine
  modified_base 14: mod_base = OTHER; note = 2'-fluoro cytidine
  modified_base 15: mod_base = OTHER; note = 2'-O-methyl uridine
  modified_base 16: mod_base = OTHER; note = 2'-fluoro adenosine
  modified_base 17: mod_base = OTHER; note = 2'-O-methyl uridine
  modified_base 18: mod_base = OTHER; note = 2'-O-methyl cytidine
  modified_base 19: mod_base = OTHER; note = 2'-O-methyl cytidine
  modified_base 20: mod_base = OTHER; note = 2'-O-methyl uridine 5'-thiophosphate
  modified_base 21: mod_base = OTHER; note = 2'-O-methyl uridine 5'-thiophosphate
tcccggtcagtaactatcctt

SEQ ID NO: 95 - RNA, 21 nt, synthetic construct
  source 1..21: mol_type = other RNA
  modified_base 1: mod_base = OTHER; note = 2'-O-methyl uridine
  modified_base 2: mod_base = OTHER; note = 2'-deoxy thymidine 5'-thiophosphate
  modified_base 3: mod_base = OTHER; note = 2'-O-methyl guanosine 5'-thiophosphate
  modified_base 4: mod_base = OTHER; note = 2'-O-methyl cytidine
  modified_base 5: mod_base = OTHER; note = 2'-O-methyl guanosine
  modified_base 6: mod_base = OTHER; note = 2'-fluoro cytidine
  modified_base 7: mod_base = OTHER; note = 2'-deoxy thymidine 5'-thiophosphate
  modified_base 8: mod_base = OTHER; note = 2'-O-methyl uridine
  modified_base 9: mod_base = OTHER; note = 2'-fluoro uridine
  modified_base 10: mod_base = OTHER; note = 2'-O-methyl uridine
  modified_base 11: mod_base = OTHER; note = 2'-O-methyl uridine
  modified_base 12: mod_base = OTHER; note = 2'-O-methyl guanosine
  modified_base 13: mod_base = OTHER; note = 2'-O-methyl guanosine
  modified_base 14: mod_base = OTHER; note = 2'-deoxy thymidine 5'-thiophosphate
  modified_base 15: mod_base = OTHER; note = 2'-O-methyl guanosine
  modified_base 16: mod_base = OTHER; note = 2'-fluoro adenosine
  modified_base 17: mod_base = OTHER; note = 2'-O-methyl cytidine
  modified_base 18: mod_base = OTHER; note = 2'-O-methyl guanosine
  modified_base 19: mod_base = OTHER; note = 2'-O-methyl cytidine
  modified_base 20: mod_base = OTHER; note = 2'-O-methyl uridine 5'-thiophosphate
  modified_base 21: mod_base = OTHER; note = 2'-O-methyl uridine 5'-thiophosphate
ttgcgctttttggtgacgctt

SEQ ID NO: 96 - RNA, 21 nt, synthetic construct
  source 1..21: mol_type = other RNA
  modified_base 1: mod_base = OTHER; note = 2'-O-methyl uridine
  modified_base 2: mod_base = OTHER; note = 2'-deoxy thymidine 5'-thiophosphate
  modified_base 3: mod_base = OTHER; note = 2'-O-methyl guanosine 5'-thiophosphate
  modified_base 4: mod_base = OTHER; note = 2'-O-methyl cytidine
  modified_base 5: mod_base = OTHER; note = 2'-O-methyl guanosine
  modified_base 6: mod_base = OTHER; note = 2'-fluoro cytidine
  modified_base 7: mod_base = OTHER; note = 2'-deoxy thymidine 5'-thiophosphate
  modified_base 8: mod_base = OTHER; note = 2'-O-methyl uridine
  modified_base 9: mod_base = OTHER; note = 2'-fluoro uridine
  modified_base 10: mod_base = OTHER; note = 2'-O-methyl uridine
  modified_base 11: mod_base = OTHER; note = 2'-O-methyl uridine
  modified_base 12: mod_base = OTHER; note = 2'-O-methyl guanosine
  modified_base 13: mod_base = OTHER; note = 2'-O-methyl guanosine
  modified_base 14: mod_base = OTHER; note = 2'-deoxy thymidine 5'-thiophosphate
  modified_base 15: mod_base = OTHER; note = 2'-O-methyl guanosine
  modified_base 16: mod_base = OTHER; note = 2'-fluoro adenosine
  modified_base 17: mod_base = OTHER; note = 2'-O-methyl cytidine
  modified_base 18: mod_base = OTHER; note = 2'-O-methyl guanosine
  modified_base 19: mod_base = OTHER; note = 2'-O-methyl cytidine
  modified_base 20: mod_base = OTHER; note = 2'-O-methyl uridine
  modified_base 21: mod_base = OTHER; note = 2'-O-methyl uridine
ttgcgctttttggtgacgctt

SEQ ID NO: 97 - RNA, 21 nt, synthetic construct
  source 1..21: mol_type = other RNA
  modified_base 1: mod_base = OTHER; note = 2'-O-methyl uridine
  modified_base 2: mod_base = OTHER; note = 2'-deoxy thymidine 5'-thiophosphate
  modified_base 3: mod_base = OTHER; note = 2'-O-methyl guanosine 5'-thiophosphate
  modified_base 4: mod_base = OTHER; note = 2'-O-methyl cytidine
  modified_base 5: mod_base = OTHER; note = 2'-O-methyl guanosine
  modified_base 6: mod_base = OTHER; note = 2'-deoxy cytidine 5'-thiophosphate
  modified_base 7: mod_base = OTHER; note = 2'-deoxy thymidine 5'-thiophosphate
  modified_base 8: mod_base = OTHER; note = 2'-O-methyl uridine
  modified_base 9: mod_base = OTHER; note = 2'-deoxy thymidine 5'-thiophosphate
  modified_base 10: mod_base = OTHER; note = 2'-O-methyl uridine
  modified_base 11: mod_base = OTHER; note = 2'-O-methyl uridine
  modified_base 12: mod_base = OTHER; note = 2'-O-methyl guanosine
  modified_base 13: mod_base = OTHER; note = 2'-O-methyl guanosine
  modified_base 14: mod_base = OTHER; note = 2'-deoxy thymidine 5'-thiophosphate
  modified_base 15: mod_base = OTHER; note = 2'-O-methyl guanosine
  modified_base 16: mod_base = OTHER; note = 2'-deoxy adenosine 5'-thiophosphate
  modified_base 17: mod_base = OTHER; note = 2'-O-methyl cytidine
  modified_base 18: mod_base = OTHER; note = 2'-O-methyl guanosine
  modified_base 19: mod_base = OTHER; note = 2'-O-methyl cytidine
  modified_base 20: mod_base = OTHER; note = 2'-O-methyl uridine 5'-thiophosphate
  modified_base 21: mod_base = OTHER; note = 2'-O-methyl uridine 5'-thiophosphate
ttgcgctttttggtgacgctt

SEQ ID NO: 98 - DNA, 19 bp, synthetic construct
  source 1..19: mol_type = other DNA
ggatagttactgaccggga

SEQ ID NO: 99 - DNA, 21 bp, synthetic construct
  source 1..21: mol_type = other DNA
aaacactgtgaggatgggatc

SEQ ID NO: 100 - DNA, 20 bp, synthetic construct
  source 1..20: mol_type = other DNA
tctgtcattcgtgcttccag

SEQ ID NO: 101 - DNA, 28 bp, synthetic construct
  source 1..28: mol_type = other DNA
tgtcacatgaagtatacccaggtttgcg

SEQ ID NO: 102 - DNA, 21 bp, synthetic construct
  source 1..21: mol_type = other DNA
gtgtcagagcccttgtaactg

SEQ ID NO: 103 - DNA, 20 bp, synthetic construct
  source 1..20: mol_type = other DNA
acatttgcccagttccgtag

SEQ ID NO: 104 - DNA, 23 bp, synthetic construct
  source 1..23: mol_type = other DNA
tcgtctgccatggtgaagatgcg

SEQ ID NO: 105 - DNA, 22 bp, synthetic construct
  source 1..22: mol_type = other DNA
aaaccgctatgaagttcctctc

SEQ ID NO: 106 - DNA, 22 bp, synthetic construct
  source 1..22: mol_type = other DNA
gtggtatcctctgtgaagtctc

SEQ ID NO: 107 - DNA, 25 bp, synthetic construct
  source 1..25: mol_type = other DNA
ttgtcaccagcatcagtcccaagaa

SEQ ID NO: 108 - DNA, 20 bp, synthetic construct
  source 1..20: mol_type = other DNA
agaccctcacactcagatca

SEQ ID NO: 109 - DNA, 20 bp, synthetic construct
  source 1..20: mol_type = other DNA
tgtctttgagatccatgccg

SEQ ID NO: 110 - DNA, 23 bp, synthetic construct
  source 1..23: mol_type = other DNA
cctgtagcccacgtcgtagcaaa

SEQ ID NO: 111 - RNA, 21 nt, synthetic construct
  source 1..21: mol_type = other RNA
  modified_base 1: mod_base = OTHER; note = 2'-O-methyl guanosine
  modified_base 2: mod_base = OTHER; note = 2'-O-methyl adenosine 5'-thiophosphate
  modified_base 3: mod_base = OTHER; note = 2'-O-methyl cytidine 5'-thiophosphate
  modified_base 4: mod_base = OTHER; note = 2'-O-methyl uridine
  modified_base 5: mod_base = OTHER; note = 2'-O-methyl uridine
  modified_base 6: mod_base = OTHER; note = 2'-O-methyl uridine
  modified_base 7: mod_base = OTHER; note = 2'-fluoro cytidine
  modified_base 8: mod_base = OTHER; note = 2'-O-methyl adenosine
  modified_base 9: mod_base = OTHER; note = 2'-fluoro uridine
  modified_base 10: mod_base = OTHER; note = 2'-fluoro cytidine
  modified_base 11: mod_base = OTHER; note = 2'-fluoro cytidine
  modified_base 12: mod_base = OTHER; note = 2'-O-methyl uridine
  modified_base 13: mod_base = OTHER; note = 2'-O-methyl guanosine
  modified_base 14: mod_base = OTHER; note = 2'-O-methyl guanosine
  modified_base 15: mod_base = OTHER; note = 2'-O-methyl adenosine
  modified_base 16: mod_base = OTHER; note = 2'-O-methyl adenosine
  modified_base 17: mod_base = OTHER; note = 2'-O-methyl adenosine
  modified_base 18: mod_base = OTHER; note = 2'-O-methyl uridine
  modified_base 19: mod_base = OTHER; note = 2'-O-methyl adenosine
  modified_base 20: mod_base = OTHER; note = 2'-O-methyl uridine
  modified_base 21: mod_base = OTHER; note = 2'-O-methyl adenosine
gactttcatcctggaaatata

SEQ ID NO: 112 - RNA, 23 nt, synthetic construct
  source 1..23: mol_type = other RNA
  modified_base 1: mod_base = OTHER; note = 2'-O-methyl uridine
  modified_base 2: mod_base = OTHER; note = 2'-fluoro adenosine 5'-thiophosphate
  modified_base 3: mod_base = OTHER; note = 2'-O-methyl uridine 5'-thiophosphate
  modified_base 4: mod_base = OTHER; note = 2'-O-methyl adenosine
  modified_base 5: mod_base = OTHER; note = 2'-O-methyl uridine
  modified_base 6: mod_base = OTHER; note = 2'-fluoro uridine
  modified_base 7: mod_base = OTHER; note = 2'-O-methyl uridine
  modified_base 8: mod_base = OTHER; note = 2'-fluoro cytidine
  modified_base 9: mod_base = OTHER; note = 2'-fluoro cytidine
  modified_base 10: mod_base = OTHER; note = 2'-O-methyl adenosine
  modified_base 11: mod_base = OTHER; note = 2'-O-methyl guanosine
  modified_base 12: mod_base = OTHER; note = 2'-O-methyl guanosine
  modified_base 13: mod_base = OTHER; note = 2'-O-methyl adenosine
  modified_base 14: mod_base = OTHER; note = 2'-fluoro uridine
  modified_base 15: mod_base = OTHER; note = 2'-O-methyl guanosine
  modified_base 16: mod_base = OTHER; note = 2'-fluoro adenosine
  modified_base 17: mod_base = OTHER; note = 2'-O-methyl adenosine
  modified_base 18: mod_base = OTHER; note = 2'-O-methyl adenosine
  modified_base 19: mod_base = OTHER; note = 2'-O-methyl guanosine
  modified_base 20: mod_base = OTHER; note = 2'-O-methyl uridine
  modified_base 21: mod_base = OTHER; note = 2'-O-methyl cytidine
  modified_base 22: mod_base = OTHER; note = 2'-O-methyl cytidine 5'-thiophosphate
  modified_base 23: mod_base = OTHER; note = 2'-O-methyl adenosine 5'-thiophosphate
tatatttccaggatgaaagtcca

SEQ ID NO: 113 - RNA, 23 nt, synthetic construct
  source 1..23: mol_type = other RNA
  modified_base 1: mod_base = OTHER; note = 2'-O-methyl uridine
  modified_base 2: mod_base = OTHER; note = 2'-deoxy adenosine 5'-thiophosphate
  modified_base 3: mod_base = OTHER; note = 2'-O-methyl uridine 5'-thiophosphate
  modified_base 4: mod_base = OTHER; note = 2'-fluoro adenosine
  modified_base 5: mod_base = OTHER; note = 2'-O-methyl uridine
  modified_base 6: mod_base = OTHER; note = 2'-fluoro uridine
  modified_base 7: mod_base = OTHER; note = 2'-O-methyl uridine
  modified_base 8: mod_base = OTHER; note = 2'-O-methyl cytidine
  modified_base 9: mod_base = OTHER; note = 2'-fluoro cytidine
  modified_base 10: mod_base = OTHER; note = 2'-O-methyl adenosine
  modified_base 11: mod_base = OTHER; note = 2'-O-methyl guanosine
  modified_base 12: mod_base = OTHER; note = 2'-fluoro guanosine
  modified_base 13: mod_base = OTHER; note = 2'-O-methyl adenosine
  modified_base 14: mod_base = OTHER; note = 2'-fluoro uridine
  modified_base 15: mod_base = OTHER; note = 2'-O-methyl guanosine
  modified_base 16: mod_base = OTHER; note = 2'-fluoro adenosine
  modified_base 17: mod_base = OTHER; note = 2'-O-methyl adenosine
  modified_base 18: mod_base = OTHER; note = 2'-O-methyl adenosine
  modified_base 19: mod_base = OTHER; note = 2'-fluoro guanosine
  modified_base 20: mod_base = OTHER; note = 2'-O-methyl uridine
  modified_base 21: mod_base = OTHER; note = 2'-fluoro cytidine
  modified_base 22: mod_base = OTHER; note = 2'-O-methyl cytidine 5'-thiophosphate
  modified_base 23: mod_base = OTHER; note = 2'-O-methyl adenosine 5'-thiophosphate
tatatttccaggatgaaagtcca

SEQ ID NO: 114 - RNA, 21 nt, synthetic construct
  source 1..21: mol_type = other RNA
  modified_base 1: mod_base = OTHER; note = 2'-O-methyl guanosine
  modified_base 2: mod_base = OTHER; note = 2'-fluoro adenosine 5'-thiophosphate
  modified_base 3: mod_base = OTHER; note = 2'-O-methyl cytidine 5'-thiophosphate
  modified_base 4: mod_base = OTHER; note = 2'-O-methyl uridine
  modified_base 5: mod_base = OTHER; note = uridine 5'-thiophosphate
  modified_base 6: mod_base = OTHER; note = 2'-O-methyl uridine 5'-thiophosphate
  modified_base 7: mod_base = OTHER; note = cytidine 5'-thiophosphate
  modified_base 8: mod_base = OTHER; note = 2'-O-methyl adenosine 5'-thiophosphate
  modified_base 9: mod_base = OTHER; note = 2'-fluoro uridine
  modified_base 10: mod_base = OTHER; note = 2'-fluoro cytidine
  modified_base 11: mod_base = OTHER; note = 2'-O-methyl cytidine
  modified_base 12: mod_base = OTHER; note = 2'-O-methyl uridine
  modified_base 13: mod_base = OTHER; note = guanosine 5'-thiophosphate
  modified_base 14: mod_base = OTHER; note = 2'-O-methyl guanosine 5'-thiophosphate
  modified_base 15: mod_base = OTHER; note = adenosine 5'-thiophosphate
  modified_base 16: mod_base = OTHER; note = 2'-O-methyl adenosine 5'-thiophosphate
  modified_base 17: mod_base = OTHER; note = 2'-O-methyl adenosine
  modified_base 18: mod_base = OTHER; note = 2'-fluoro uridine
  modified_base 19: mod_base = OTHER; note = 2'-O-methyl adenosine
  modified_base 20: mod_base = OTHER; note = 2'-deoxy thymidine 5'-thiophosphate
  modified_base 21: mod_base = OTHER; note = 2'-deoxy adenosine 5'-thiophosphate
gactttcatcctggaaatata

SEQ ID NO: 115 - RNA, 21 nt, synthetic construct
  source 1..21: mol_type = other RNA
  modified_base 1: mod_base = OTHER; note = 2'-O-methyl uridine
  modified_base 2: mod_base = OTHER; note = 2'-deoxy adenosine 5'-thiophosphate
  modified_base 3: mod_base = OTHER; note = 2'-O-methyl uridine 5'-thiophosphate
  modified_base 4: mod_base = OTHER; note = 2'-fluoro adenosine
  modified_base 5: mod_base = OTHER; note = 2'-O-methyl uridine
  modified_base 6: mod_base = OTHER; note = 2'-fluoro uridine
  modified_base 7: mod_base = OTHER; note = 2'-O-methyl uridine
  modified_base 8: mod_base = OTHER; note = 2'-O-methyl cytidine
  modified_base 9: mod_base = OTHER; note = 2'-fluoro cytidine
  modified_base 10: mod_base = OTHER; note = 2'-O-methyl adenosine
  modified_base 11: mod_base = OTHER; note = 2'-O-methyl guanosine
  modified_base 12: mod_base = OTHER; note = 2'-fluoro guanosine
  modified_base 13: mod_base = OTHER; note = 2'-O-methyl adenosine
  modified_base 14: mod_base = OTHER; note = 2'-fluoro uridine
  modified_base 15: mod_base = OTHER; note = 2'-O-methyl guanosine
  modified_base 16: mod_base = OTHER; note = 2'-fluoro adenosine
  modified_base 17: mod_base = OTHER; note = 2'-O-methyl adenosine
  modified_base 18: mod_base = OTHER; note = 2'-O-methyl adenosine
  modified_base 19: mod_base = OTHER; note = 2'-fluoro guanosine
  modified_base 20: mod_base = OTHER; note = 2'-O-methyl uridine 5'-thiophosphate
  modified_base 21: mod_base = OTHER; note = 2'-O-methyl cytidine 5'-thiophosphate
tatatttccaggatgaaagtc

SEQ ID NO: 116 - RNA, 23 nt, synthetic construct
  source 1..23: mol_type = other RNA
  modified_base 1: mod_base = OTHER; note = 2'-O-methyl uridine
  modified_base 2: mod_base = OTHER; note = 2'-deoxy adenosine 5'-thiophosphate
  modified_base 3: mod_base = OTHER; note = 2'-O-methyl uridine 5'-thiophosphate
  modified_base 4: mod_base = OTHER; note = 2'-fluoro adenosine
  modified_base 5: mod_base = OTHER; note = 2'-O-methyl uridine
  modified_base 6: mod_base = OTHER; note = 2'-fluoro uridine
  modified_base 7: mod_base = OTHER; note = 2'-deoxy thymidine
  modified_base 8: mod_base = OTHER; note = 2'-O-methyl cytidine 5'-thiophosphate
  modified_base 9: mod_base = OTHER; note = 2'-fluoro cytidine
  modified_base 10: mod_base = OTHER; note = 2'-O-methyl adenosine
  modified_base 11: mod_base = OTHER; note = 2'-O-methyl guanosine
  modified_base 12: mod_base = OTHER; note = 2'-fluoro guanosine
  modified_base 13: mod_base = OTHER; note = 2'-O-methyl adenosine
  modified_base 14: mod_base = OTHER; note = 2'-fluoro uridine
  modified_base 15: mod_base = OTHER; note = 2'-O-methyl guanosine
  modified_base 16: mod_base = OTHER; note = 2'-fluoro adenosine
  modified_base 17: mod_base = OTHER; note = 2'-O-methyl adenosine
  modified_base 18: mod_base = OTHER; note = 2'-O-methyl adenosine
  modified_base 19: mod_base = OTHER; note = 2'-deoxy guanosine
  modified_base 20: mod_base = OTHER; note = 2'-O-methyl uridine 5'-thiophosphate
  modified_base 21: mod_base = OTHER; note = 2'-fluoro cytidine
  modified_base 22: mod_base = OTHER; note = 2'-O-methyl cytidine 5'-thiophosphate
  modified_base 23: mod_base = OTHER; note = 2'-O-methyl adenosine 5'-thiophosphate
tatatttccaggatgaaagtcca

SEQ ID NO: 117 - RNA, 21 nt, synthetic construct
  source 1..21: mol_type = other RNA
  modified_base 1: mod_base = OTHER; note = 2'-O-methyl uridine
  modified_base 2: mod_base = OTHER; note = 2'-deoxy adenosine 5'-thiophosphate
  modified_base 3: mod_base = OTHER; note = 2'-O-methyl uridine 5'-thiophosphate
  modified_base 4: mod_base = OTHER; note = 2'-fluoro adenosine
  modified_base 5: mod_base = OTHER; note = 2'-O-methyl uridine
  modified_base 6: mod_base = OTHER; note = 2'-fluoro uridine
  modified_base 7: mod_base = OTHER; note = 2'-deoxy thymidine
  modified_base 8: mod_base = OTHER; note = 2'-O-methyl cytidine 5'-thiophosphate
  modified_base 9: mod_base = OTHER; note = 2'-fluoro cytidine
  modified_base 10: mod_base = OTHER; note = 2'-O-methyl adenosine
  modified_base 11: mod_base = OTHER; note = 2'-O-methyl guanosine
  modified_base 12: mod_base = OTHER; note = 2'-fluoro guanosine
  modified_base 13: mod_base = OTHER; note = 2'-O-methyl adenosine
  modified_base 14: mod_base = OTHER; note = 2'-fluoro uridine
  modified_base 15: mod_base = OTHER; note = 2'-O-methyl guanosine
  modified_base 16: mod_base = OTHER; note = 2'-fluoro adenosine
  modified_base 17: mod_base = OTHER; note = 2'-O-methyl adenosine
  modified_base 18: mod_base = OTHER; note = 2'-O-methyl adenosine
  modified_base 19: mod_base = OTHER; note = 2'-deoxy guanosine
  modified_base 20: mod_base = OTHER; note = 2'-O-methyl uridine 5'-thiophosphate
  modified_base 21: mod_base = OTHER; note = 2'-O-methyl cytidine 5'-thiophosphate
tatatttccaggatgaaagtc

SEQ ID NO: 118 - RNA, 21 nt, synthetic construct
  source 1..21: mol_type = other RNA
  modified_base 1: mod_base = OTHER; note = 2'-O-methyl cytidine
  modified_base 2: mod_base = OTHER; note = 2'-O-methyl adenosine 5'-thiophosphate
  modified_base 3: mod_base = OTHER; note = 2'-O-methyl guanosine 5'-thiophosphate
  modified_base 4: mod_base = OTHER; note = 2'-O-methyl cytidine
  modified_base 5: mod_base = OTHER; note = 2'-O-methyl guanosine
  modified_base 6: mod_base = OTHER; note = 2'-O-methyl uridine
  modified_base 7: mod_base = OTHER; note = 2'-fluoro cytidine
  modified_base 8: mod_base = OTHER; note = 2'-O-methyl adenosine
  modified_base 9: mod_base = OTHER; note = 2'-fluoro cytidine
  modified_base 10: mod_base = OTHER; note = 2'-fluoro cytidine
  modified_base 11: mod_base = OTHER; note = 2'-fluoro adenosine
  modified_base 12: mod_base = OTHER; note = 2'-O-methyl adenosine
  modified_base 13: mod_base = OTHER; note = 2'-O-methyl adenosine
  modified_base 14: mod_base = OTHER; note = 2'-O-methyl adenosine
  modified_base 15: mod_base = OTHER; note = 2'-O-methyl adenosine
  modified_base 16: mod_base = OTHER; note = 2'-O-methyl guanosine
  modified_base 17: mod_base = OTHER; note = 2'-O-methyl cytidine
  modified_base 18: mod_base = OTHER; note = 2'-O-methyl guanosine
  modified_base 19: mod_base = OTHER; note = 2'-O-methyl cytidine
  modified_base 20: mod_base = OTHER; note = 2'-O-methyl adenosine
  modified_base 21: mod_base = OTHER; note = 2'-O-methyl adenosine
cagcgtcaccaaaaagcgcaa

SEQ ID NO: 119 - RNA, 23 nt, synthetic construct
  source 1..23: mol_type = other RNA
  modified_base 1: mod_base = OTHER; note = 2'-O-methyl uridine
  modified_base 2: mod_base = OTHER; note = 2'-fluoro uridine 5'-thiophosphate
  modified_base 3: mod_base = OTHER; note = 2'-O-methyl guanosine 5'-thiophosphate
  modified_base 4: mod_base = OTHER; note = 2'-O-methyl cytidine
  modified_base 5: mod_base = OTHER; note = 2'-O-methyl guanosine
  modified_base 6: mod_base = OTHER; note = 2'-fluoro cytidine
  modified_base 7: mod_base = OTHER; note = 2,3-dihydroxypropyl thymidine
  modified_base 8: mod_base = OTHER; note = 2'-fluoro uridine
  modified_base 9: mod_base = OTHER; note = 2'-fluoro uridine
  modified_base 10: mod_base = OTHER; note = 2'-O-methyl uridine
  modified_base 11: mod_base = OTHER; note = 2'-O-methyl uridine
  modified_base 12: mod_base = OTHER; note = 2'-O-methyl guanosine
  modified_base 13: mod_base = OTHER; note = 2'-O-methyl guanosine
  modified_base 14: mod_base = OTHER; note = 2'-fluoro uridine
  modified_base 15: mod_base = OTHER; note = 2'-O-methyl guanosine
  modified_base 16: mod_base = OTHER; note = 2'-fluoro adenosine
  modified_base 17: mod_base = OTHER; note = 2'-O-methyl cytidine
  modified_base 18: mod_base = OTHER; note = 2'-O-methyl guanosine
  modified_base 19: mod_base = OTHER; note = 2'-O-methyl cytidine
  modified_base 20: mod_base = OTHER; note = 2'-O-methyl uridine
  modified_base 21: mod_base = OTHER; note = 2'-O-methyl guanosine
  modified_base 22: mod_base = OTHER; note = 2'-O-methyl cytidine 5'-thiophosphate
  modified_base 23: mod_base = OTHER; note = 2'-O-methyl cytidine 5'-thiophosphate
ttgcgctttttggtgacgctgcc

SEQ ID NO: 120 - RNA, 21 nt, synthetic construct
  source 1..21: mol_type = other RNA
  modified_base 1: mod_base = OTHER; note = 2'-O-methyl guanosine
  modified_base 2: mod_base = OTHER; note = 2'-fluoro guanosine 5'-thiophosphate
  modified_base 3: mod_base = OTHER; note = 2'-O-methyl adenosine 5'-thiophosphate
  modified_base 4: mod_base = OTHER; note = 2'-O-methyl cytidine
  modified_base 6: mod_base = OTHER; note = 2'-O-methyl uridine 5'-thiophosphate
  modified_base 8: mod_base = OTHER; note = 2'-O-methyl cytidine 5'-thiophosphate
  modified_base 9: mod_base = OTHER; note = 2'-fluoro cytidine
  modified_base 10: mod_base = OTHER; note = 2'-fluoro adenosine
  modified_base 11: mod_base = OTHER; note = 2'-O-methyl adenosine
  modified_base 12: mod_base = OTHER; note = 2'-O-methyl guanosine
  modified_base 14: mod_base = OTHER; note = 2'-O-methyl cytidine 5'-thiophosphate
  modified_base 16: mod_base = OTHER; note = 2'-O-methyl guanosine 5'-thiophosphate
  modified_base 17: mod_base = OTHER; note = 2'-O-methyl uridine
  modified_base 18: mod_base = OTHER; note = 2'-fluoro adenosine
  modified_base 19: mod_base = OTHER; note = 2'-O-methyl uridine
  modified_base 20: mod_base = OTHER; note = 2'-deoxy thymidine 5'-thiophosphate
  modified_base 21: mod_base = OTHER; note = 2'-deoxy thymidine 5'-thiophosphate
ggacattccaagacagtattt

SEQ ID NO: 121 - RNA, 21 nt, synthetic construct
  source 1..21: mol_type = other RNA
  modified_base 1: mod_base = OTHER; note = 2'-O-methyl adenosine
  modified_base 2: mod_base = OTHER; note = 2'-deoxy thymidine 5'-thiophosphate
  modified_base 3: mod_base = OTHER; note = 2'-O-methyl adenosine 5'-thiophosphate
  modified_base 4: mod_base = OTHER; note = 2'-fluoro cytidine
  modified_base 5: mod_base = OTHER; note = 2'-O-methyl uridine
  modified_base 6: mod_base = OTHER; note = 2'-fluoro guanosine
  modified_base 7: mod_base = OTHER; note = 2'-deoxy thymidine
  modified_base 8: mod_base = OTHER; note = 2'-O-methyl cytidine 5'-thiophosphate
  modified_base 9: mod_base = OTHER; note = 2'-fluoro uridine
  modified_base 10: mod_base = OTHER; note = 2'-O-methyl uridine
  modified_base 11: mod_base = OTHER; note = 2'-O-methyl guanosine
  modified_base 12: mod_base = OTHER; note = 2'-fluoro guanosine
  modified_base 13: mod_base = OTHER; note = 2'-O-methyl adenosine
  modified_base 14: mod_base = OTHER; note = 2'-fluoro adenosine
  modified_base 15: mod_base = OTHER; note = 2'-O-methyl uridine
  modified_base 16: mod_base = OTHER; note = 2'-fluoro guanosine
  modified_base 17: mod_base = OTHER; note = 2'-O-methyl uridine
  modified_base 18: mod_base = OTHER; note = 2'-O-methyl cytidine
  modified_base 19: mod_base = OTHER; note = 2'-deoxy cytidine
  modified_base 20: mod_base = OTHER; note = 2'-O-methyl uridine 5'-thiophosphate
  modified_base 21: mod_base = OTHER; note = 2'-O-methyl uridine 5'-thiophosphate
atactgtcttggaatgtcctt

SEQ ID NO: 122 - RNA, 21 nt, synthetic construct
  source 1..21: mol_type = other RNA
  modified_base 1: mod_base = OTHER; note = 2'-O-methyl guanosine
  modified_base 2: mod_base = OTHER; note = 2'-O-methyl adenosine 5'-thiophosphate
  modified_base 3: mod_base = OTHER; note = 2'-O-methyl guanosine 5'-thiophosphate
  modified_base 4: mod_base = OTHER; note = 2'-O-methyl guanosine
  modified_base 5: mod_base = OTHER; note = 2'-O-methyl adenosine
  modified_base 6: mod_base = OTHER; note = 2'-O-methyl cytidine
  modified_base 7: mod_base = OTHER; note = 2'-fluoro adenosine
  modified_base 8: mod_base = OTHER; note = 2'-O-methyl uridine
  modified_base 9: mod_base = OTHER; note = 2'-fluoro uridine
  modified_base 10: mod_base = OTHER; note = 2'-fluoro cytidine
  modified_base 11: mod_base = OTHER; note = 2'-fluoro cytidine
  modified_base 12: mod_base = OTHER; note = 2'-O-methyl adenosine
  modified_base 13: mod_base = OTHER; note = 2'-O-methyl adenosine
  modified_base 14: mod_base = OTHER; note = 2'-O-methyl guanosine
  modified_base 15: mod_base = OTHER; note = 2'-O-methyl adenosine
  modified_base 16: mod_base = OTHER; note = 2'-O-methyl cytidine
  modified_base 17: mod_base = OTHER; note = 2'-O-methyl adenosine
  modified_base 18: mod_base = OTHER; note = 2'-O-methyl guanosine
  modified_base 19: mod_base = OTHER; note = 2'-O-methyl uridine
  modified_base 20: mod_base = OTHER; note = 2'-O-methyl adenosine
  modified_base 21: mod_base = OTHER; note = 2'-O-methyl uridine
gaggacattccaagacagtat

SEQ ID NO: 123 - RNA, 23 nt, synthetic construct
  source 1..23: mol_type = other RNA
  modified_base 1: mod_base = OTHER; note = 2'-O-methyl adenosine
  modified_base 2: mod_base = OTHER; note = 2'-fluoro uridine 5'-thiophosphate
  modified_base 3: mod_base = OTHER; note = 2'-O-methyl adenosine 5'-thiophosphate
  modified_base 4: mod_base = OTHER; note = 2'-O-methyl cytidine
  modified_base 5: mod_base = OTHER; note = 2'-O-methyl uridine
  modified_base 6: mod_base = OTHER; note = 2'-fluoro guanosine
  modified_base 7: mod_base = OTHER; note = 2,3-dihydroxypropyl thymidine
  modified_base 8: mod_base = OTHER; note = 2'-fluoro cytidine
  modified_base 9: mod_base = OTHER; note = 2'-fluoro uridine
  modified_base 10: mod_base = OTHER; note = 2'-O-methyl uridine
  modified_base 11: mod_base = OTHER; note = 2'-O-methyl guanosine
  modified_base 12: mod_base = OTHER; note = 2'-O-methyl guanosine
  modified_base 13: mod_base = OTHER; note = 2'-O-methyl adenosine
  modified_base 14: mod_base = OTHER; note = 2'-fluoro adenosine
  modified_base 15: mod_base = OTHER; note = 2'-O-methyl uridine
  modified_base 16: mod_base = OTHER; note = 2'-fluoro guanosine
  modified_base 17: mod_base = OTHER; note = 2'-O-methyl uridine
  modified_base 18: mod_base = OTHER; note = 2'-O-methyl cytidine
  modified_base 19: mod_base = OTHER; note = 2'-O-methyl cytidine
  modified_base 20: mod_base = OTHER; note = 2'-O-methyl uridine
  modified_base 21: mod_base = OTHER; note = 2'-O-methyl cytidine
  modified_base 22: mod_base = OTHER; note = 2'-O-methyl adenosine 5'-thiophosphate
  modified_base 23: mod_base = OTHER; note = 2'-O-methyl guanosine 5'-thiophosphate
atactgtcttggaatgtcctcag

SEQ ID NO: 124 - RNA, 21 nt, synthetic construct
  source 1..21: mol_type = other RNA
  modified_base 1: mod_base = OTHER; note = 2'-O-methyl uridine
  modified_base 2: mod_base = OTHER; note = 2'-O-methyl uridine 5'-thiophosphate
  modified_base 3: mod_base = OTHER; note = 2'-O-methyl cytidine 5'-thiophosphate
  modified_base 4: mod_base = OTHER; note = 2'-O-methyl uridine
  modified_base 5: mod_base = OTHER; note = 2'-O-methyl cytidine
  modified_base 6: mod_base = OTHER; note = 2'-O-methyl uridine
  modified_base 7: mod_base = OTHER; note = 2'-fluoro guanosine
  modified_base 8: mod_base = OTHER; note = 2'-O-methyl adenosine
  modified_base 9: mod_base = OTHER; note = 2'-fluoro guanosine
  modified_base 10: mod_base = OTHER; note = 2'-fluoro uridine
  modified_base 11: mod_base = OTHER; note = 2'-fluoro uridine
  modified_base 12: mod_base = OTHER; note = 2'-O-methyl cytidine
  modified_base 13: mod_base = OTHER; note = 2'-O-methyl uridine
  modified_base 14: mod_base = OTHER; note = 2'-O-methyl guanosine
  modified_base 15: mod_base = OTHER; note = 2'-O-methyl guanosine
  modified_base 16: mod_base = OTHER; note = 2'-O-methyl guanosine
  modified_base 17: mod_base = OTHER; note = 2'-O-methyl adenosine
  modified_base 18: mod_base = OTHER; note = 2'-O-methyl uridine
  modified_base 19: mod_base = OTHER; note = 2'-O-methyl uridine
  modified_base 20: mod_base = OTHER; note = 2'-O-methyl uridine
  modified_base 21: mod_base = OTHER; note = 2'-O-methyl guanosine
ttctctgagttctgggatttg

SEQ ID NO: 125 - RNA, 23 nt, synthetic construct
  source 1..23: mol_type = other RNA
  modified_base 1: mod_base = OTHER; note = 2'-O-methyl cytidine
  modified_base 2: mod_base = OTHER; note = 2'-fluoro adenosine 5'-thiophosphate
  modified_base 3: mod_base = OTHER; note = 2'-O-methyl adenosine 5'-thiophosphate
  modified_base 4: mod_base = OTHER; note = 2'-O-methyl adenosine
  modified_base 5: mod_base = OTHER; note = 2'-O-methyl uridine
  modified_base 6: mod_base = OTHER; note = 2'-fluoro cytidine
  modified_base 7: mod_base = OTHER; note = 2,3-dihydroxypropyl cytidine
  modified_base 8: mod_base = OTHER; note = 2'-fluoro cytidine
  modified_base 9: mod_base = OTHER; note = 2'-fluoro adenosine
  modified_base 10: mod_base = OTHER; note = 2'-O-methyl guanosine
  modified_base 11: mod_base = OTHER; note = 2'-O-methyl adenosine
  modified_base 12: mod_base = OTHER; note = 2'-O-methyl adenosine
  modified_base 13: mod_base = OTHER; note = 2'-O-methyl cytidine
  modified_base 14: mod_base = OTHER; note = 2'-fluoro uridine
  modified_base 15: mod_base = OTHER; note = 2'-O-methyl cytidine
  modified_base 16: mod_base = OTHER; note = 2'-fluoro adenosine
  modified_base 17: mod_base = OTHER; note = 2'-O-methyl guanosine
  modified_base 18: mod_base = OTHER; note = 2'-O-methyl adenosine
  modified_base 19: mod_base = OTHER; note = 2'-O-methyl guanosine
  modified_base 20: mod_base = OTHER; note = 2'-O-methyl adenosine
  modified_base 21: mod_base = OTHER; note = 2'-O-methyl adenosine
  modified_base 22: mod_base = OTHER; note = 2'-O-methyl cytidine 5'-thiophosphate
  modified_base 23: mod_base = OTHER; note = 2'-O-methyl uridine 5'-thiophosphate
caaatcccagaactcagagaact

SEQ ID NO: 126 - RNA, 23 nt, synthetic construct
  source 1..23: mol_type = other RNA
  modified_base 1: mod_base = OTHER; note = 2'-O-methyl cytidine
  modified_base 2: mod_base = OTHER; note = 2'-fluoro adenosine 5'-thiophosphate
  modified_base 3: mod_base = OTHER; note = 2'-O-methyl guanosine 5'-thiophosphate
  modified_base 4: mod_base = OTHER; note = 2'-O-methyl cytidine
  modified_base 6: mod_base = OTHER; note = 2'-O-methyl uridine 5'-thiophosphate
  modified_base 8: mod_base = OTHER; note = 2'-O-methyl adenosine 5'-thiophosphate
  modified_base 9: mod_base = OTHER; note = 2'-fluoro cytidine
  modified_base 10: mod_base = OTHER; note = 2'-fluoro cytidine
  modified_base 11: mod_base = OTHER; note = 2'-O-methyl adenosine
  modified_base 12: mod_base = OTHER; note = 2'-O-methyl adenosine
  modified_base 14: mod_base = OTHER; note = 2'-O-methyl adenosine 5'-thiophosphate
  modified_base 16: mod_base = OTHER; note = 2'-O-methyl guanosine 5'-thiophosphate
  modified_base 17: mod_base = OTHER; note = 2'-O-methyl cytidine
  modified_base 18: mod_base = OTHER; note = 2'-fluoro guanosine
  modified_base 19: mod_base = OTHER; note = 2'-O-methyl cytidine
  modified_base 20: mod_base = OTHER; note = 2'-O-methyl adenosine
  modified_base 21: mod_base = OTHER; note = 2'-fluoro adenosine
  modified_base 22: mod_base = OTHER; note = 2'-deoxy thymidine 5'-thiophosphate
  modified_base 23: mod_base = OTHER; note = 2'-deoxy thymidine 5'-thiophosphate
cagcgtcaccaaaaagcgcaatt

SEQ ID NO: 127 - RNA, 23 nt, synthetic construct
  source 1..23: mol_type = other RNA
  modified_base 1: mod_base = OTHER; note = 2'-O-methyl uridine
  modified_base 2: mod_base = OTHER; note = 2'-deoxy thymidine 5'-thiophosphate
  modified_base 3: mod_base = OTHER; note = 2'-O-methyl guanosine 5'-thiophosphate
  modified_base 4: mod_base = OTHER; note = 2'-fluoro cytidine
  modified_base 5: mod_base = OTHER; note = 2'-O-methyl guanosine
  modified_base 6: mod_base = OTHER; note = 2'-fluoro cytidine
  modified_base 7: mod_base = OTHER; note = 2'-deoxy thymidine
  modified_base 8: mod_base = OTHER; note = 2'-O-methyl uridine 5'-thiophosphate
  modified_base 9: mod_base = OTHER; note = 2'-fluoro uridine
  modified_base 10: mod_base = OTHER; note = 2'-O-methyl uridine
  modified_base 11: mod_base = OTHER; note = 2'-O-methyl uridine
  modified_base 12: mod_base = OTHER; note = 2'-fluoro guanosine
  modified_base 13: mod_base = OTHER; note = 2'-O-methyl guanosine
  modified_base 14: mod_base = OTHER; note = 2'-fluoro uridine
  modified_base 15: mod_base = OTHER; note = 2'-O-methyl guanosine
  modified_base 16: mod_base = OTHER; note = 2'-fluoro adenosine
  modified_base 17: mod_base = OTHER; note = 2'-O-methyl cytidine
  modified_base 18: mod_base = OTHER; note = 2'-O-methyl guanosine
  modified_base 19: mod_base = OTHER; note = 2'-deoxy cytidine
  modified_base 20: mod_base = OTHER; note = 2'-O-methyl uridine 5'-thiophosphate
  modified_base 21: mod_base = OTHER; note = 2'-O-methyl guanosine
  modified_base 22: mod_base = OTHER; note = 2'-deoxy cytidine 5'-thiophosphate
  modified_base 23: mod_base = OTHER; note = 2'-deoxy cytidine 5'-thiophosphate
ttgcgctttttggtgacgctgcc

SEQ ID NO: 128 - RNA, 23 nt, synthetic construct
  source 1..23: mol_type = other RNA
  modified_base 1: mod_base = OTHER; note = 2'-O-methyl guanosine
  modified_base 2: mod_base = OTHER; note = 2'-fluoro adenosine 5'-thiophosphate
  modified_base 3: mod_base = OTHER; note = 2'-O-methyl guanosine 5'-thiophosphate
  modified_base 4: mod_base = OTHER; note = 2'-O-methyl guanosine
  modified_base 6: mod_base = OTHER; note = 2'-O-methyl cytidine 5'-thiophosphate
  modified_base 8: mod_base = OTHER; note = 2'-O-methyl uridine 5'-thiophosphate
  modified_base 9: mod_base = OTHER; note = 2'-fluoro uridine
  modified_base 10: mod_base = OTHER; note = 2'-fluoro cytidine
  modified_base 11: mod_base = OTHER; note = 2'-O-methyl cytidine
  modified_base 12: mod_base = OTHER; note = 2'-O-methyl adenosine
  modified_base 14: mod_base = OTHER; note = 2'-O-methyl guanosine 5'-thiophosphate
  modified_base 16: mod_base = OTHER; note = 2'-O-methyl cytidine 5'-thiophosphate
  modified_base 17: mod_base = OTHER; note = 2'-O-methyl adenosine
  modified_base 18: mod_base = OTHER; note = 2'-fluoro guanosine
  modified_base 19: mod_base = OTHER; note = 2'-O-methyl uridine
  modified_base 20: mod_base = OTHER; note = 2'-O-methyl adenosine
  modified_base 21: mod_base = OTHER; note = 2'-fluoro uridine
  modified_base 22: mod_base = OTHER; note = 2'-deoxy thymidine 5'-thiophosphate
  modified_base 23: mod_base = OTHER; note = 2'-deoxy thymidine 5'-thiophosphate
gaggacattccaagacagtattt

SEQ ID NO: 129 - RNA, 23 nt, synthetic construct
  source 1..23: mol_type = other RNA
  modified_base 1: mod_base = OTHER; note = 2'-O-methyl adenosine
  modified_base 2: mod_base = OTHER; note = 2'-deoxy thymidine 5'-thiophosphate
  modified_base 3: mod_base = OTHER; note = 2'-O-methyl adenosine 5'-thiophosphate
  modified_base 4: mod_base = OTHER; note = 2'-fluoro cytidine
  modified_base 5: mod_base = OTHER; note = 2'-O-methyl uridine
  modified_base 6: mod_base = OTHER; note = 2'-fluoro guanosine
  modified_base 7: mod_base = OTHER; note = 2'-deoxy thymidine
  modified_base 8: mod_base = OTHER; note = 2'-O-methyl cytidine 5'-thiophosphate
  modified_base 9: mod_base = OTHER; note = 2'-fluoro uridine
  modified_base 10: mod_base = OTHER; note = 2'-O-methyl uridine
  modified_base 11: mod_base = OTHER; note = 2'-O-methyl guanosine
  modified_base 12: mod_base = OTHER; note = 2'-fluoro guanosine
  modified_base 13: mod_base = OTHER; note = 2'-O-methyl adenosine
  modified_base 14: mod_base = OTHER; note = 2'-fluoro adenosine
  modified_base 15: mod_base = OTHER; note = 2'-O-methyl uridine
  modified_base 16: mod_base = OTHER; note = 2'-fluoro guanosine
  modified_base 17: mod_base = OTHER; note = 2'-O-methyl uridine
  modified_base 18: mod_base = OTHER; note = 2'-O-methyl cytidine
  modified_base 19: mod_base = OTHER; note = 2'-fluoro cytidine
  modified_base 20: mod_base = OTHER; note = 2'-O-methyl uridine
  modified_base 21: mod_base = OTHER; note = 2'-deoxy cytidine
  modified_base 22: mod_base = OTHER; note = 2'-O-methyl adenosine 5'-thiophosphate
  modified_base 23: mod_base = OTHER; note = 2'-O-methyl guanosine 5'-thiophosphate
atactgtcttggaatgtcctcag

SEQ ID NO: 130 - RNA, 21 nt, synthetic construct
  source 1..21: mol_type = other RNA
  modified_base 1: mod_base = OTHER; note = 2'-O-methyl cytidine
  modified_base 2: mod_base = OTHER; note = 2'-fluoro cytidine 5'-thiophosphate
  modified_base 3: mod_base = OTHER; note = 2'-O-methyl adenosine 5'-thiophosphate
  modified_base 4: mod_base = OTHER; note = 2'-O-methyl adenosine
  modified_base 5: mod_base = OTHER; note = 2'-fluoro uridine
  modified_base 6: mod_base = OTHER; note = 2'-O-methyl adenosine
  modified_base 7: mod_base = OTHER; note = 2'-fluoro guanosine
  modified_base 8: mod_base = OTHER; note = 2'-O-methyl cytidine
  modified_base 9: mod_base = OTHER; note = 2'-fluoro uridine
  modified_base 10: mod_base = OTHER; note = 2'-fluoro uridine
  modified_base 11: mod_base = OTHER; note = 2'-O-methyl adenosine
  modified_base 12: mod_base = OTHER; note = 2'-O-methyl adenosine
  modified_base 13: mod_base = OTHER; note = 2'-fluoro cytidine
  modified_base 14: mod_base = OTHER; note = 2'-O-methyl adenosine
  modified_base 15: mod_base = OTHER; note = 2'-fluoro adenosine
  modified_base 16: mod_base = OTHER; note = 2'-O-methyl guanosine
  modified_base 17: mod_base = OTHER; note = 2'-O-methyl cytidine
  modified_base 18: mod_base = OTHER; note = 2'-fluoro cytidine
  modified_base 19: mod_base = OTHER; note = 2'-O-methyl uridine
  modified_base 20: mod_base = OTHER; note = 2'-deoxy thymidine 5'-thiophosphate
  modified_base 21: mod_base = OTHER; note = 2'-deoxy thymidine 5'-thiophosphate
ccaatagcttaacaagccttt

SEQ ID NO: 131 - RNA, 21 nt, synthetic construct
  source 1..21: mol_type = other RNA
  modified_base 1: mod_base = OTHER; note = 2'-O-methyl cytidine
  modified_base 2: mod_base = OTHER; note = 2'-fluoro cytidine 5'-thiophosphate
  modified_base 3: mod_base = OTHER; note = 2'-O-methyl adenosine 5'-thiophosphate
  modified_base 4: mod_base = OTHER; note = 2'-O-methyl adenosine
  modified_base 5: mod_base = OTHER; note = 2'-fluoro uridine
  modified_base 6: mod_base = OTHER; note = 2'-O-methyl adenosine
  modified_base 7: mod_base = OTHER; note = 2'-fluoro guanosine
  modified_base 8: mod_base = OTHER; note = 2'-O-methyl cytidine
  modified_base 9: mod_base = OTHER; note = 2'-fluoro uridine
  modified_base 10: mod_base = OTHER; note = 2'-fluoro uridine
  modified_base 11: mod_base = OTHER; note = 2'-O-methyl adenosine
  modified_base 12: mod_base = OTHER; note = 2'-O-methyl adenosine
  modified_base 13: mod_base = OTHER; note = 2'-fluoro cytidine
  modified_base 14: mod_base = OTHER; note = 2'-O-methyl adenosine
  modified_base 15: mod_base = OTHER; note = 2'-fluoro adenosine
  modified_base 16: mod_base = OTHER; note = 2'-O-methyl guanosine
  modified_base 17: mod_base = OTHER; note = 2'-O-methyl cytidine
  modified_base 18: mod_base = OTHER; note = 2'-fluoro cytidine
  modified_base 19: mod_base = OTHER; note = 2'-O-methyl uridine
  modified_base 20: mod_base = OTHER; note = 2'-deoxy thymidine 5'-thiophosphate
  modified_base 21: mod_base = OTHER; note = 2'-deoxy thymidine 5'-thiophosphate
  misc_feature 21: note = 3'-O attached to a GalNAc-comprising compound via a linker
ccaatagcttaacaagccttt

SEQ ID NO: 132 - RNA, 21 nt, synthetic construct
  source 1..21: mol_type = other RNA
  modified_base 1: mod_base = OTHER; note = 2'-O-methyl cytidine
  modified_base 2: mod_base = OTHER; note = 2'-fluoro cytidine 5'-thiophosphate
  modified_base 3: mod_base = OTHER; note = 2'-O-methyl adenosine 5'-thiophosphate
  modified_base 4: mod_base = OTHER; note = 2'-O-methyl adenosine
  modified_base 5: mod_base = OTHER; note = uridine 5'-thiophosphate
  modified_base 6: mod_base = OTHER; note = 2'-O-methyl adenosine 5'-thiophosphate
  modified_base 7: mod_base = OTHER; note = guanosine 5'-thiophosphate
  modified_base 8: mod_base = OTHER; note = 2'-O-methyl cytidine 5'-thiophosphate
  modified_base 9: mod_base = OTHER; note = 2'-fluoro uridine
  modified_base 10: mod_base = OTHER; note = 2'-fluoro uridine
  modified_base 11: mod_base = OTHER; note = 2'-O-methyl adenosine
  modified_base 12: mod_base = OTHER; note = 2'-O-methyl adenosine
  modified_base 13: mod_base = OTHER; note = cytidine 5'-thiophosphate
  modified_base 14: mod_base = OTHER; note = 2'-O-methyl adenosine 5'-thiophosphate
  modified_base 15: mod_base = OTHER; note = adenosine 5'-thiophosphate
  modified_base 16: mod_base = OTHER; note = 2'-O-methyl guanosine 5'-thiophosphate
  modified_base 17: mod_base = OTHER; note = 2'-O-methyl cytidine
  modified_base 18: mod_base = OTHER; note = 2'-fluoro cytidine
  modified_base 19: mod_base = OTHER; note = 2'-O-methyl uridine
  modified_base 20: mod_base = OTHER; note = 2'-deoxy thymidine 5'-thiophosphate
  modified_base 21: mod_base = OTHER; note = 2'-deoxy thymidine 5'-thiophosphate
  misc_feature 21: note = 3'-O attached to a GalNAc-comprising compound via a linker
ccaatagcttaacaagccttt

SEQ ID NO: 133 - RNA, 21 nt, synthetic construct
  source 1..21: mol_type = other RNA
  modified_base 1: mod_base = OTHER; note = 2'-O-methyl adenosine
  modified_base 2: mod_base = OTHER; note = 2'-deoxy guanosine 5'-thiophosphate
  modified_base 3: mod_base = OTHER; note = 2'-O-methyl guanosine 5'-thiophosphate
  modified_base 4: mod_base = OTHER; note = 2'-fluoro cytidine
  modified_base 5: mod_base = OTHER; note = 2'-O-methyl uridine
  modified_base 6: mod_base = OTHER; note = 2'-fluoro uridine
  modified_base 7: mod_base = OTHER; note = 2'-deoxy guanosine
  modified_base 8: mod_base = OTHER; note = 2'-O-methyl uridine 5'-thiophosphate
  modified_base 9: mod_base = OTHER; note = 2'-fluoro uridine
  modified_base 10: mod_base = OTHER; note = 2'-O-methyl adenosine
  modified_base 11: mod_base = OTHER; note = 2'-O-methyl adenosine
  modified_base 12: mod_base = OTHER; note = 2'-fluoro guanosine
  modified_base 13: mod_base = OTHER; note = 2'-O-methyl cytidine
  modified_base 14: mod_base = OTHER; note = 2'-fluoro uridine
  modified_base 15: mod_base = OTHER; note = 2'-O-methyl adenosine
  modified_base 16: mod_base = OTHER; note = 2'-fluoro uridine
  modified_base 17: mod_base = OTHER; note = 2'-O-methyl uridine
  modified_base 18: mod_base = OTHER; note = 2'-O-methyl guanosine
  modified_base 19: mod_base = OTHER; note = 2'-deoxy guanosine
  modified_base 20: mod_base = OTHER; note = 2'-O-methyl guanosine 5'-thiophosphate
  modified_base 21: mod_base = OTHER; note = 2'-O-methyl uridine 5'-thiophosphate
aggcttgttaagctattgggt

SEQ ID NO: 134 - RNA, 21 nt, synthetic construct
  source 1..21: mol_type = other RNA
  modified_base 1: mod_base = OTHER; note = 2'-O-methyl adenosine
  modified_base 2: mod_base = OTHER; note = 2'-deoxy guanosine 5'-thiophosphate
  modified_base 3: mod_base = OTHER; note = 2'-O-methyl guanosine 5'-thiophosphate
  modified_base 4: mod_base = OTHER; note = 2'-fluoro cytidine
  modified_base 5: mod_base = OTHER; note = 2'-O-methyl uridine
  modified_base 6: mod_base = OTHER; note = 2'-fluoro uridine
  modified_base 7: mod_base = OTHER; note = 2'-O-methyl guanosine
  modified_base 8: mod_base = OTHER; note = 2'-O-methyl uridine
  modified_base 9: mod_base = OTHER; note = 2'-fluoro uridine
  modified_base 10: mod_base = OTHER; note = 2'-O-methyl adenosine
  modified_base 11: mod_base = OTHER; note = 2'-O-methyl adenosine
  modified_base 12: mod_base = OTHER; note = 2'-fluoro guanosine
  modified_base 13: mod_base = OTHER; note = 2'-O-methyl cytidine
  modified_base 14: mod_base = OTHER; note = 2'-fluoro uridine
  modified_base 15: mod_base = OTHER; note = 2'-O-methyl adenosine
  modified_base 16: mod_base = OTHER; note = 2'-fluoro uridine
  modified_base 17: mod_base = OTHER; note = 2'-O-methyl uridine
  modified_base 18: mod_base = OTHER; note = 2'-O-methyl guanosine
  modified_base 19: mod_base = OTHER; note = 2'-fluoro guanosine
  modified_base 20: mod_base = OTHER; note = 2'-O-methyl guanosine 5'-thiophosphate
  modified_base 21: mod_base = OTHER; note = 2'-O-methyl uridine 5'-thiophosphate
aggcttgttaagctattgggt

SEQ ID NO: 135 - RNA, 21 nt, synthetic construct
  source 1..21: mol_type = other RNA
  modified_base 1: mod_base = OTHER; note = 2'-O-methyl adenosine
  modified_base 2: mod_base = OTHER; note = 2'-deoxy guanosine 5'-thiophosphate
  modified_base 3: mod_base = OTHER; note = 2'-O-methyl guanosine 5'-thiophosphate
  modified_base 4: mod_base = OTHER; note = 2'-fluoro cytidine
  modified_base 5: mod_base = OTHER; note = 2'-O-methyl uridine
  modified_base 6: mod_base = OTHER; note = 2'-fluoro uridine
  modified_base 7: mod_base = OTHER; note = 2'-deoxy guanosine
  modified_base 8: mod_base = OTHER; note = 2'-O-methyl uridine 5'-thiophosphate
  modified_base 9: mod_base = OTHER; note = 2'-fluoro uridine
  modified_base 10: mod_base = OTHER; note = 2'-O-methyl adenosine
  modified_base 11: mod_base = OTHER; note = 2'-O-methyl adenosine
  modified_base 12: mod_base = OTHER; note = 2'-fluoro guanosine
  modified_base 13: mod_base = OTHER; note = 2'-O-methyl cytidine
  modified_base 14: mod_base = OTHER; note = 2'-fluoro uridine
  modified_base 15: mod_base = OTHER; note = 2'-O-methyl adenosine
  modified_base 16: mod_base = OTHER; note = 2'-fluoro uridine
  modified_base 17: mod_base = OTHER; note = 2'-O-methyl uridine
  modified_base 18: mod_base = OTHER; note = 2'-O-methyl guanosine
  modified_base 19: mod_base = OTHER; note = 2'-deoxy guanosine
  modified_base 20: mod_base = OTHER; note = 2'-O-methyl guanosine 5'-thiophosphate
  modified_base 21: mod_base = OTHER; note = 2'-O-methyl uridine 5'-thiophosphate
aggcttgttaagctattgggt

SEQ ID NO: 136 - RNA, 23 nt, synthetic construct
  source 1..23: mol_type = other RNA
  modified_base 1: mod_base = OTHER; note = 2'-O-methyl adenosine
  modified_base 2: mod_base = OTHER; note = 2'-fluoro cytidine 5'-thiophosphate
  modified_base 3: mod_base = OTHER; note = 2'-O-methyl cytidine 5'-thiophosphate
  modified_base 4: mod_base = OTHER; note = 2'-O-methyl cytidine
  modified_base 5: mod_base = OTHER; note = 2'-fluoro adenosine
  modified_base 6: mod_base = OTHER; note = 2'-O-methyl adenosine
  modified_base 7: mod_base = OTHER; note = 2'-fluoro uridine
  modified_base 8: mod_base = OTHER; note = 2'-O-methyl adenosine
  modified_base 9: mod_base = OTHER; note = 2'-fluoro guanosine
  modified_base 10: mod_base = OTHER; note = 2'-fluoro cytidine
  modified_base 11: mod_base = OTHER; note = 2'-O-methyl uridine
  modified_base 12: mod_base = OTHER; note = 2'-O-methyl uridine
  modified_base 13: mod_base = OTHER; note = 2'-fluoro adenosine
  modified_base 14: mod_base = OTHER; note = 2'-O-methyl adenosine
  modified_base 15: mod_base = OTHER; note = 2'-fluoro cytidine
  modified_base 16: mod_base = OTHER; note = 2'-O-methyl adenosine
  modified_base 17: mod_base = OTHER; note = 2'-O-methyl adenosine
  modified_base 18: mod_base = OTHER; note = 2'-fluoro guanosine
  modified_base 19: mod_base = OTHER; note = 2'-O-methyl cytidine
  modified_base 20: mod_base = OTHER; note = 2'-O-methyl cytidine
  modified_base 21: mod_base = OTHER; note = 2'-fluoro uridine
  modified_base 22: mod_base = OTHER; note = 2'-deoxy thymidine 5'-thiophosphate
  modified_base 23: mod_base = OTHER; note = 2'-deoxy thymidine 5'-thiophosphate
  misc_feature 23: note = 3'-O attached to a GalNAc-comprising compound via a linker
acccaatagcttaacaagccttt

SEQ ID NO: 137 - RNA, 23 nt, synthetic construct
  source 1..23: mol_type = other RNA
  modified_base 1: mod_base = OTHER; note = 2'-O-methyl adenosine
  modified_base 2: mod_base = OTHER; note = 2'-deoxy guanosine 5'-thiophosphate
  modified_base 3: mod_base = OTHER; note = 2'-O-methyl guanosine 5'-thiophosphate
  modified_base 4: mod_base = OTHER; note = 2'-fluoro cytidine
  modified_base 5: mod_base = OTHER; note = 2'-O-methyl uridine
  modified_base 6: mod_base = OTHER; note = 2'-fluoro uridine
  modified_base 7: mod_base = OTHER; note = 2'-O-methyl guanosine
  modified_base 8: mod_base = OTHER; note = 2'-O-methyl uridine
  modified_base 9: mod_base = OTHER; note = 2'-fluoro uridine
  modified_base 10: mod_base = OTHER; note = 2'-O-methyl adenosine
  modified_base 11: mod_base = OTHER; note = 2'-O-methyl adenosine
  modified_base 12: mod_base = OTHER; note = 2'-fluoro guanosine
  modified_base 13: mod_base = OTHER; note = 2'-O-methyl cytidine
  modified_base 14: mod_base = OTHER; note = 2'-fluoro uridine
  modified_base 15: mod_base = OTHER; note = 2'-O-methyl adenosine
  modified_base 16: mod_base = OTHER; note = 2'-fluoro uridine
  modified_base 17: mod_base = OTHER; note = 2'-O-methyl uridine
  modified_base 18: mod_base = OTHER; note = 2'-O-methyl guanosine
  modified_base 19: mod_base = OTHER; note = 2'-fluoro guanosine
  modified_base 20: mod_base = OTHER; note = 2'-O-methyl guanosine
  modified_base 21: mod_base = OTHER; note = 2'-O-methyl uridine
  modified_base 22: mod_base = OTHER; note = 2'-deoxy thymidine 5'-thiophosphate
  modified_base 23: mod_base = OTHER; note = 2'-deoxy thymidine 5'-thiophosphate
aggcttgttaagctattgggttt

SEQ ID NO: 138 - DNA, 20 bp, synthetic construct
  source 1..20: mol_type = other DNA
ctgatccagcctcactatgc

SEQ ID NO: 139 - DNA, 21 bp, synthetic construct
  source 1..21: mol_type = other DNA
aggtcataagatccttgcagc

SEQ ID NO: 140 - DNA, 26 bp, synthetic construct
  source 1..26: mol_type = other DNA
agggtctcactttccagcaaaactcc

SEQ ID NO: 141 - RNA, 21 nt, synthetic construct
  source 1..21: mol_type = other RNA
  modified_base 1: mod_base = OTHER; note = 2'-O-methyl uridine
  modified_base 2: mod_base = OTHER; note = 2'-fluoro adenosine 5'-thiophosphate
  modified_base 3: mod_base = OTHER; note = 2'-O-methyl guanosine 5'-thiophosphate
  modified_base 4: mod_base = OTHER; note = 2'-O-methyl uridine
  modified_base 6: mod_base = OTHER; note = 2'-O-methyl guanosine 5'-thiophosphate
  modified_base 8: mod_base = OTHER; note = 2'-O-methyl uridine 5'-thiophosphate
  modified_base 9: mod_base = OTHER; note = 2'-fluoro guanosine
  modified_base 10: mod_base = OTHER; note = 2'-fluoro cytidine
  modified_base 11: mod_base = OTHER; note = 2'-O-methyl adenosine
  modified_base 12: mod_base = OTHER; note = 2'-O-methyl adenosine
  modified_base 14: mod_base = OTHER; note = 2'-O-methyl adenosine 5'-thiophosphate
  modified_base 16: mod_base = OTHER; note = 2'-O-methyl uridine 5'-thiophosphate
  modified_base 17: mod_base = OTHER; note = 2'-O-methyl uridine
  modified_base 18: mod_base = OTHER; note = 2'-fluoro guanosine
  modified_base 19: mod_base = OTHER; note = 2'-O-methyl adenosine
  modified_base 20: mod_base = OTHER; note = 2'-deoxy thymidine 5'-thiophosphate
  modified_base 21: mod_base = OTHER; note = 2'-deoxy thymidine 5'-thiophosphate
tagtcgctgcaaaacttgatt

SEQ ID NO: 142 - RNA, 21 nt, synthetic construct
  source 1..21: mol_type = other RNA
  modified_base 1: mod_base = OTHER; note = 2'-O-methyl uridine
  modified_base 2: mod_base = OTHER; note = 2'-deoxy cytidine 5'-thiophosphate
  modified_base 3: mod_base = OTHER; note = 2'-O-methyl adenosine 5'-thiophosphate
  modified_base 4: mod_base = OTHER; note = 2'-fluoro adenosine
  modified_base 5: mod_base = OTHER; note = 2'-O-methyl guanosine
  modified_base 6: mod_base = OTHER; note = 2'-fluoro uridine
  modified_base 7: mod_base = OTHER; note = 2'-deoxy thymidine
  modified_base 8: mod_base = OTHER; note = 2'-O-methyl uridine 5'-thiophosphate
  modified_base 9: mod_base = OTHER; note = 2'-fluoro uridine
  modified_base 10: mod_base = OTHER; note = 2'-O-methyl guanosine
  modified_base 11: mod_base = OTHER; note = 2'-O-methyl cytidine
  modified_base 12: mod_base = OTHER; note = 2'-fluoro adenosine
  modified_base 13: mod_base = OTHER; note = 2'-O-methyl guanosine
  modified_base 14: mod_base = OTHER; note = 2'-fluoro cytidine
  modified_base 15: mod_base = OTHER; note = 2'-O-methyl guanosine
  modified_base 16: mod_base = OTHER; note = 2'-fluoro adenosine
  modified_base 17: mod_base = OTHER; note = 2'-O-methyl cytidine
  modified_base 18: mod_base = OTHER; note = 2'-O-methyl uridine
  modified_base 19: mod_base = OTHER; note = 2'-deoxy adenosine
  modified_base 20: mod_base = OTHER; note = 2'-O-methyl guanosine 5'-thiophosphate
  modified_base 21: mod_base = OTHER; note = 2'-O-methyl cytidine 5'-thiophosphate
tcaagttttgcagcgactagc

SEQ ID NO: 143 - RNA, 21 nt, synthetic construct
  source 1..21: mol_type = other RNA
  modified_base 1: mod_base = OTHER; note = 2'-O-methyl uridine
  modified_base 2: mod_base = OTHER; note = 2'-fluoro adenosine 5'-thiophosphate
  modified_base 3: mod_base = OTHER; note = 2'-O-methyl guanosine 5'-thiophosphate
  modified_base 4: mod_base = OTHER; note = 2'-O-methyl uridine
  modified_base 5: mod_base = OTHER; note = 2'-fluoro cytidine
  modified_base 6: mod_base = OTHER; note = 2'-O-methyl guanosine
  modified_base 7: mod_base = OTHER; note = 2'-fluoro cytidine
  modified_base 8: mod_base = OTHER; note = 2'-O-methyl uridine
  modified_base 9: mod_base = OTHER; note = 2'-fluoro guanosine
  modified_base 10: mod_base = OTHER; note = 2'-fluoro cytidine
  modified_base 11: mod_base = OTHER; note = 2'-O-methyl guanosine
  modified_base 12: mod_base = OTHER; note = 2'-O-methyl adenosine
  modified_base 13: mod_base = OTHER; note = 2'-fluoro adenosine
  modified_base 14: mod_base = OTHER; note = 2'-O-methyl adenosine
  modified_base 15: mod_base = OTHER; note = 2'-fluoro cytidine
  modified_base 16: mod_base = OTHER; note = 2'-O-methyl uridine
  modified_base 17: mod_base = OTHER; note = 2'-O-methyl uridine
  modified_base 18: mod_base = OTHER; note = 2'-fluoro guanosine
  modified_base 19: mod_base = OTHER; note = 2'-O-methyl adenosine
  modified_base 20: mod_base = OTHER; note = 2'-deoxy thymidine 5'-thiophosphate
  modified_base 21: mod_base = OTHER; note = 2'-deoxy thymidine 5'-thiophosphate
tagtcgctgcgaaacttgatt

SEQ ID NO: 144 - RNA, 21 nt, synthetic construct
  source 1..21: mol_type = other RNA
  modified_base 1: mod_base = OTHER; note = 2'-O-methyl uridine
  modified_base 2: mod_base = OTHER; note = 2'-deoxy cytidine 5'-thiophosphate
  modified_base 3: mod_base = OTHER; note = 2'-O-methyl adenosine 5'-thiophosphate
  modified_base 4: mod_base = OTHER; note = 2'-fluoro adenosine
  modified_base 5: mod_base = OTHER; note = 2'-O-methyl guanosine
  modified_base 6: mod_base = OTHER; note = 2'-fluoro uridine
  modified_base 7: mod_base = OTHER; note = 2'-O-methyl uridine
  modified_base 8: mod_base = OTHER; note = 2'-O-methyl uridine
  modified_base 9: mod_base = OTHER; note = 2'-fluoro cytidine
  modified_base 10: mod_base = OTHER; note = 2'-O-methyl guanosine
  modified_base 11: mod_base = OTHER; note = 2'-O-methyl cytidine
  modified_base 12: mod_base = OTHER; note = 2'-fluoro adenosine
  modified_base 13: mod_base = OTHER; note = 2'-O-methyl guanosine
  modified_base 14: mod_base = OTHER; note = 2'-fluoro cytidine
  modified_base 15: mod_base = OTHER; note = 2'-O-methyl guanosine
  modified_base 16: mod_base = OTHER; note = 2'-fluoro adenosine
  modified_base 17: mod_base = OTHER; note = 2'-O-methyl cytidine
  modified_base 18: mod_base = OTHER; note = 2'-O-methyl uridine
  modified_base 19: mod_base = OTHER; note = 2'-fluoro adenosine
  modified_base 20: mod_base = OTHER; note = 2'-O-methyl guanosine 5'-thiophosphate
  modified_base 21: mod_base = OTHER; note = 2'-O-methyl cytidine 5'-thiophosphate
tcaagtttcgcagcgactagc

SEQ ID NO: 145 - RNA, 21 nt, synthetic construct
  source 1..21: mol_type = other RNA
  modified_base 1: mod_base = OTHER; note = 2'-O-methyl guanosine
  modified_base 2: mod_base = OTHER; note = 2'-O-methyl cytidine 5'-thiophosphate
  modified_base 3: mod_base = OTHER; note = 2'-O-methyl uridine 5'-thiophosphate
  modified_base 4: mod_base = OTHER; note = 2'-O-methyl adenosine
  modified_base 5: mod_base = OTHER; note = 2'-O-methyl guanosine
  modified_base 6: mod_base = OTHER; note = 2'-O-methyl uridine
  modified_base 7: mod_base = OTHER; note = 2'-fluoro cytidine
  modified_base 8: mod_base = OTHER; note = 2'-O-methyl guanosine
  modified_base 9: mod_base = OTHER; note = 2'-fluoro cytidine
  modified_base 10: mod_base = OTHER; note = 2'-fluoro uridine
  modified_base 11: mod_base = OTHER; note = 2'-fluoro guanosine
  modified_base 12: mod_base = OTHER; note = 2'-O-methyl cytidine
  modified_base 13: mod_base = OTHER; note = 2'-O-methyl guanosine
  modified_base 14: mod_base = OTHER; note = 2'-O-methyl adenosine
  modified_base 15: mod_base = OTHER; note = 2'-O-methyl adenosine
  modified_base 16: mod_base = OTHER; note = 2'-O-methyl adenosine
  modified_base 17: mod_base = OTHER; note = 2'-O-methyl cytidine
  modified_base 18: mod_base = OTHER; note = 2'-O-methyl uridine
  modified_base 19: mod_base = OTHER; note = 2'-O-methyl uridine
  modified_base 20: mod_base = OTHER; note = 2'-O-methyl guanosine
  modified_base 21: mod_base = OTHER; note = 2'-O-methyl adenosine
gctagtcgctgcgaaacttga

SEQ ID NO: 146 - RNA, 23 nt, synthetic construct
  source 1..23: mol_type = other RNA
  modified_base 1: mod_base = OTHER; note = 2'-O-methyl uridine
  modified_base 2: mod_base = OTHER; note = 2'-fluoro cytidine 5'-thiophosphate
  modified_base 3: mod_base = OTHER; note = 2'-O-methyl adenosine 5'-thiophosphate
  modified_base 4: mod_base = OTHER; note = 2'-O-methyl adenosine
  modified_base 5: mod_base = OTHER; note = 2'-O-methyl guanosine
  modified_base 6: mod_base = OTHER; note = 2'-fluoro uridine
  modified_base 7: mod_base = OTHER; note = 2,3-dihydroxypropyl thymidine
  modified_base 8: mod_base = OTHER; note = 2'-fluoro uridine
  modified_base 9: mod_base = OTHER; note = 2'-fluoro cytidine
  modified_base 10: mod_base = OTHER; note = 2'-O-methyl guanosine
  modified_base 11: mod_base = OTHER; note = 2'-O-methyl cytidine
  modified_base 12: mod_base = OTHER; note = 2'-O-methyl adenosine
  modified_base 13: mod_base = OTHER; note = 2'-O-methyl guanosine
  modified_base 14: mod_base = OTHER; note = 2'-fluoro cytidine
  modified_base 15: mod_base = OTHER; note = 2'-O-methyl guanosine
  modified_base 16: mod_base = OTHER; note = 2'-fluoro adenosine
  modified_base 17: mod_base = OTHER; note = 2'-O-methyl cytidine
  modified_base 18: mod_base = OTHER; note = 2'-O-methyl uridine
  modified_base 19: mod_base = OTHER; note = 2'-O-methyl adenosine
  modified_base 20: mod_base = OTHER; note = 2'-O-methyl guanosine
  modified_base 21: mod_base = OTHER; note = 2'-O-methyl cytidine
  modified_base 22: mod_base = OTHER; note = 2'-O-methyl adenosine 5'-thiophosphate
  modified_base 23: mod_base = OTHER; note = 2'-O-methyl cytidine 5'-thiophosphate
tcaagtttcgcagcgactagcac

SEQ ID NO: 147 - RNA, 21 nt, synthetic construct
  source 1..21: mol_type = other RNA
  modified_base 1: mod_base = OTHER; note = 2'-O-methyl uridine
  modified_base 2: mod_base = OTHER; note = 2'-fluoro guanosine 5'-thiophosphate
  modified_base 3: mod_base = OTHER; note = 2'-O-methyl cytidine 5'-thiophosphate
  modified_base 4: mod_base = OTHER; note = 2'-O-methyl adenosine
  modified_base 5: mod_base = OTHER; note = 2'-fluoro adenosine
  modified_base 6: mod_base = OTHER; note = 2'-O-methyl guanosine
  modified_base 7: mod_base = OTHER; note = 2'-fluoro adenosine
  modified_base 8: mod_base = OTHER; note = 2'-O-methyl cytidine
  modified_base 9: mod_base = OTHER; note = 2'-fluoro uridine
  modified_base 10: mod_base = OTHER; note = 2'-fluoro uridine
  modified_base 11: mod_base = OTHER; note = 2'-O-methyl guanosine
  modified_base 12: mod_base = OTHER; note = 2'-O-methyl adenosine
  modified_base 13: mod_base = OTHER; note = 2'-fluoro cytidine
  modified_base 14: mod_base = OTHER; note = 2'-O-methyl adenosine
  modified_base 15: mod_base = OTHER; note = 2'-fluoro cytidine
  modified_base 16: mod_base = OTHER; note = 2'-O-methyl cytidine
  modified_base 17: mod_base = OTHER; note = 2'-O-methyl guanosine
  modified_base 18: mod_base = OTHER; note = 2'-fluoro adenosine
  modified_base 19: mod_base = OTHER; note = 2'-O-methyl adenosine
  modified_base 20: mod_base = OTHER; note = 2'-deoxy thymidine 5'-thiophosphate
  modified_base 21: mod_base = OTHER; note = 2'-deoxy thymidine 5'-thiophosphate
tgcaagacttgacaccgaatt

SEQ ID NO: 148 - RNA, 21 nt, synthetic construct
  source 1..21: mol_type = other RNA
  modified_base 1: mod_base = OTHER; note = 2'-O-methyl uridine
  modified_base 2: mod_base = OTHER; note = 2'-fluoro guanosine 5'-thiophosphate
  modified_base 3: mod_base = OTHER; note = 2'-O-methyl cytidine 5'-thiophosphate
  modified_base 4: mod_base = OTHER; note = 2'-O-methyl adenosine
  modified_base 5: mod_base = OTHER; note = 2'-fluoro adenosine
  modified_base 6: mod_base = OTHER; note = 2'-O-methyl guanosine
  modified_base 7: mod_base = OTHER; note = 2'-fluoro adenosine
  modified_base 8: mod_base = OTHER; note = 2'-O-methyl cytidine
  modified_base 9: mod_base = OTHER; note = 2'-fluoro uridine
  modified_base 10: mod_base = OTHER; note = 2'-fluoro uridine
  modified_base 11: mod_base = OTHER; note = 2'-O-methyl guanosine
  modified_base 12: mod_base = OTHER; note = 2'-O-methyl adenosine
  modified_base 13: mod_base = OTHER; note = 2'-fluoro cytidine
  modified_base 14: mod_base = OTHER; note = 2'-O-methyl adenosine
  modified_base 15: mod_base = OTHER; note = 2'-fluoro cytidine
  modified_base 16: mod_base = OTHER; note = 2'-O-methyl cytidine
  modified_base 17: mod_base = OTHER; note = 2'-O-methyl guanosine
  modified_base 18: mod_base = OTHER; note = 2'-fluoro adenosine
  modified_base 19: mod_base = OTHER; note = 2'-O-methyl adenosine
  modified_base 20: mod_base = OTHER; note = 2'-deoxy thymidine 5'-thiophosphate
  modified_base 21: mod_base = OTHER; note = 2'-deoxy thymidine 5'-thiophosphate
  misc_feature 21: note = 3'-O attached to a GalNAc-comprising compound via a linker
tgcaagacttgacaccgaatt

SEQ ID NO: 149 - RNA, 21 nt, synthetic construct
  source 1..21: mol_type = other RNA
  modified_base 1: mod_base = OTHER; note = 2'-O-methyl uridine
  modified_base 2: mod_base = OTHER; note = 2'-deoxy thymidine 5'-thiophosphate
  modified_base 3: mod_base = OTHER; note = 2'-O-methyl cytidine 5'-thiophosphate
  modified_base 4: mod_base = OTHER; note = 2'-fluoro guanosine
  modified_base 5: mod_base = OTHER; note = 2'-O-methyl guanosine
  modified_base 6: mod_base = OTHER; note = 2'-fluoro uridine
  modified_base 7: mod_base = OTHER; note = 2'-deoxy guanosine
  modified_base 8: mod_base = OTHER; note = 2'-O-methyl uridine 5'-thiophosphate
  modified_base 9: mod_base = OTHER; note = 2'-fluoro cytidine
  modified_base 10: mod_base = OTHER; note = 2'-O-methyl adenosine
  modified_base 11: mod_base = OTHER; note = 2'-O-methyl adenosine
  modified_base 12: mod_base = OTHER; note = 2'-fluoro guanosine
  modified_base 13: mod_base = OTHER; note = 2'-O-methyl uridine
  modified_base 14: mod_base = OTHER; note = 2'-fluoro cytidine
  modified_base 15: mod_base = OTHER; note = 2'-O-methyl uridine
  modified_base 16: mod_base = OTHER; note = 2'-fluoro uridine
  modified_base 17: mod_base = OTHER; note = 2'-O-methyl guanosine
  modified_base 18: mod_base = OTHER; note = 2'-O-methyl cytidine
  modified_base 19: mod_base = OTHER; note = 2'-deoxy adenosine
  modified_base 20: mod_base = OTHER; note = 2'-O-methyl guanosine 5'-thiophosphate
  modified_base 21: mod_base = OTHER; note = 2'-O-methyl cytidine 5'-thiophosphate
ttcggtgtcaagtcttgcagc

SEQ ID NO: 150 - RNA, 21 nt, synthetic construct
  source 1..21: mol_type = other RNA
  modified_base 1: mod_base = OTHER; note = 2'-O-methyl uridine
  modified_base 2: mod_base = OTHER; note = 2'-deoxy thymidine 5'-thiophosphate
  modified_base 3: mod_base = OTHER; note = 2'-O-methyl cytidine 5'-thiophosphate
  modified_base 4: mod_base = OTHER; note = 2'-fluoro guanosine
  modified_base 5: mod_base = OTHER; note = 2'-O-methyl guanosine
  modified_base 6: mod_base = OTHER; note = 2'-fluoro uridine
  modified_base 7: mod_base = OTHER; note = 2'-deoxy guanosine
  modified_base 8: mod_base = OTHER; note = 2'-O-methyl uridine 5'-thiophosphate
  modified_base 9: mod_base = OTHER; note = 2'-fluoro cytidine
  modified_base 10: mod_base = OTHER; note = 2'-O-methyl adenosine
  modified_base 11: mod_base = OTHER; note = 2'-O-methyl adenosine
  modified_base 12: mod_base = OTHER; note = 2'-fluoro guanosine
  modified_base 13: mod_base = OTHER; note = 2'-O-methyl uridine
  modified_base 14: mod_base = OTHER; note = 2'-fluoro cytidine
  modified_base 15: mod_base = OTHER; note = 2'-O-methyl uridine
  modified_base 16: mod_base = OTHER; note = 2'-fluoro uridine
  modified_base 17: mod_base = OTHER; note = 2'-O-methyl guanosine
  modified_base 18: mod_base = OTHER; note = 2'-O-methyl cytidine
  modified_base 19: mod_base = OTHER; note = 2'-deoxy adenosine
  modified_base 20: mod_base = OTHER; note = 2'-O-methyl guanosine 5'-thiophosphate
  modified_base 21: mod_base = OTHER; note = 2'-O-methyl cytidine 5'-thiophosphate
ttcggtgtcaagtcttgcagc

SEQ ID NO: 151 - RNA, 21 nt, synthetic construct
  source 1..21: mol_type = other RNA
  modified_base 1: mod_base = OTHER; note = 2'-O-methyl uridine
  modified_base 2: mod_base = OTHER; note = 2'-deoxy thymidine 5'-thiophosphate
  modified_base 3: mod_base = OTHER; note = 2'-O-methyl cytidine 5'-thiophosphate
  modified_base 4: mod_base = OTHER; note = 2'-fluoro guanosine
  modified_base 5: mod_base = OTHER; note = 2'-O-methyl guanosine
  modified_base 6: mod_base = OTHER; note = 2'-fluoro uridine
  modified_base 7: mod_base = OTHER; note = 2'-O-methyl guanosine
  modified_base 8: mod_base = OTHER; note = 2'-O-methyl uridine
  modified_base 9: mod_base = OTHER; note = 2'-fluoro cytidine
  modified_base 10: mod_base = OTHER; note = 2'-O-methyl adenosine
  modified_base 11: mod_base = OTHER; note = 2'-O-methyl adenosine
  modified_base 12: mod_base = OTHER; note = 2'-fluoro guanosine
  modified_base 13: mod_base = OTHER; note = 2'-O-methyl uridine
  modified_base 14: mod_base = OTHER; note = 2'-fluoro cytidine
  modified_base 15: mod_base = OTHER; note = 2'-O-methyl uridine
  modified_base 16: mod_base = OTHER; note = 2'-fluoro uridine
  modified_base 17: mod_base = OTHER; note = 2'-O-methyl guanosine
  modified_base 18: mod_base = OTHER; note = 2'-O-methyl cytidine
  modified_base 19: mod_base = OTHER; note = 2'-fluoro adenosine
  modified_base 20: mod_base = OTHER; note = 2'-O-methyl guanosine 5'-thiophosphate
  modified_base 21: mod_base = OTHER; note = 2'-O-methyl cytidine 5'-thiophosphate
ttcggtgtcaagtcttgcagc

SEQ ID NO: 152 - RNA, 21 nt, synthetic construct
  source 1..21: mol_type = other RNA
  modified_base 1: mod_base = OTHER; note = 2'-O-methyl guanosine
  modified_base 2: mod_base = OTHER; note = 2'-O-methyl cytidine 5'-thiophosphate
  modified_base 3: mod_base = OTHER; note = 2'-O-methyl uridine 5'-thiophosphate
  modified_base 4: mod_base = OTHER; note = 2'-O-methyl guanosine
  modified_base 5: mod_base = OTHER; note = 2'-O-methyl cytidine
  modified_base 6: mod_base = OTHER; note = 2'-O-methyl adenosine
  modified_base 7: mod_base = OTHER; note = 2'-fluoro adenosine
  modified_base 8: mod_base = OTHER; note = 2'-O-methyl guanosine
  modified_base 9: mod_base = OTHER; note = 2'-fluoro adenosine
  modified_base 10: mod_base = OTHER; note = 2'-fluoro cytidine
  modified_base 11: mod_base = OTHER; note = 2'-fluoro uridine
  modified_base 12: mod_base = OTHER; note = 2'-O-methyl uridine
  modified_base 13: mod_base = OTHER; note = 2'-O-methyl guanosine
  modified_base 14: mod_base = OTHER; note = 2'-O-methyl adenosine
  modified_base 15: mod_base = OTHER; note = 2'-O-methyl cytidine
  modified_base 16: mod_base = OTHER; note = 2'-O-methyl adenosine
  modified_base 17: mod_base = OTHER; note = 2'-O-methyl cytidine
  modified_base 18: mod_base = OTHER; note = 2'-O-methyl cytidine
  modified_base 19: mod_base = OTHER; note = 2'-O-methyl guanosine
  modified_base 20: mod_base = OTHER; note = 2'-O-methyl adenosine
  modified_base 21: mod_base = OTHER; note = 2'-O-methyl adenosine
gctgcaagacttgacaccgaa

SEQ ID NO: 153 - RNA, 23 nt, synthetic construct
  source 1..23: mol_type = other RNA
  modified_base 1: mod_base = OTHER; note = 2'-O-methyl uridine
  modified_base 2: mod_base = OTHER; note = 2'-fluoro uridine 5'-thiophosphate
  modified_base 3: mod_base = OTHER; note = 2'-O-methyl cytidine 5'-thiophosphate
  modified_base 4: mod_base = OTHER; note = 2'-O-methyl guanosine
  modified_base 5: mod_base = OTHER; note = 2'-O-methyl guanosine
  modified_base 6: mod_base = OTHER; note = 2,3-dihydroxypropyl thymidine
  modified_base 7: mod_base = OTHER; note = 2'-O-methyl guanosine
  modified_base 8: mod_base = OTHER; note = 2'-fluoro uridine
  modified_base 9: mod_base = OTHER; note = 2'-fluoro cytidine
  modified_base 10: mod_base = OTHER; note = 2'-O-methyl adenosine
  modified_base 11: mod_base = OTHER; note = 2'-O-methyl adenosine
  modified_base 12: mod_base = OTHER; note = 2'-O-methyl guanosine
  modified_base 13: mod_base = OTHER; note = 2'-O-methyl uridine
  modified_base 14: mod_base = OTHER; note = 2'-fluoro cytidine
  modified_base 15: mod_base = OTHER; note = 2'-O-methyl uridine
  modified_base 16: mod_base = OTHER; note = 2'-fluoro uridine
  modified_base 17: mod_base = OTHER; note = 2'-O-methyl guanosine
  modified_base 18: mod_base = OTHER; note = 2'-O-methyl cytidine
  modified_base 19: mod_base = OTHER; note = 2'-O-methyl adenosine
  modified_base 20: mod_base = OTHER; note = 2'-O-methyl guanosine
  modified_base 21: mod_base = OTHER; note = 2'-O-methyl cytidine
  modified_base 22: mod_base = OTHER; note = 2'-O-methyl guanosine 5'-thiophosphate
  modified_base 23: mod_base = OTHER; note = 2'-O-methyl adenosine 5'-thiophosphate
ttcggtgtcaagtcttgcagcga

SEQ ID NO: 154 - RNA, 21 nt, synthetic construct
  source 1..21: mol_type = other RNA
  modified_base 1: mod_base = OTHER; note = 2'-O-methyl guanosine
  modified_base 2: mod_base = OTHER; note = 2'-fluoro adenosine 5'-thiophosphate
  modified_base 3: mod_base = OTHER; note = 2'-O-methyl cytidine 5'-thiophosphate
  modified_base 4: mod_base = OTHER; note = 2'-O-methyl cytidine
  modified_base 5: mod_base = OTHER; note = 2'-fluoro cytidine
  modified_base 6: mod_base = OTHER; note = 2'-O-methyl uridine
  modified_base 7: mod_base = OTHER; note = 2'-fluoro adenosine
  modified_base 8: mod_base = OTHER; note = 2'-O-methyl cytidine
  modified_base 9: mod_base = OTHER; note = 2'-fluoro cytidine
  modified_base 10: mod_base = OTHER; note = 2'-fluoro uridine
  modified_base 11: mod_base = OTHER; note = 2'-O-methyl uridine
  modified_base 12: mod_base = OTHER; note = 2'-O-methyl cytidine
  modified_base 13: mod_base = OTHER; note = 2'-fluoro adenosine
  modified_base 14: mod_base = OTHER; note = 2'-O-methyl uridine
  modified_base 15: mod_base = OTHER; note = 2'-fluoro adenosine
  modified_base 16: mod_base = OTHER; note = 2'-O-methyl cytidine
  modified_base 17: mod_base = OTHER; note = 2'-O-methyl cytidine
  modified_base 18: mod_base = OTHER; note = 2'-fluoro uridine
  modified_base 19: mod_base = OTHER; note = 2'-O-methyl guanosine
  modified_base 20: mod_base = OTHER; note = 2'-deoxy thymidine 5'-thiophosphate
  modified_base 21: mod_base = OTHER; note = 2'-deoxy thymidine 5'-thiophosphate
gaccctaccttcatacctgtt

SEQ ID NO: 155 - RNA, 21 nt, synthetic construct
  source 1..21: mol_type = other RNA
  modified_base 1: mod_base = OTHER; note = 2'-O-methyl cytidine
  modified_base 2: mod_base = OTHER; note = 2'-deoxy adenosine 5'-thiophosphate
  modified_base 3: mod_base = OTHER; note = 2'-O-methyl guanosine 5'-thiophosphate
  modified_base 4: mod_base = OTHER; note = 2'-fluoro guanosine
  modified_base 5: mod_base = OTHER; note = 2'-O-methyl uridine
  modified_base 6: mod_base = OTHER; note = 2'-fluoro adenosine
  modified_base 7: mod_base = OTHER; note = 2'-deoxy thymidine
  modified_base 8: mod_base = OTHER; note = 2'-O-methyl guanosine 5'-thiophosphate
  modified_base 9: mod_base = OTHER; note = 2'-fluoro adenosine
  modified_base 10: mod_base = OTHER; note = 2'-O-methyl adenosine
  modified_base 11: mod_base = OTHER; note = 2'-O-methyl guanosine
  modified_base 12: mod_base = OTHER; note = 2'-fluoro guanosine
  modified_base 13: mod_base = OTHER; note = 2'-O-methyl uridine
  modified_base 14: mod_base = OTHER; note = 2'-fluoro adenosine
  modified_base 15: mod_base = OTHER; note = 2'-O-methyl guanosine
  modified_base 16: mod_base = OTHER; note = 2'-fluoro guanosine
  modified_base 17: mod_base = OTHER; note = 2'-O-methyl guanosine
  modified_base 18: mod_base = OTHER; note = 2'-O-methyl uridine
  modified_base 19: mod_base = OTHER; note = 2'-deoxy cytidine
  modified_base 20: mod_base = OTHER; note = 2'-O-methyl uridine 5'-thiophosphate
  modified_base 21: mod_base = OTHER; note = 2'-O-methyl uridine 5'-thiophosphate
caggtatgaaggtagggtctt

SEQ ID NO: 156 - RNA, 21 nt, synthetic construct
  source 1..21: mol_type = other RNA
  modified_base 1: mod_base = OTHER; note = 2'-O-methyl adenosine
  modified_base 2: mod_base = OTHER; note = 2'-O-methyl adenosine 5'-thiophosphate
  modified_base 3: mod_base = OTHER; note = 2'-O-methyl guanosine 5'-thiophosphate
  modified_base 4: mod_base = OTHER; note = 2'-O-methyl adenosine
  modified_base 5: mod_base = OTHER; note = 2'-O-methyl cytidine
  modified_base 6: mod_base = OTHER; note = 2'-O-methyl cytidine
  modified_base 7: mod_base = OTHER; note = 2'-fluoro cytidine
  modified_base 8: mod_base = OTHER; note = 2'-O-methyl uridine
  modified_base 9: mod_base = OTHER; note = 2'-fluoro adenosine
  modified_base 10: mod_base = OTHER; note = 2'-fluoro cytidine
  modified_base 11: mod_base = OTHER; note = 2'-fluoro cytidine
  modified_base 12: mod_base = OTHER; note = 2'-O-methyl uridine
  modified_base 13: mod_base = OTHER; note = 2'-O-methyl uridine
  modified_base 14: mod_base = OTHER; note = 2'-O-methyl cytidine
  modified_base 15: mod_base = OTHER; note = 2'-O-methyl adenosine
  modified_base 16: mod_base = OTHER; note = 2'-O-methyl uridine
  modified_base 17: mod_base = OTHER; note = 2'-O-methyl adenosine
  modified_base 18: mod_base = OTHER; note = 2'-O-methyl cytidine
  modified_base 19: mod_base = OTHER; note = 2'-O-methyl cytidine
  modified_base 20: mod_base = OTHER; note = 2'-O-methyl uridine
  modified_base 21: mod_base = OTHER; note = 2'-O-methyl guanosine
aagaccctaccttcatacctg

SEQ ID NO: 157 - RNA, 23 nt, synthetic construct
  source 1..23: mol_type = other RNA
  modified_base 1: mod_base = OTHER; note = 2'-O-methyl cytidine
  modified_base 2: mod_base = OTHER; note = 2'-fluoro adenosine 5'-thiophosphate
  modified_base 3: mod_base = OTHER; note = 2'-O-methyl guanosine 5'-thiophosphate
  modified_base 4: mod_base = OTHER; note = 2'-O-methyl guanosine
  modified_base 5: mod_base = OTHER; note = 2'-O-methyl uridine
  modified_base 6: mod_base = OTHER; note = 2'-fluoro adenosine
  modified_base 7: mod_base = OTHER; note = 2,3-dihydroxypropyl thymidine
  modified_base 8: mod_base = OTHER; note = 2'-fluoro guanosine
  modified_base 9: mod_base = OTHER; note = 2'-fluoro adenosine
  modified_base 10: mod_base = OTHER; note = 2'-O-methyl adenosine
  modified_base 11: mod_base = OTHER; note = 2'-O-methyl guanosine
  modified_base 12: mod_base = OTHER; note = 2'-O-methyl guanosine
  modified_base 13: mod_base = OTHER; note = 2'-O-methyl uridine
  modified_base 14: mod_base = OTHER; note = 2'-fluoro adenosine
  modified_base 15: mod_base = OTHER; note = 2'-O-methyl guanosine
  modified_base 16: mod_base = OTHER; note = 2'-fluoro guanosine
  modified_base 17: mod_base = OTHER; note = 2'-O-methyl guanosine
  modified_base 18: mod_base = OTHER; note = 2'-O-methyl uridine
  modified_base 19: mod_base = OTHER; note = 2'-O-methyl cytidine
  modified_base 20: mod_base = OTHER; note = 2'-O-methyl uridine
  modified_base 21: mod_base = OTHER; note = 2'-O-methyl uridine
  modified_base 22: mod_base = OTHER; note = 2'-O-methyl uridine 5'-thiophosphate
  modified_base 23: mod_base = OTHER; note = 2'-O-methyl guanosine 5'-thiophosphate
caggtatgaaggtagggtctttg

SEQ ID NO: 158 - RNA, 21 nt, synthetic construct
  source 1..21: mol_type = other RNA
  modified_base 1: mod_base = OTHER; note = 2'-O-methyl uridine
  modified_base 2: mod_base = OTHER; note = 2'-fluoro uridine 5'-thiophosphate
  modified_base 3: mod_base = OTHER; note = 2'-O-methyl adenosine 5'-thiophosphate
  modified_base 4: mod_base = OTHER; note = 2'-O-methyl adenosine
  modified_base 5: mod_base = OTHER; note = 2'-fluoro cytidine
  modified_base 6: mod_base = OTHER; note = 2'-O-methyl adenosine
  modified_base 7: mod_base = OTHER; note = 2'-fluoro adenosine
  modified_base 8: mod_base = OTHER; note = 2'-O-methyl guanosine
  modified_base 9: mod_base = OTHER; note = 2'-fluoro cytidine
  modified_base 10: mod_base = OTHER; note = 2'-fluoro cytidine
  modified_base 11: mod_base = OTHER; note = 2'-O-methyl uridine
  modified_base 12: mod_base = OTHER; note = 2'-O-methyl adenosine
  modified_base 13: mod_base = OTHER; note = 2'-fluoro adenosine
  modified_base 14: mod_base = OTHER; note = 2'-O-methyl guanosine
  modified_base 15: mod_base = OTHER; note = 2'-fluoro guanosine
  modified_base 16: mod_base = OTHER; note = 2'-O-methyl uridine
  modified_base 17: mod_base = OTHER; note = 2'-O-methyl cytidine
  modified_base 18: mod_base = OTHER; note = 2'-fluoro uridine
  modified_base 19: mod_base = OTHER; note = 2'-O-methyl uridine
  modified_base 20: mod_base = OTHER; note = 2'-deoxy thymidine 5'-thiophosphate
  modified_base 21: mod_base = OTHER; note = 2'-deoxy thymidine 5'-thiophosphate
ttaacaagcctaaggtctttt

SEQ ID NO: 159 - RNA, 21 nt, synthetic construct
  source 1..21: mol_type = other RNA
  modified_base 1: mod_base = OTHER; note = 2'-O-methyl uridine
  modified_base 2: mod_base = OTHER; note = 2'-fluoro uridine 5'-thiophosphate
  modified_base 3: mod_base = OTHER; note = 2'-O-methyl adenosine 5'-thiophosphate
  modified_base 4: mod_base = OTHER; note = 2'-O-methyl adenosine
  modified_base 5: mod_base = OTHER; note = 2'-fluoro cytidine
  modified_base 6: mod_base = OTHER; note = 2'-O-methyl adenosine
  modified_base 7: mod_base = OTHER; note = 2'-fluoro adenosine
  modified_base 8: mod_base = OTHER; note = 2'-O-methyl guanosine
  modified_base 9: mod_base = OTHER; note = 2'-fluoro cytidine
  modified_base 10: mod_base = OTHER; note = 2'-fluoro cytidine
  modified_base 11: mod_base = OTHER; note = 2'-O-methyl uridine
  modified_base 12: mod_base = OTHER; note = 2'-O-methyl adenosine
  modified_base 13: mod_base = OTHER; note = 2'-fluoro adenosine
  modified_base 14: mod_base = OTHER; note = 2'-O-methyl guanosine
  modified_base 15: mod_base = OTHER; note = 2'-fluoro guanosine
  modified_base 16: mod_base = OTHER; note = 2'-O-methyl uridine
  modified_base 17: mod_base = OTHER; note = 2'-O-methyl cytidine
  modified_base 18: mod_base = OTHER; note = 2'-fluoro uridine
  modified_base 19: mod_base = OTHER; note = 2'-O-methyl uridine
  modified_base 20: mod_base = OTHER; note = 2'-deoxy thymidine 5'-thiophosphate
  modified_base 21: mod_base = OTHER; note = 2'-deoxy thymidine 5'-thiophosphate
  misc_feature 21: note = 3'-O attached to a GalNAc-comprising compound via a linker
ttaacaagcctaaggtctttt

SEQ ID NO: 160 - RNA, 21 nt, synthetic construct
  source 1..21: mol_type = other RNA
  modified_base 1: mod_base = OTHER; note = 2'-O-methyl uridine
  modified_base 2: mod_base = OTHER; note = 2'-fluoro uridine 5'-thiophosphate
  modified_base 3: mod_base = OTHER; note = 2'-O-methyl adenosine 5'-thiophosphate
  modified_base 4: mod_base = OTHER; note = 2'-O-methyl adenosine
  modified_base 5: mod_base = OTHER; note = cytidine 5'-thiophosphate
  modified_base 6: mod_base = OTHER; note = 2'-O-methyl adenosine 5'-thiophosphate
  modified_base 7: mod_base = OTHER; note = adenosine 5'-thiophosphate
  modified_base 8: mod_base = OTHER; note = 2'-O-methyl guanosine 5'-thiophosphate
  modified_base 9: mod_base = OTHER; note = 2'-fluoro cytidine
  modified_base 10: mod_base = OTHER; note = 2'-fluoro cytidine
  modified_base 11: mod_base = OTHER; note = 2'-O-methyl uridine
  modified_base 12: mod_base = OTHER; note = 2'-O-methyl adenosine
  modified_base 13: mod_base = OTHER; note = adenosine 5'-thiophosphate
  modified_base 14: mod_base = OTHER; note = 2'-O-methyl guanosine 5'-thiophosphate
  modified_base 15: mod_base = OTHER; note = guanosine 5'-thiophosphate
  modified_base 16: mod_base = OTHER; note = 2'-O-methyl uridine 5'-thiophosphate
  modified_base 17: mod_base = OTHER; note = 2'-O-methyl cytidine
  modified_base 18: mod_base = OTHER; note = 2'-fluoro uridine
  modified_base 19: mod_base = OTHER; note = 2'-O-methyl uridine
  modified_base 20: mod_base = OTHER; note = 2'-deoxy thymidine 5'-thiophosphate
  modified_base 21: mod_base = OTHER; note = 2'-deoxy thymidine 5'-thiophosphate
  misc_feature 21: note = 3'-O attached to a GalNAc-comprising compound via a linker
ttaacaagcctaaggtctttt

SEQ ID NO: 161 - RNA, 21 nt, synthetic construct
  source 1..21: mol_type = other RNA
  modified_base 1: mod_base = OTHER; note = 2'-O-methyl adenosine
  modified_base 2: mod_base = OTHER; note = 2'-deoxy adenosine 5'-thiophosphate
  modified_base 3: mod_base = OTHER; note = 2'-O-methyl guanosine 5'-thiophosphate
  modified_base 4: mod_base = OTHER; note = 2'-fluoro adenosine
  modified_base 5: mod_base = OTHER; note = 2'-O-methyl cytidine
  modified_base 6: mod_base = OTHER; note = 2'-fluoro cytidine
  modified_base 7: mod_base = OTHER; note = 2'-deoxy thymidine
  modified_base 8: mod_base = OTHER; note = 2'-O-methyl uridine 5'-thiophosphate
  modified_base 9: mod_base = OTHER; note = 2'-fluoro adenosine
  modified_base 10: mod_base = OTHER; note = 2'-O-methyl guanosine
  modified_base 11: mod_base = OTHER; note = 2'-O-methyl guanosine
  modified_base 12: mod_base = OTHER; note = 2'-fluoro cytidine
  modified_base 13: mod_base = OTHER; note = 2'-O-methyl uridine
  modified_base 14: mod_base = OTHER; note = 2'-fluoro uridine
  modified_base 15: mod_base = OTHER; note = 2'-O-methyl guanosine
  modified_base 16: mod_base = OTHER; note = 2'-fluoro uridine
  modified_base 17: mod_base = OTHER; note = 2'-O-methyl uridine
  modified_base 18: mod_base = OTHER; note = 2'-O-methyl adenosine
  modified_base 19: mod_base = OTHER; note = 2'-deoxy adenosine
  modified_base 20: mod_base = OTHER; note = 2'-O-methyl guanosine 5'-thiophosphate
  modified_base 21: mod_base = OTHER; note = 2'-O-methyl cytidine 5'-thiophosphate
aagaccttaggcttgttaagc

SEQ ID NO: 162 - RNA, 21 nt, synthetic construct
  source 1..21: mol_type = other RNA
  modified_base 1: mod_base = OTHER; note = 2'-O-methyl adenosine
  modified_base 2: mod_base = OTHER; note = 2'-deoxy adenosine 5'-thiophosphate
  modified_base 3: mod_base = OTHER; note = 2'-O-methyl guanosine 5'-thiophosphate
  modified_base 4: mod_base = OTHER; note = 2'-fluoro adenosine
  modified_base 5: mod_base = OTHER; note = 2'-O-methyl cytidine
  modified_base 6: mod_base = OTHER; note = 2'-fluoro cytidine
  modified_base 7: mod_base = OTHER; note = 2'-deoxy thymidine
  modified_base 8: mod_base = OTHER; note = 2'-O-methyl uridine 5'-thiophosphate
  modified_base 9: mod_base = OTHER; note = 2'-fluoro adenosine
  modified_base 10: mod_base = OTHER; note = 2'-O-methyl guanosine
  modified_base 11: mod_base = OTHER; note = 2'-O-methyl guanosine
  modified_base 12: mod_base = OTHER; note = 2'-fluoro cytidine
  modified_base 13: mod_base = OTHER; note = 2'-O-methyl uridine
  modified_base 14: mod_base = OTHER; note = 2'-fluoro uridine
  modified_base 15: mod_base = OTHER; note = 2'-O-methyl guanosine
  modified_base 16: mod_base = OTHER; note = 2'-fluoro uridine
  modified_base 17: mod_base = OTHER; note = 2'-O-methyl uridine
  modified_base 18: mod_base = OTHER; note = 2'-O-methyl adenosine
  modified_base 19: mod_base = OTHER; note = 2'-fluoro adenosine
  modified_base 20: mod_base = OTHER; note = 2'-O-methyl guanosine 5'-thiophosphate
  modified_base 21: mod_base = OTHER; note = 2'-O-methyl cytidine 5'-thiophosphate
aagaccttaggcttgttaagc

SEQ ID NO: 163 - RNA, 21 nt, synthetic construct
  source 1..21: mol_type = other RNA
  modified_base 1: mod_base = OTHER; note = 2'-O-methyl guanosine
  modified_base 2: mod_base = OTHER; note = 2'-O-methyl cytidine 5'-thiophosphate
  modified_base 3: mod_base = OTHER; note = 2'-O-methyl uridine 5'-thiophosphate
  modified_base 4: mod_base = OTHER; note = 2'-O-methyl uridine
  modified_base 5: mod_base = OTHER; note = 2'-O-methyl adenosine
  modified_base 6: mod_base = OTHER; note = 2'-O-methyl adenosine
  modified_base 7: mod_base = OTHER; note = 2'-fluoro cytidine
  modified_base 8: mod_base = OTHER; note = 2'-O-methyl adenosine
  modified_base 9: mod_base = OTHER; note = 2'-fluoro adenosine
  modified_base 10: mod_base = OTHER; note = 2'-fluoro guanosine
  modified_base 11: mod_base = OTHER; note = 2'-fluoro cytidine
  modified_base 12: mod_base = OTHER; note = 2'-O-methyl cytidine
  modified_base 13: mod_base = OTHER; note = 2'-O-methyl uridine
  modified_base 14: mod_base = OTHER; note = 2'-O-methyl adenosine
  modified_base 15: mod_base = OTHER; note = 2'-O-methyl adenosine
  modified_base 16: mod_base = OTHER; note = 2'-O-methyl guanosine
  modified_base 17: mod_base = OTHER; note = 2'-O-methyl guanosine
  modified_base 18: mod_base = OTHER; note = 2'-O-methyl uridine
  modified_base 19: mod_base = OTHER; note = 2'-O-methyl cytidine
  modified_base 20: mod_base = OTHER; note = 2'-O-methyl uridine
  modified_base 21: mod_base = OTHER; note = 2'-O-methyl uridine
gcttaacaagcctaaggtctt

SEQ ID NO: 164 - RNA, 23 nt, synthetic construct
  source 1..23: mol_type = other RNA
  modified_base 1: mod_base = OTHER; note = 2'-O-methyl adenosine
  modified_base 2: mod_base = OTHER; note = 2'-fluoro adenosine 5'-thiophosphate
  modified_base 3: mod_base = OTHER; note = 2'-O-methyl guanosine 5'-thiophosphate
  modified_base 4: mod_base = OTHER; note = 2'-O-methyl adenosine
  modified_base 5: mod_base = OTHER; note = 2'-O-methyl cytidine
  modified_base 6: mod_base = OTHER; note = 2'-fluoro cytidine
  modified_base 7: mod_base = OTHER; note = 2,3-dihydroxypropyl thymidine
  modified_base 8: mod_base = OTHER; note = 2'-fluoro uridine
  modified_base 9: mod_base = OTHER; note = 2'-fluoro adenosine
  modified_base 10: mod_base = OTHER; note = 2'-O-methyl guanosine
  modified_base 11: mod_base = OTHER; note = 2'-O-methyl guanosine
  modified_base 12: mod_base = OTHER; note = 2'-O-methyl cytidine
  modified_base 13: mod_base = OTHER; note = 2'-O-methyl uridine
  modified_base 14: mod_base = OTHER; note = 2'-fluoro uridine
  modified_base 15: mod_base = OTHER; note = 2'-O-methyl guanosine
  modified_base 16: mod_base = OTHER; note = 2'-fluoro uridine
  modified_base 17: mod_base = OTHER; note = 2'-O-methyl uridine
  modified_base 18: mod_base = OTHER; note = 2'-O-methyl adenosine
  modified_base 19: mod_base = OTHER; note = 2'-O-methyl adenosine
  modified_base 20: mod_base = OTHER; note = 2'-O-methyl guanosine
  modified_base 21: mod_base = OTHER; note = 2'-O-methyl cytidine
  modified_base 22: mod_base = OTHER; note = 2'-O-methyl uridine 5'-thiophosphate
  modified_base 23: mod_base = OTHER; note = 2'-O-methyl guanosine 5'-thiophosphate
aagaccttaggcttgttaagctg

SEQ ID NO: 165 - RNA, 21 nt, synthetic construct
  source 1..21: mol_type = other RNA
  modified_base 1: mod_base = OTHER; note = 2'-O-methyl adenosine
  modified_base 2: mod_base = OTHER; note = 2'-O-methyl cytidine 5'-thiophosphate
  modified_base 3: mod_base = OTHER; note = 2'-O-methyl cytidine 5'-thiophosphate
  modified_base 4: mod_base = OTHER; note = 2'-O-methyl cytidine
  modified_base 5: mod_base = OTHER; note = 2'-O-methyl adenosine
  modified_base 6: mod_base = OTHER; note = 2'-O-methyl adenosine
  modified_base 7: mod_base = OTHER; note = 2'-fluoro uridine
  modified_base 8: mod_base = OTHER; note = 2'-O-methyl adenosine
  modified_base 9: mod_base = OTHER; note = 2'-fluoro guanosine
  modified_base 10: mod_base = OTHER; note = 2'-fluoro cytidine
  modified_base 11: mod_base = OTHER; note = 2'-fluoro uridine
  modified_base 12: mod_base = OTHER; note = 2'-O-methyl uridine
  modified_base 13: mod_base = OTHER; note = 2'-O-methyl adenosine
  modified_base 14: mod_base = OTHER; note = 2'-O-methyl adenosine
  modified_base 15: mod_base = OTHER; note = 2'-O-methyl cytidine
  modified_base 16: mod_base = OTHER; note = 2'-O-methyl adenosine
  modified_base 17: mod_base = OTHER; note = 2'-O-methyl adenosine
  modified_base 18: mod_base = OTHER; note = 2'-O-methyl guanosine
  modified_base 19: mod_base = OTHER; note = 2'-O-methyl cytidine
  modified_base 20: mod_base = OTHER; note = 2'-O-methyl cytidine
  modified_base 21: mod_base = OTHER; note = 2'-O-methyl uridine
acccaatagcttaacaagcct

SEQ ID NO: 166 - RNA, 23 nt, synthetic construct
  source 1..23: mol_type = other RNA
  modified_base 1: mod_base = OTHER; note = 2'-O-methyl adenosine
  modified_base 2: mod_base = OTHER; note = 2'-fluoro guanosine 5'-thiophosphate
  modified_base 3: mod_base = OTHER; note = 2'-O-methyl guanosine 5'-thiophosphate
  modified_base 4: mod_base = OTHER; note = 2'-O-methyl cytidine
  modified_base 5: mod_base = OTHER; note = 2'-O-methyl uridine
  modified_base 6: mod_base = OTHER; note = 2'-fluoro uridine
  modified_base 7: mod_base = OTHER; note = 2'-O-methyl guanosine
  modified_base 8: mod_base = OTHER; note = 2'-fluoro uridine
  modified_base 9: mod_base = OTHER; note = 2'-fluoro uridine
  modified_base 10: mod_base = OTHER; note = 2'-O-methyl adenosine
  modified_base 11: mod_base = OTHER; note = 2'-O-methyl adenosine
  modified_base 12: mod_base = OTHER; note = 2'-O-methyl guanosine
  modified_base 13: mod_base = OTHER; note = 2'-O-methyl cytidine
  modified_base 14: mod_base = OTHER; note = 2'-fluoro uridine
  modified_base 15: mod_base = OTHER; note = 2'-O-methyl adenosine
  modified_base 16: mod_base = OTHER; note = 2'-fluoro uridine
  modified_base 17: mod_base = OTHER; note = 2'-O-methyl uridine
  modified_base 18: mod_base = OTHER; note = 2'-O-methyl guanosine
  modified_base 19: mod_base = OTHER; note = 2'-O-methyl guanosine
  modified_base 20: mod_base = OTHER; note = 2'-O-methyl guanosine
  modified_base 21: mod_base = OTHER; note = 2'-O-methyl uridine
  modified_base 22: mod_base = OTHER; note = 2'-O-methyl adenosine 5'-thiophosphate
  modified_base 23: mod_base = OTHER; note = 2'-O-methyl guanosine 5'-thiophosphate
aggcttgttaagctattgggtag

SEQ ID NO: 167 - RNA, 21 nt, synthetic construct
  source 1..21: mol_type = other RNA
  modified_base 1: mod_base = OTHER; note = 2'-O-methyl adenosine
  modified_base 2: mod_base = OTHER; note = 2'-deoxy adenosine 5'-thiophosphate
  modified_base 3: mod_base = OTHER; note = 2'-O-methyl guanosine 5'-thiophosphate
  modified_base 4: mod_base = OTHER; note = 2'-fluoro adenosine
  modified_base 5: mod_base = OTHER; note = 2'-O-methyl cytidine
  modified_base 6: mod_base = OTHER; note = 2'-fluoro cytidine
  modified_base 7: mod_base = OTHER; note = 2'-O-methyl uridine
  modified_base 8: mod_base = OTHER; note = 2'-O-methyl uridine
  modified_base 9: mod_base = OTHER; note = 2'-fluoro adenosine
  modified_base 10: mod_base = OTHER; note = 2'-O-methyl guanosine
  modified_base 11: mod_base = OTHER; note = 2'-O-methyl guanosine
  modified_base 12: mod_base = OTHER; note = 2'-fluoro cytidine
  modified_base 13: mod_base = OTHER; note = 2'-O-methyl uridine
  modified_base 14: mod_base = OTHER; note = 2'-fluoro uridine
  modified_base 15: mod_base = OTHER; note = 2'-O-methyl guanosine
  modified_base 16: mod_base = OTHER; note = 2'-fluoro uridine
  modified_base 17: mod_base = OTHER; note = 2'-O-methyl uridine
  modified_base 18: mod_base = OTHER; note = 2'-O-methyl adenosine
  modified_base 19: mod_base = OTHER; note = 2'-fluoro adenosine
  modified_base 20: mod_base = OTHER; note = 2'-O-methyl guanosine 5'-thiophosphate
  modified_base 21: mod_base = OTHER; note = 2'-O-methyl cytidine 5'-thiophosphate
aagaccttaggcttgttaagc

SEQ ID NO: 168 - RNA, 21 nt, synthetic construct
  source 1..21: mol_type = other RNA
  modified_base 20: mod_base = OTHER; note = 2'-deoxy thymidine
  modified_base 21: mod_base = OTHER; note = 2'-deoxy thymidine
gcgtcaccaaaaagcgcaatt

SEQ ID NO: 169 - RNA, 21 nt, synthetic construct
  source 1..21: mol_type = other RNA
  modified_base 20: mod_base = OTHER; note = 2'-deoxy thymidine
  modified_base 21: mod_base = OTHER; note = 2'-deoxy thymidine
ttgcgctttttggtgacgctt

SEQ ID NO: 170 - RNA, 21 nt, synthetic construct
  source 1..21: mol_type = other RNA
gcgtcaccaaaaagcgcaatt

SEQ ID NO: 171 - RNA, 21 nt, synthetic construct
  source 1..21: mol_type = other RNA
ttgcgctttttggtgacgctt

SEQ ID NO: 172 - RNA, 21 nt, synthetic construct
  source 1..21: mol_type = other RNA
  modified_base 2: mod_base = OTHER; note = 2'-deoxy thymidine
ttgcgctttttggtgacgctt

SEQ ID NO: 173 - RNA, 21 nt, synthetic construct
  source 1..21: mol_type = other RNA
  modified_base 2: mod_base = OTHER; note = 2'-deoxy thymidine
  modified_base 7: mod_base = OTHER; note = 2'-deoxy thymidine
ttgcgctttttggtgacgctt

SEQ ID NO: 174 - RNA, 21 nt, synthetic construct
  source 1..21: mol_type = other RNA
  modified_base 7: mod_base = OTHER; note = 2'-deoxy thymidine
ttgcgctttttggtgacgctt

SEQ ID NO: 175 - RNA, 21 nt, synthetic construct
  source 1..21: mol_type = other RNA
  modified_base 20: mod_base = OTHER; note = 2'-deoxy thymidine
  modified_base 21: mod_base = OTHER; note = 2'-deoxy thymidine
ctctgagttctgggatttgtt

SEQ ID NO: 176 - RNA, 21 nt, synthetic construct
  source 1..21: mol_type = other RNA
  modified_base 20: mod_base = OTHER; note = 2'-deoxy thymidine
  modified_base 21: mod_base = OTHER; note = 2'-deoxy thymidine
caaatcccagaactcagagtt

SEQ ID NO: 177 - RNA, 19 nt, synthetic construct
  source 1..19: mol_type = other RNA
ctctgagttctgggatttg

SEQ ID NO: 178 - RNA, 21 nt, synthetic construct
  source 1..21: mol_type = other RNA
ctctgagttctgggatttgtt

SEQ ID NO: 179 - RNA, 21 nt, synthetic construct
  source 1..21: mol_type = other RNA
caaatcccagaactcagagtt

SEQ ID NO: 180 - RNA, 21 nt, synthetic construct
  source 1..21: mol_type = other RNA
  modified_base 20: mod_base = OTHER; note = 2'-deoxy thymidine
  modified_base 21: mod_base = OTHER; note = 2'-deoxy thymidine
ggatagttactgaccgggatt

SEQ ID NO: 181 - RNA, 21 nt, synthetic construct
  source 1..21: mol_type = other RNA
  modified_base 20: mod_base = OTHER; note = 2'-deoxy thymidine
  modified_base 21: mod_base = OTHER; note = 2'-deoxy thymidine
tcccggtcagtaactatcctt

SEQ ID NO: 182 - RNA, 21 nt, synthetic construct
  source 1..21: mol_type = other RNA
ggatagttactgaccgggatt

SEQ ID NO: 183 - RNA, 21 nt, synthetic construct
  source 1..21: mol_type = other RNA
  modified_base 7: mod_base = OTHER; note = 2'-deoxy thymidine
tcccggtcagtaactatcctt

SEQ ID NO: 184 - RNA, 22 nt, synthetic construct
  source 1..22: mol_type = other RNA
caaatccccagaactcagagtt

SEQ ID NO: 185 - RNA, 21 nt, synthetic construct
  source 1..21: mol_type = other RNA
  modified_base 2: mod_base = OTHER; note = 2'-deoxy thymidine
  modified_base 7: mod_base = OTHER; note = 2'-deoxy thymidine
  modified_base 14: mod_base = OTHER; note = 2'-deoxy thymidine
ttgcgctttttggtgacgctt

SEQ ID NO: 186 - RNA, 21 nt, synthetic construct
  source 1..21: mol_type = other RNA
  modified_base 2: mod_base = OTHER; note = 2'-deoxy thymidine
  modified_base 7: mod_base = OTHER; note = 2'-deoxy thymidine
  modified_base 9: mod_base = OTHER; note = 2'-deoxy thymidine
  modified_base 14: mod_base = OTHER; note = 2'-deoxy thymidine
ttgcgctttttggtgacgctt

SEQ ID NO: 187 - RNA, 21 nt, synthetic construct
  source 1..21: mol_type = other RNA
gactttcatcctggaaatata

SEQ ID NO: 188 - RNA, 23 nt, synthetic construct
  source 1..23: mol_type = other RNA
tatatttccaggatgaaagtcca

SEQ ID NO: 189 - RNA, 21 nt, synthetic construct
  source 1..21: mol_type = other RNA
  modified_base 20: mod_base = OTHER; note = 2'-deoxy thymidine
gactttcatcctggaaatata

SEQ ID NO: 190 - RNA, 21 nt, synthetic construct
  source 1..21: mol_type = other RNA
tatatttccaggatgaaagtc

SEQ ID NO: 191 - RNA, 23 nt, synthetic construct
  source 1..23: mol_type = other RNA
  modified_base 7: mod_base = OTHER; note = 2'-deoxy thymidine
tatatttccaggatgaaagtcca

SEQ ID NO: 192 - RNA, 21 nt, synthetic construct
  source 1..21: mol_type = other RNA
  modified_base 7: mod_base = OTHER; note = 2'-deoxy thymidine
tatatttccaggatgaaagtc

SEQ ID NO: 193 - RNA, 21 nt, synthetic construct
  source 1..21: mol_type = other RNA
cagcgtcaccaaaaagcgcaa

SEQ ID NO: 194 - RNA, 23 nt, synthetic construct
  source 1..23: mol_type = other RNA
  modified_base 7: mod_base = OTHER; note = 2'-deoxy thymidine
ttgcgctttttggtgacgctgcc

SEQ ID NO: 195 - RNA, 21 nt, synthetic construct
  source 1..21: mol_type = other RNA
  modified_base 20: mod_base = OTHER; note = 2'-deoxy thymidine
  modified_base 21: mod_base = OTHER; note = 2'-deoxy thymidine
ggacattccaagacagtattt

SEQ ID NO: 196 - RNA, 21 nt, synthetic construct
  source 1..21: mol_type = other RNA
  modified_base 2: mod_base = OTHER; note = 2'-deoxy thymidine
  modified_base 7: mod_base = OTHER; note = 2'-deoxy thymidine
atactgtcttggaatgtcctt

SEQ ID NO: 197 - RNA, 21 nt, synthetic construct
  source 1..21: mol_type = other RNA
gaggacattccaagacagtat

SEQ ID NO: 198 - RNA, 23 nt, synthetic construct
  source 1..23: mol_type = other RNA
  modified_base 7: mod_base = OTHER; note = 2'-deoxy thymidine
atactgtcttggaatgtcctcag

SEQ ID NO: 199 - RNA, 21 nt, synthetic construct
  source 1..21: mol_type = other RNA
ttctctgagttctgggatttg

SEQ ID NO: 200 - RNA, 23 nt, synthetic construct
  source 1..23: mol_type = other RNA
caaatcccagaactcagagaact

SEQ ID NO: 201 - RNA, 23 nt, synthetic construct
  source 1..23: mol_type = other RNA
  modified_base 22: mod_base = OTHER; note = 2'-deoxy thymidine
  modified_base 23: mod_base = OTHER; note = 2'-deoxy thymidine
cagcgtcaccaaaaagcgcaatt

SEQ ID NO: 202 - RNA, 23 nt, synthetic construct
  source 1..23: mol_type = other RNA
  modified_base 2: mod_base = OTHER; note = 2'-deoxy thymidine
  modified_base 7: mod_base = OTHER; note = 2'-deoxy thymidine
ttgcgctttttggtgacgctgcc

SEQ ID NO: 203 - RNA, 23 nt, synthetic construct
  source 1..23: mol_type = other RNA
  modified_base 22: mod_base = OTHER; note = 2'-deoxy thymidine
  modified_base 23: mod_base = OTHER; note = 2'-deoxy thymidine
gaggacattccaagacagtattt

SEQ ID NO: 204 - RNA, 23 nt, synthetic construct
  source 1..23: mol_type = other RNA
  modified_base 2: mod_base = OTHER; note = 2'-deoxy thymidine
  modified_base 7: mod_base = OTHER; note = 2'-deoxy thymidine
atactgtcttggaatgtcctcag

SEQ ID NO: 205 - RNA, 21 nt, synthetic construct
  source 1..21: mol_type = other RNA
  modified_base 20: mod_base = OTHER; note = 2'-deoxy thymidine
  modified_base 21: mod_base = OTHER; note = 2'-deoxy thymidine
ccaatagcttaacaagccttt

SEQ ID NO: 206 - RNA, 21 nt, synthetic construct
  source 1..21: mol_type = other RNA
aggcttgttaagctattgggt

SEQ ID NO: 207 - RNA, 23 nt, synthetic construct
  source 1..23: mol_type = other RNA
  modified_base 22: mod_base = OTHER; note = 2'-deoxy thymidine
  modified_base 23: mod_base = OTHER; note = 2'-deoxy thymidine
acccaatagcttaacaagccttt

SEQ ID NO: 208 - RNA, 23 nt, synthetic construct
  source 1..23: mol_type = other RNA
  modified_base 22: mod_base = OTHER; note = 2'-deoxy thymidine
  modified_base 23: mod_base = OTHER; note = 2'-deoxy thymidine
aggcttgttaagctattgggttt

SEQ ID NO: 209 - RNA, 21 nt, synthetic construct
  source 1..21: mol_type = other RNA
  modified_base 20: mod_base = OTHER; note = 2'-deoxy thymidine
  modified_base 21: mod_base = OTHER; note = 2'-deoxy thymidine
tagtcgctgcaaaacttgatt

SEQ ID NO: 210 - RNA, 21 nt, synthetic construct
  source 1..21: mol_type = other RNA
  modified_base 7: mod_base = OTHER; note = 2'-deoxy thymidine
tcaagttttgcagcgactagc

SEQ ID NO: 211 - RNA, 21 nt, synthetic construct
  source 1..21: mol_type = other RNA
  modified_base 20: mod_base = OTHER; note = 2'-deoxy thymidine
  modified_base 21: mod_base = OTHER; note = 2'-deoxy thymidine
tagtcgctgcgaaacttgatt

SEQ ID NO: 212 - RNA, 21 nt, synthetic construct
  source 1..21: mol_type = other RNA
tcaagtttcgcagcgactagc

SEQ ID NO: 213 - RNA, 21 nt, synthetic construct
  source 1..21: mol_type = other RNA
gctagtcgctgcgaaacttga

SEQ ID NO: 214 - RNA, 23 nt, synthetic construct
  source 1..23: mol_type = other RNA
tcaagtttcgcagcgactagcac

SEQ ID NO: 215 - RNA, 21 nt, synthetic construct
  source 1..21: mol_type = other RNA
  modified_base 20: mod_base = OTHER; note = 2'-deoxy thymidine
  modified_base 21: mod_base = OTHER; note = 2'-deoxy thymidine
tgcaagacttgacaccgaatt

SEQ ID NO: 216 - RNA, 21 nt, synthetic construct
  source 1..21: mol_type = other RNA
  modified_base 2: mod_base = OTHER; note = 2'-deoxy thymidine
ttcggtgtcaagtcttgcagc

SEQ ID NO: 217 - RNA, 21 nt, synthetic construct
  source 1..21: mol_type = other RNA
gctgcaagacttgacaccgaa

SEQ ID NO: 218 - RNA, 23 nt, synthetic construct
  source 1..23: mol_type = other RNA
ttcggtgtcaagtcttgcagcga

SEQ ID NO: 219 - RNA, 21 nt, synthetic construct
  source 1..21: mol_type = other RNA
  modified_base 20: mod_base = OTHER; note = 2'-deoxy thymidine
  modified_base 21: mod_base = OTHER; note = 2'-deoxy thymidine
gaccctaccttcatacctgtt

SEQ ID NO: 220 - RNA, 21 nt, synthetic construct
  source 1..21: mol_type = other RNA
  modified_base 7: mod_base = OTHER; note = 2'-deoxy thymidine
caggtatgaaggtagggtctt

SEQ ID NO: 221 - RNA, 21 nt, synthetic construct
  source 1..21: mol_type = other RNA
aagaccctaccttcatacctg

SEQ ID NO: 222 - RNA, 23 nt, synthetic construct
  source 1..23: mol_type = other RNA
caggtatgaaggtagggtctttg

SEQ ID NO: 223 - RNA, 21 nt, synthetic construct
  source 1..21: mol_type = other RNA
  modified_base 20: mod_base = OTHER; note = 2'-deoxy thymidine
  modified_base 21: mod_base = OTHER; note = 2'-deoxy thymidine
ttaacaagcctaaggtctttt

SEQ ID NO: 224 - RNA, 21 nt, synthetic construct
  source 1..21: mol_type = other RNA
  modified_base 7: mod_base = OTHER; note = 2'-deoxy thymidine
aagaccttaggcttgttaagc

SEQ ID NO: 225 - RNA, 21 nt, synthetic construct
  source 1..21: mol_type = other RNA
gcttaacaagcctaaggtctt

SEQ ID NO: 226 - RNA, 23 nt, synthetic construct
  source 1..23: mol_type = other RNA
aagaccttaggcttgttaagctg

SEQ ID NO: 227 - RNA, 21 nt, synthetic construct
  source 1..21: mol_type = other RNA
acccaatagcttaacaagcct

SEQ ID NO: 228 - RNA, 23 nt, synthetic construct
  source 1..23: mol_type = other RNA
aggcttgttaagctattgggtag

SEQ ID NO: 229 - RNA, 21 nt, synthetic construct
  source 1..21: mol_type = other RNA
aagaccttaggcttgttaagc

SEQ ID NO: 230 - RNA, 21 nt, synthetic construct
  source 1..21: mol_type = other RNA
  modified_base 1: mod_base = OTHER; note = 2'-O-methyl guanosine
  modified_base 2: mod_base = OTHER; note = 2'-O-methyl cytidine 5'-thiophosphate
  modified_base 3: mod_base = OTHER; note = 2'-O-methyl guanosine 5'-thiophosphate
  modified_base 4: mod_base = OTHER; note = 2'-O-methyl uridine
  modified_base 6: mod_base = OTHER; note = 2'-O-methyl adenosine 5'-thiophosphate
  modified_base 8: mod_base = OTHER; note = 2'-O-methyl cytidine 5'-thiophosphate
  modified_base 9: mod_base = OTHER; note = 2'-fluoro adenosine
  modified_base 10: mod_base = OTHER; note = 2'-fluoro adenosine
  modified_base 11: mod_base = OTHER; note = 2'-O-methyl adenosine
  modified_base 12: mod_base = OTHER; note = 2'-O-methyl adenosine
  modified_base 14: mod_base = OTHER; note = 2'-O-methyl guanosine 5'-thiophosphate
  modified_base 16: mod_base = OTHER; note = 2'-O-methyl guanosine 5'-thiophosphate
  modified_base 17: mod_base = OTHER; note = 2'-O-methyl cytidine
  modified_base 18: mod_base = OTHER; note = 2'-O-methyl adenosine
  modified_base 19: mod_base = OTHER; note = 2'-O-methyl adenosine
  modified_base 20: mod_base = OTHER; note = 2'-O-methyl uridine
  modified_base 21: mod_base = OTHER; note = 2'-O-methyl uridine
gcgtcaccaaaaagcgcaatt

SEQ ID NO: 231 - RNA, 21 nt, synthetic construct
  source 1..21: mol_type = other RNA
  modified_base 1: mod_base = OTHER; note = 2'-O-methyl guanosine
  modified_base 2: mod_base = OTHER; note = 2'-O-methyl cytidine 5'-thiophosphate
  modified_base 3: mod_base = OTHER; note = 2'-O-methyl guanosine 5'-thiophosphate
  modified_base 4: mod_base = OTHER; note = 2'-O-methyl uridine 5'-thiophosphate
  modified_base 6: mod_base = OTHER; note = 2'-O-methyl adenosine
  modified_base 8: mod_base = OTHER; note = 2'-O-methyl cytidine
  modified_base 12: mod_base = OTHER; note = 2'-O-methyl adenosine
  modified_base 14: mod_base = OTHER; note = 2'-O-methyl guanosine
  modified_base 16: mod_base = OTHER; note = 2'-O-methyl guanosine
  modified_base 17: mod_base = OTHER; note = 2'-O-methyl cytidine
  modified_base 18: mod_base = OTHER; note = 2'-O-methyl adenosine
  modified_base 19: mod_base = OTHER; note = 2'-O-methyl adenosine
  modified_base 20: mod_base = OTHER; note = 2'-O-methyl uridine
  modified_base 21: mod_base = OTHER; note = 2'-O-methyl uridine
gcgtcaccaaaaagcgcaatt

SEQ ID NO: 232 - RNA, 21 nt, synthetic construct
  source 1..21: mol_type = other RNA
  modified_base 1: mod_base = OTHER; note = 2'-O-methyl guanosine
  modified_base 2: mod_base = OTHER; note = 2'-O-methyl cytidine 5'-thiophosphate
  modified_base 3: mod_base = OTHER; note = 2'-O-methyl guanosine 5'-thiophosphate
  modified_base 4: mod_base = OTHER; note = uridine 5'-thiophosphate
  modified_base 5: mod_base = OTHER; note = 2'-O-methyl cytidine
  modified_base 6: mod_base = OTHER; note = 2'-O-methyl adenosine
  modified_base 8: mod_base = OTHER; note = 2'-O-methyl cytidine
  modified_base 12: mod_base = OTHER; note = 2'-O-methyl adenosine
  modified_base 14: mod_base = OTHER; note = 2'-O-methyl guanosine
  modified_base 16: mod_base = OTHER; note = 2'-O-methyl guanosine
  modified_base 17: mod_base = OTHER; note = 2'-O-methyl cytidine
  modified_base 18: mod_base = OTHER; note = 2'-O-methyl adenosine
  modified_base 19: mod_base = OTHER; note = 2'-O-methyl adenosine
  modified_base 20: mod_base = OTHER; note = 2'-O-methyl uridine 5'-thiophosphate
  modified_base 21: mod_base = OTHER; note = 2'-O-methyl uridine 5'-thiophosphate
gcgtcaccaaaaagcgcaatt

SEQ ID NO: 233 - RNA, 21 nt, synthetic construct
  source 1..21: mol_type = other RNA
  modified_base 1: mod_base = OTHER; note = 2'-O-methyl guanosine
  modified_base 2: mod_base = OTHER; note = 2'-O-methyl cytidine 5'-thiophosphate
  modified_base 3: mod_base = OTHER; note = 2'-O-methyl guanosine 5'-thiophosphate
  modified_base 4: mod_base = OTHER; note = 2'-O-methyl uridine 5'-thiophosphate
  modified_base 6: mod_base = OTHER; note = 2'-O-methyl adenosine
  modified_base 8: mod_base = OTHER; note = 2'-O-methyl cytidine
  modified_base 12: mod_base = OTHER; note = 2'-O-methyl adenosine
  modified_base 14: mod_base = OTHER; note = 2'-O-methyl guanosine
  modified_base 15: mod_base = OTHER; note = 2'-O-methyl cytidine
  modified_base 17: mod_base = OTHER; note = 2'-O-methyl cytidine
  modified_base 18: mod_base = OTHER; note = 2'-O-methyl adenosine
  modified_base 19: mod_base = OTHER; note = 2'-O-methyl adenosine
  modified_base 20: mod_base = OTHER; note = 2'-O-methyl uridine 5'-thiophosphate
  modified_base 21: mod_base = OTHER; note = 2'-O-methyl uridine 5'-thiophosphate
gcgtcaccaaaaagcgcaatt

SEQ ID NO: 234 - RNA, 21 nt, synthetic construct
  source 1..21: mol_type = other RNA
  modified_base 1: mod_base = OTHER; note = 2'-O-methyl uridine
  modified_base 2: mod_base = OTHER; note = 2'-fluoro uridine 5'-thiophosphate
  modified_base 3: mod_base = OTHER; note = 2'-O-methyl guanosine 5'-thiophosphate
  modified_base 4: mod_base = OTHER; note = 2'-O-methyl cytidine
  modified_base 5: mod_base = OTHER; note = 2'-O-methyl guanosine
  modified_base 6: mod_base = OTHER; note = 2'-fluoro cytidine
  modified_base 7: mod_base = OTHER; note = 2'-deoxy thymidine
  modified_base 8: mod_base = OTHER; note = 2'-O-methyl uridine 5'-thiophosphate
  modified_base 9: mod_base = OTHER; note = 2'-fluoro uridine
  modified_base 10: mod_base = OTHER; note = 2'-O-methyl uridine
  modified_base 11: mod_base = OTHER; note = 2'-O-methyl uridine
  modified_base 12: mod_base = OTHER; note = 2'-O-methyl guanosine
  modified_base 13: mod_base = OTHER; note = 2'-O-methyl guanosine
  modified_base 14: mod_base = OTHER; note = 2'-fluoro uridine
  modified_base 15: mod_base = OTHER; note = 2'-O-methyl guanosine
  modified_base 16: mod_base = OTHER; note = 2'-fluoro adenosine
  modified_base 17: mod_base = OTHER; note = 2'-O-methyl cytidine
  modified_base 18: mod_base = OTHER; note = 2'-O-methyl guanosine
  modified_base 19: mod_base = OTHER; note = 2'-O-methyl cytidine
  modified_base 20: mod_base = OTHER; note = 2'-O-methyl uridine 5'-thiophosphate
  modified_base 21: mod_base = OTHER; note = 2'-O-methyl uridine 5'-thiophosphate
ttgcgctttttggtgacgctt